European Patent Application EP 4 299 725 A1, published January 3, 2024. Title: Novel bacteriophage having a specific bactericidal activity against enterotoxigenic Escherichia coli and antibacterial composition comprising the same. Applicant: CJ CheilJedang Corporation. The sequence listing filed with the application follows.

SEQUENCE LISTING (1 sequence)

SEQ ID NO: 1 - DNA, 170632 bp, bacteriophage CJ_Eco_20-4
cctatttattacttgctaaagcagcattaatgaatttttggagttcgtccatccgctctttagatggtttagggcatttattgatgactggtttacgataactcatttgcccgcctcaaattgtctcatctcatgcatggtcttaaggttaaaaccacgcgccttaatagcatcaagtgctgaactacaaaagtcttgtaataaagcccaatactgaattgatgtgtcgattttaattacactagaatccgcagccataacggtctttaattcagatttctcatattggtccatacaaacctcatcaccaggctctccacgtcccgtgtagaaatctaatcgcttcttaagtgaggtctttttctggatttctaatctcattatttctttcttacaattcgtatacagccttagccatttgctgtgcagcaaaacgttgttctgtacttcatattgtaaacgagttccatcaatctttaaatcctcgtctaatgcgtcctggaatgattctaacttatattcaatctctttactcatcgcatgtttcctgtgtaataaccataggaccattatacactattcatttgaacagcaattaaccactctgtgagagctggattctaatttgctctaatgtatctgggtcatcaacgatactaaactgaacggtcacgataatcgagttatcatcgtacacaggtgtcacacctacagctagagcagaaattctgggttcgaagttccgcactgcggaaactatattacgcttaatggtatccgtgattaatggagtaatattctcaaacaattggttgctgatgtcacaaccgaattcaggcataaaagggcgcgaacccttgcgagtagtaataatgcctaacaaactattttttactgcgcgagcacctgtagctttagcgacgtctctattccaagacgtcctcatttcagggtctaaatctgaatacattttattgatattcattacatcaccttaaagaactctttaagtccctcaataacgtggacggtgtgttcaccacattcacaagaaataggtatagccaaaataggcttaggggcgactagtgcatcataaacttcttttatatctttttctgttatcacagaataaaggtcatcaagttccgcatcgcttaaatcggaaagaaaaagcttttcgcctgcagaagttaaaatataatcgatacacccggcgaccatcatagctctatttttatcttcaaagagtttaggatatctgaaaacaattttaaagttgccaaagtctttaataacatccggctctttacccaatgttgctcgagttagtgtcatagggacaacctgtgagcgaccacaactacaactccactcacgttctatattcacttcagctaatgaatgggcccacaggtttatcaccaggagctcagattcttgcttgtttaaatcacgagcatctgtgcaattcgaaatgagttcattgataaaggactctattctgccttctaatttagcttggagcaagtccttatactctctgagggtaaatgctctgcattttatggttttgtttttaatttttacgtcaaaagtataattcattgtcttctcctttaagcttatttataaatacatcaataagaggacaccctatggctaatatagtacgttgtgaaatgcctgatggagtccaccgatttaaaccttttacagtagctgattatcgtgattttattttgattcgaaatgacatgaataataaatcgcctgaagagcaaaaacaaattttagatgagttactggaagaatacttcggtgaatatcctatgtcatggcgcccatatatgttcattgaactttatacgtcatcactcggcaagaccaaaattcctatccgatacacttgtagtaagtgtgaaaaggatagacaagttttattcaatttgaaacagaccaagttagataatcccacaattgaagtggccggcttgaagctaacattcaaatttccggaaatagaatatcaagacaaatccgaattgattctgaacaccctccaaaccgtggaagatgaaaacgggaaatataattggactgacctttctgaagaagaccaattagccgtaatagatgctatagacttatccactttagaggatatagtcaaacaaactagccctattaattttgaactaaaatatggatgctgtaatcgtagaacaattacgtataccgatattttagaggtgtttaagcttatagtcaacccggatgagatatttttattttaccaaataaaccatttactggtaaagaacaattattcattagaaagcattatgcagatgattccaatcgaacgcggtattgctttgtctttggttgaaaaggaccttaagaaatgagttcaaaaactatgcaacgtgaaggctttcctaatattagtatacgcctttacgaagattatgacgcctggttagagcatcgttttgttgaactaggcgcgacatttactactctaacaatgcgagatgggctttacggtagtaatgaagggttgcttcagttttatgatgcaaagaaccttcatactaaaatggacggtgagcagattattcaaatttctgttaagaatgctaactctgaacgtacccaatcaagaatttatggaagtaaacactttgctgtaggagtggattcgaagggcgacaatatcataacaatacaactcgccccaatccactttttagagaatcttaaatttagtcgtatgttcttcccgagtgttcaagaaacattaactgaaatgattggtgttatttatcaagaccgtccgcttcttgctcctcctttgaacgggataaacgtttacgttcctaatgttccttggtgtgattcaatggaccgttatatggaatttgtacgagaagtaggtatggccgttgaatctgataaatttgtatttgtctgggaagatatagatggtatttctatcatggactacgaatttatggttaaccaagagcctattaattttgtagtgggtgagccgcgattaataggtcaatacgttcaagatatggatacacctatcgcatttgattttgaatggttaactaaagccaaccaacattccagaaaaccatatgaaaacgctactgtatacgcccactctttcttagacaaaaacgccacacgaattacttttggtgacgggcaaaacagtatattggtttctcgctccggtggatattctgattatacctaccgaaacggttttgaagaagccgatagattagttactatggcccaatacgatggatacgctcattgtaaggtatatggtaactttgaactaactccaggcgataagattaatttctatgaccctaaaaaccaattccagtacgatttttatgtagacgaagttattcatgaagtgagtaacaatacatcaattacaaacctttatatgtttactaatggtaagcctattaagattgaagaaccgccgaaggttaaaaatgaacttaaaactgatactcccgatcaagaaaataacgctgggtgacaaagagatttccattcctaaattgggtcttaaacaccagaaattggttaaagatgaaaaggacccttacaaggccctctatatgacaatggaatccatttgtaaaggactgtctgcagcagaaacagattttgctgctttacaccttttagaattcaacggacgattaaaagaaaaagtaactaaagatggattcacatataatttaaatgacctttatatttgccaacgacttgaattccagttccaaggtaagacatttaaatttaaatcacacgaaccatttcaaacatttggtcctgttgatagtgtactacaatctctttatcttggtgatgatgtaccagattttctggatatgcctgcctttgttgctacatgggccgacgatataacttctactgtagctatccctggtcctaatggtcctatcaaaggattgcttaaaatcatggatatcttaaatgaagaacgaatctaatcagaatagttttcgtcgcaataaactgattgaagaaatggctcctcagcgtcgtgctgaggcgctagcccaaactcagaacgacgaattaggaaatatatcagatgttttatccgattcccaggcggcgtctgaattgctctctgaagttgttgagacaaagtctaaccagattattaattctgtagaccgagtagacaaaagcgtccaagatgttgtcgctggaacagaattaacggccgaagccatatcagaacaaacccaacagtctaaagctctttcggatgcattaaacgaaaagattaataagctttctaatatgttggaggctaaattttctggtatttctattccaccggaagggagctcattaaaggttattgaagactctattccagaagaacctaaggccgaaactcctaaagttcctgctgttgttgaagatattcttccacctgaagataataaacctgacgccgaatttatgcctgagcctcctaaaaattcagatgaaggtaaagaaggtgataagacttctctttccgagaaaatcgaagcccttactaaaataactgaaaagggatttaaagcttctataggcgtcgctgatagaatttcaggcatgctttttaagtataccattaccgctgccgctgaagctgctaaactcgcagcaggtttagtccttttaatatttggtatagatgccattcgcgtatacttccaatatttcatggaccaatttgagtcagggtggaaagaatttaacgataagtttaaagagtggggaccattacttgaagggctaatgacatgggccaagaatgctgaagccatgtttagtgaaggaaactggttaggtctggctgaagctattattcgtggtatggttaatcttaccaaaaatatggcacaacttttaatgcttggtatttctaagttgatttctgctattttaagtaaaatacctggtatgggtgatttagctgaaaacgtagaggcttctgctttaatgtcatatcagcaaaataccggagccactttggacgatgaagaccaaactaaagtggccaagtaccatgatagacgttcagccgaggctttagaaacagccgagaaaatgaataagaagtataaggataaacctgagcttataaaccaggcagagaaatacggtaatcttactaaagaacaagccgaccaattacgcgcaggtggaattgacacaagcttccgtgacctccctgaagaagaacgtttagagtatttcaagaaacgtgataaagctcaggctgatattattcgtttgacacaaaccgctgataatataatgaagccagattctaaagatatcgaaaatgctaaagcatttaaagctgatatcgagaaacaattggccgaccctattatggctaaaggtggggcaccgaaagaccttaatatccagcaattacttgataagatgaataaatctttagagaaatttaatgaagctgaaaagcctaaacctgcttctgtagtggaatctcctgaaaatacccaggttaaaaaggttgatgagcaaatgagagcaaaggaaaatgctaaatatagtcagcaagctccaactcaaataaatcagcaaacgaatatcaagaaaacgagtaagacaagctataatatgcccccacagtcctctactcctgctcctggtatgcgtcaagctactaaagttaattaggattaataatgaaagtaaaagaacttgactttgatgtagcctccttgtttaaaggaggttcaaagacctccgcaggtcaatctaaaacaccaccaataaaaaccacggtaaccgctcagtatccagctgagcgggcttcaggtaatgatacctcaaccgatatggtattaaacgacctctataaaaatggattgctttttaccgcatataattttagttctcgtgtatctccggatttgcgtaacgaccgttcgagtcaaatgactaaaaagttctcaagtgcagccagcaaattaacaggcaatagtggaacatatagtgctgttaaaaacttatttggtggaaatactaagggcgttaaatttgatacccaagccttagctaatatccttttacctcgttctaaatctgatgtggattccgtatcacacaaatttaatgatgttggtgagtccttaattactaaaggcggtggtactgctacaggtattttaagtaacgttgctagtaccgcggtatttggtgcattagaatctgtgactaacggcgtaatggctgattcaggcgaacagatatacactacagctcgtagtatgtacgccggtccggataaccgtactaaggtattcacttgggaaatgactccacgaaatgcccaagaccttatccagattattaaaatatacgaaatcttcaactattattcttacggcgaaacgggtaattcggctttcgcaggtgaattaaaagagaagattgatacttggtatcgttctacatttaaaaaagaagctattgacaagtttgatggtaagctattaggggaaagtattacaagcttcctttctaatgttattgtggtaagtaacccaaccatttggtatatccgaaactttggtgatagcagttcatatgatggtcgtgaagatatttttggcccatgccaaatccagagtatccgttttgataaaactccggacggccattttaacggattggctattgctcctaacttaccatctacgtttagtttagaagttactttccgtgaaattattactcttaaccgtggctcactttatacggaaggattctaatgtatactttacaagaatttcagaaccaggcaattaatattgacctacagaggaataacctgtttagtgtagtatttgctacggttccttcttctaaatcccaagcgctcctcgaccagtttggtggagctttatttaacaatatcccattgaatagcgatttgtttggtattacacaaggagagttgacccaaggtgttacgacattagtgacagcgggcactcagaagttgattcgtaagtcaggcataagtaaatatttgattggagctatgtcatccagggttgtgcagagcttactaggggagtttgaagtaggtacatatctgatggattttttcaatatggcctatcctacggcaggtcttttagtccacgccgttaaaatcccggataatactttgaactatgaaatggatttgaaccacaactcacctaacatcaaaattaccggaagagaatattctccattagtattaagcttccgtatggattctgaagctgctaactaccgtgcttttaatgattgggttaatagtgttcaagaccctattacacaattaagagcattacccgaggatgttgaagccgacattcaagtcaaccttcattctcgtaatggattaccccatacagtagtaatgcttaatggttgtgttcctgttggtgtttcgtcaccggaattatcctacgacggtgataaccaaattgcttcatttgatgttacatttgcttatagaagtgtacagacgggtgcagttggtaaacaagctgcttatgagtggttggaagataagattattaaaggcgtcgctgggctaagtgagagcaattcgctgagttcttcagtggccaaattaagtagactttcaggagcttctagtggattaacaggattggttaatacatttggtgggcgtgctattaataatggaatatcgaggctgttataacaaaaaaggagagcatatgctctcctttaggggtttatttacggaacgaaatgaaacctgctgcagtcattaatggctgctttttaacaaagaccgtgatagaaataggagcttcagattcgagttgtcctgtcactacaccgttaaaaatgttttcggtttgttctggataagaaaaattctcaacaggtcggatatcaaactgtttgtcttcaccgaaaactcgacgtaattcattacctacggcactgtcaaactcttcggaagcagggataacgttttcaactaccagttcttgaccattaaaacggaatgcagatttcataatgttctcctcatgtttgtgtaaggtaatagtaccacatccttgtggtgttgtaaactacattttgaatttatttgataaagaagagatatccaaagacgcggcaaggatttccatagcttcgttgctttcagaaacggattcattaaccaagaattgactaaatccatccatcaggcgaacttcaccagtttccatcaaatggtcaccatcgtaaacagattcgctgagctctgaaggaggcgttacggtagcttccataaggtatttgtgagatactctatcattcatggcaaaagccgctactttatcaaccttcaacaataatccacgcggaaggataatttctgcttcttcggcatattctgtaaggtcaccaggagcgataactttaactgcttcagcacctcgaataaccataccaatttcagcaattctatctgcaggaccttcaggtgcaattggattaccaaactcgtcttcttcccattctacctcttcgtcatcgacttcacccacatcagatgaactaccactagccaatttaaacaactcatcagcggaggacaaagaaccttcaccaccaacaaaaacggcttggttgtcgagggccatataatttttaccgaattcaccaaagatgttaggctttaatgaggctgacacaaagttcttaaagtaaaatgttttgttatcgatattatggcgcagaattttgtatggcaaatcctgaccacgatacaaaatagtacccttaggaagtttaatacccttagtaaatgctgagtctaaatccttaatcaatttaatagccgttgtattgttttcggattcaggtttacctaaaaggaataagttcataggagcatattcagccgcgcaatattcaataatagcattgctttcgtctttggttaggtccttaggtttaatgagctcgcctgaataagcatatgcatcactaatagaatcgttaaccagtttataaacggcttccatagcgaaagcaattctagatgctttctctgaaggggaacccttaaaacgggtactcaggttattaacaattttcttaataatatccagactattggttgtattgatttgcgaaaggccacttaaaagtctatcgacttctgtattaaaaaatgccatattattagagtaaatttcaaacccttgtttatctctattagcataatttagtttaaatttactatcagtcattaaagcgtgtgtgagagcaatagtgtatctaaagttggcaaggtcctcgctcttagatttaaactgagaagcctggcgcattttggtaatagcaccttttttaaagttctgactaatctgttcaataccttcattctcagggccttcagccgtgtgaaccggtacagaagcttcaaactcgttataaacctgcaattctttaggggacaaagtttcaggctcagcagtagaatactgtgcggctgctgccatacgacgggaaatcttagtacgggtaatgacagccttatcagtacgtttctcttcaacttgtgcaatagatgccgctactgcttcgaccttacttacggcctggccggttttcttagaaacatacacttcgccaactttagactcaactttagtataaagatcggcattaatttcaggcatacccttgatatcttcaatattagcaccacgacgtactaaaagaacgtaggtatgttttccgctgaattggaacatgtcgtcaacaactttaaacttaccaccggtacgagccatggccaagcgagctaatacgcgctgaacggtaggacctttacctttcattttcttagtagggaaacggaacaaaaccgcgtccattttaagtttgtttatttgttcatatatggtatcgaaaatggtgttcagtgtaccgagtggatcggtacccaaaccacccttgagttctgccggggcgcctttagcagataaactcattaggatgacatggacgtacttatcgcctggcttaaccattttaatagcatcgccttcagacgcataagataccatacgagcaaccaggttatcgttacctggcgcttggatagagaaaatctgtggaataccggaacccggtttaagatttgttactggatagtttttagcggaatcactatcaaaaacttcgtttaaattttccattatttacccttggatgaatttttctgggatgtcatagaggtctatgcatgaagccaaaagaggcagtacatcaaaccgtgtagatttaacaaatgaatcaaaagataaggggctttcggaagtatcgaagtcatcttgatatacgaccaactcgccggtttccattagtacatcaccatcatataccacagattcttgaagctcatctgttgtcataacttcagcttgaatgagttttgtattactagatgttgttccatcattattagaagcatctgttattttattaactttgaccattaatccacgcggtagaataacttcggcttcagttgctattccgagatttcctggatatacgacattaactttatgggccccatcaatagcccatcctatttgaactttaacataatcaggattttctttatatgctcttatttcattaggattaatagttattccttcttcatttttatcgactgtcaattcattgcgaacttcaggttctaaaagaccgataccagcgtgcgtaacaccaaaacgtccgaaaattataggggtcaatgaagtggatacaaaatttctaaaataaaacactttatttttaactagtgcttcgtatataggagcagtcatactctgggcacgataaactgtgatgccctctggtatacggtcgccattttcaaaagcagaatccaaattattaactgcagattcgatatctttttcgctcataacctcatagttctgaggattataacgtcctaaaagaagattatttatgtctgtatatcctgaaccacaatattctctgatgccgcgcttttgtgatggggtatatttagagccctcacgagcaatagtaatatcgaccataataccaccacctacaccagcaaaactatacacacgttttttaatgaacttagtcttggctgctttccacttggactcggttaattcattccagacgtcgtcaggttggcctttacgagttctgttatggatagccagccattcgcctttgtattcttcgaaaacggtattaatagcagaggcatatttttctagagctttaacagaggtcaaaggttcgtttttgatggccgtaagaattttatctttaattttctcttggatttcaccaataccgtgaagtgggaacaatttatagtcgtaatgcaattcttcagcagtgccttcagctactatattagcaaccttatttttagccgcaggagaattgttattagtaaccatttcctgagcctcagggattaatggaactgttgccggtttattaaaatccgctgcagtagcttcatatttcttaaacaattcactttcattacgataagattccaatgattggcttgctgcaatggcgcgcctagaaatcttagtcttggttataaccattttatcagtgcgacgttcttcaaccttagcaatactaccggcgatagcagtttctttagtaacctgcacgccttcttttttagaaatataaacttcaccgacatcagaatctaccttagtatacaattcagcattaattccaggcatacctttgatatcttctatatcagcttgtttacgaactaccaggatgtaagtatgtttaccggtaaattggtacatagccggaactactttaaaacgtccacctgttttctgtgctaccaaacgttggataatccgttgaacgatagggccttgacctttcattttcttagtagggaaacggaacatcacggcatccatacgaagctttttaacttggtcataaaccacatcaaaaatagtattaatcgcatctacgggagtagggcctaggccacctttaagttcggcaggcgaacctttagctgaaaggctcataaggataacgtgggcatatttatcacccatcttaacctgtttaatagcatcaccttcagaagcgtaggataccatacgcgccactaattgggattctgcgtcaccaatcttccaaatctggggtactttaagttttgggttcaagtttactgtaggcagtgtgccttcggactcaaacacttcatttaattgttcggtcataataattcctctttaataaccttatttatgccagaaaaggcccgaaggcctttattaaagtactaacagcgtacggtacacttcaaatttaggacccttttcatagcggtcgaaattatctttaaaatcagcgaacgcgatttcattttcaaattcaaggacaatttgggacactgcagtggagacatccccaccttctttatatccaataaccacggtttctaaataagctttcatattatagaccagtttgagaccaatcaccgaatacatcttcaaatgtatcagcttctgttttatcgaaacgccaacctttaatgattggaaggaaaatacctacagtatcagtacgtcctttagaatgaacccaaccattacattcacagtcagcaatacggccaatcaatttaccttcacgagcttgtttcataagaagttcacggtctaaatcaggccggtcttccaatggaatcaatacctttttacctgatttatctttcttatgggtggtatctttaaagcctgaaccacagtcacttgtaattcgacgacaacgtgatactaattcaacaccaccaagtttgttagggtccttcgagtgttcataataacctactacttctaaagcaatatcgattacttctttgaacttgataagattcttagaacggcggttttcccagtaggagtccatgttcttaaggataataccttccagaccttggtcgacatatttcttataaacgactttagcttcttcaagattattaacccactggttttcgatagcttcaacacgcgttgtaccatgcaatacgacattatgagcaaccataagttctaaggctgtaaagcgtacatcatacttatcgcctttaattttaccttcggaatatacgacatccaatgggacataatcccatgcctgtaataccataccagcggcttcagtagccgaaatagttccttgaagagctttgttagccaagccatttgacgtagaacgatcggcgacagtttggaattccttagccttacttaattcaggaagttcctcgtcaaacatactaaacaaatcattagatgctttaggttctaccttaggagtatggtaaactaattcgccatcaatcataacgccattaggatggcgttgtcgagcttcttcggtcatggccattaattcagccgccaaaagattaagcccttgatattcgttaccaccacgagtaaggaatgtcacaccatcgttacgaacttcggcaaaacaacgagcaccatcagcttttaattgagcaaacgctggccatttaatatttttcttaatcaaagcttcatcataagaactcgccaacatctgcggttgttcagggattaaacctttccaaaccttgttagcaatagaaatcgatgcaccacattcaaggtcgcgcatcattacacgacgtaatacctcggcatccggggccttagcatcagcaatgatttgagccagttcttcaatagccgcattacccgtaatcttacgtgtggctaatgtgaattcagcgaaatcaagaaggtcttcaagagtaatcataccaaaggattgagatgtaaatccaggttctggccactttttaataccgtagttcagacgacgggtataagccatacgataaacacgtttcagaagctcattgtccttttcacgagcaataatggcttctttagctttagtagaatcaatagcagcaatttcgtttaaaatatctaaaatcataatcacctcattagtcatggattctattataagccacatcagccaaaagcaagtctaatcgcttatgataagagaacacaaatctcattcgcccatcagatttgaacttggacataaagtggacataaatgaatccctgttcgacgcattcgcgccaaacaggatggtctttagccggatttacatcaaatgagtaatcatgattcacatgacgaataaactggtttacatgaccataatccattgtagtggtaggaccatagtctgaaattgtatgaactacaaacatattaacctcgagcaatccattcaactgcggcattattacgaagggattcgattgctgcgatatcgtcccatgaattaacctttacggctaaattaggtttaaagtcacgttcaccacgagctaaccaataaacttggatatccatgagaacattagatgcagcatcacagtggtgagccaaatcatcaacataaaacttaatacgtttaccgtacgtatttttagctcttatgaagaggtcttcttttgattctgaatgaccacacatcagaatctccttgaatgcgccagggaacaaagcattcaaattgaattgtctattcagcagtgcatcaattgagtcgcctagcgcagtcacggctacaaaatcgaagtcttttttgagcttgttgatatgttttaatgcgtccatgtaaggagacagataacgaataaaatctgactgattgtacttctcgattaaacgagcgcctaattcattatcacaattaaacagctcaccaggagataagaaacgttcgtcctgaatcatattcaaaatatgttctaaaggcaaattatatttctgtgcgaaataaggcaagccggactgccaacttaaacatactccatcgatatctgttaagataactggtttcataataaatctctcaatttgtttaggatgtcgataaactctttttcagttagtattgtatcacattctgtaaggtggctcgccatcgaatgctttaaaactttgccctttgtagcttgtaatgcgtcgcggaatcctttgttttggagcgctgcttcaaaataagcatttgtatacaactctttccatgatgcagagtatcttgaaaagggaattccaagccagaacagcgtcccacggtccgcagctctagcataagctcttccagtttgttgtgcggccagaccggacatcccaaatatacgtttttgttgttcatgatttctcaccttacatccttggaggaatccttcgagcccaccaaattggataccatccataacgaaaggccatttagcaaagttacttaatgcacacgatggccatggaaaattgcttcttatttctaactcagacatctttgacacttataatttcgacatcagcccaatgaccataaccaggtagacggtctttaatagataatccgccgtcagatttcagcattttaattgttttagtatatggttcatcttgtggatgcacaggagataaatcagttacacgataagtcacttcgaccatttccgtacctaataatttctgaatcaatttcttaaacatattatcctcgctttaaacatttgattacagacagttcaccgcccatgcgaacgtcttcagttccatcgacccataagacggtgtaggcttctttaataataacattacctaatttaaaagcaggtagaaccttggaaatcattccaggaatacctacgccttttaactggactgtttgcgataaaaatagttgcattagaacctcatctgaaagccgtgtgatttaacattaccaccatagatgtcagaggtattgacttcacgggcggcactagggtcgatattgatatcacggttgagcttagtgattgctaaggtatcacgaccattaacagtacggaattctacagggcatacaacatcagcataggccttaatagattcacgagtaggttgtttgtcggcaggaacgtctttacctgctttagagaaaacaacttcacagaaatttttacgagtatcgaaataagtggtcataaacataatattttcctcaaaggaggccgaagcctccatttttaagattagatatcgaattcgttcagaactacatcaaagattgcttccaggtgttcaggtttagctcggttgctcaggatgtgacgaatccaggttttaaccagaagcttacgattaacgccgttccagcaaggatgagtacctaaatcacgttgacggaaatcatcatctaaagctattttaaaagaagaaccttctttagtgattgaaagagtgataccattttcaaatcgcatataaacataatcaggagaaacccaatggtcgatttcgcaaactgaaccgtttttatgctcccataaacacatgtattcgttagaaccaaccgcaccgatagaaacatatttacgttcgaagttgatgtggttcattttattatcctttggtttagtttgttttcgtattatttggtacaggtctataataacacaacctgtaccaaagtaaactgttttatgcaactttaatccaattatctaaatttaattcacctttggctttcattttttcaatcaactcgtcagcagtagtgcgaccattttgataccatgtaacatcttcagaataaccggtttcttcatcttcataggtcttacaacgaatcttaccggttatgatagttttcagttcgtaggtatcaccggtaaaaaagtttgttaccataattttccaagagaagtcatcagaaggaccttccggagtcatgcaacctacaaattcaaattgttctttgtacaagtgccattgcatttctttagtttcgattgctttgtaaccgtcgtggtctttacatttgatatatgagttaagattgattttcattttattctccagtttgttttcgtattatttggtacatgtctatagtatcatgcctaccggagatgtacaccattttttaaagatttagaaacaaaaatgggactccgaagagtcccataacttatgcctgaggcttaccaaagcaagcagcatctgcacgcaataccgcacgagcacgagcttgaagcttatcaactacctgatcgatacgcttgttggacgcacgcttgtaaccagcgcgtttagaggtaccgtcaactactttaacttctttcttggccatttcaaatctcttaaattagaatgcaggacttattggcgttgcctgcgcaagccctcaaggggaacataggtttcggatatttaacgacaggataaccataaacctcgtcatcataccaaccacggcttagacagataacctttttctgacgcgtgatagtacaaaatacattcaagaggtacaccgtaaaactgttggggtcttaaaactataatgattcgcaaatcattaatcaaacagttcgacggctcctcgatttaacttacttcagggtaataataaaatgacgtactgctttacgagctgctgaagccaaaggcttagcaaatttcagttcatctttagcttccagttcagcagccagagtagcctgagcaggattcagatgtttgaaataacgcaggatttccagtgcttcggcctcaacatcaatagatgcgccgtagttttcgtgaccgttgttccaagcgttgcgttgcagttcaagagcgtgattcaattgtttgttcattttagtttctcaattcgagataaagattggtggacacgttcttctgaatttcacttcctttcggcaagtctctcagttgtagtccaccgcttaggattctccggttaactaactagtccggcagccaatccatattattatttatatcacttataaaggcaaggaatagctttatagtgacaggtaacgaatttttgtttaatttctttaggttgtttaatacccaatgcaaccaacggatgaggcacgttagcaatcttaccaacaggaagtggagtcaaatcgcctacttcacaaaaatcttcagggacatcaggtcctacagaataaatttcacaaagttcagggatttcaccttgatgaagtttgccaataacgataccagatgcagtagtttcttcatcaccggcttgttttggttcggaaacgagaataacatattctccgaccgctttaataggaagttccatatttaatccatattgttttgttgatagattaataataacacgctattcttaaagcatattacaggacaagcagagtttcagtctgaaggccgttaatagaaatcagcttatcgaaacggaatgagcgccaatcattaaccttggtatcaaatactctgatataattaacaggttctttattggcttctggcccaggggcctggacttctttatacggcagcaggtctaagtcgcgagtacaagtcatacgacgggcactaccatcagctttttcaaacaggacttcgtgaaaaccaacagacaaaatagtcttgactttttcacggagacgaatagtttcttgttcggttaaaatcataattattccagaatagttttgatagtggttgcattacgctcttttagagctcttaataggctatggcaattatcaagaataggcaccgttttatatttcatttcagcgcgaacccactcggatttatagtacgatttccaacgagagaaaaagtactttttatattctactgaataagctatcaggttttcaccttttgagttcagacctgaaaacttaactaaacgaaatttcattttgtttccttcaattaggatgcttagccttcgatttttatataatcaatgcggacaatatacttggtttcgccgccacgagtttctttacgaacttcacggactaataccaattctgggtttacatttaccaattggtcgataacatattcgatatcactagtagaatgagtcgaaatttcgccagtagaattgcctttaagctgttcaataacataaagtggacctactttaatagatttgatacctttttggagaagagcatcaataaatgtatctgtgtaatcaacagtaaccacttgtttaggtttttcaaataaaatattcattattcaccgcaatagttttgaattgattcccagttcaaagaacggagtcctgtacgattatactggataacttcgatgcctgattcacggaggatatcgtcccacccttcaggatttcggtcatagagctcagcataaaccaatgttttaattccagactgcgcaatagacttagcacaatcggcgcacggagataatgtcacgtacatcgtagcgccatcaatagaacttccggtacgagctgcaaacaaaatagcattcagttcagcatggatttcatttttagatgaccatgcagcgtgagccatgcggtgttctttaagaagaacagatttatgcgacatccgcgctgggtcatacacaacacgggtccagtcttgttccacagcatggtcacaacagttaacaccaccagaaggcgaaccgttatagcctgtagagataatgcgaccattcttttcgataaccgcacccactttccacgaacaacattttgattcttgagaaatcagatatgcaatctgaaggtatgtgcttgctttcattacatcaccactagataagctgtattattggtttcgacacgatataaatcggtacgaagtttagtgatagatttcacacgtgaggttaatataccataaccgtctgggaagcgtttttgtttatcgaaaaataccgctgccggaattcgatcaccaatttcaaccggaagaacagtagccagcacagcatcatatgttgaagtatggatgctttggaaatcttcactcagtttaaaaaggtctttgatgtactgagtagccttttcagagagacctcgatggtctccgtcttcgtcagattgtaaggtggcattaactgccggttttaaattaagcatcaatatacacccgctgcgcttcgaccagaccatcagaaccaagtttcaattgggtaacctggccgccatttttaagattaactataaccaataccgcacgtggtgtttcctggattactcgcagagttgcatcaggaaaatgtacagaaaccttattaatcagggcctgagcaaattctttaactttaacttggaactgctctacagtaataggttgttcgctcagcattagatggtctccaacttaagttgtttggtagtggtagcttgggtaacgtcgcctttaacaatataacacacttgttggaacgaattagtcaaaagctcttcggcctgacgatcggcttgttcctttgtgttatggcgagaatgaacttcaatcttaccatttttaacaataagcactttccaatcggctggagttttaataggtttgatttcagggttctggaaaactaactgcacttctttagggtctaccacttcgataaagtattcgaattcatggctaaaaaagcccgctgaattaaaaagaacactatttgcatcgtcaggattacctgtcattttgctcgggtcgacaaacatcatctcgtcatatacacgaattcggcttacacgtggcttcccgttatggtaatcaatttcaacttcaaacggattcatacccacatacttagcaaaagctgtattgaggccataagcaccgttattagtgaatttgtttttagtgtattcaccaacgaacttataaaacttacgctcttcaaagaactggctcatttcgatttcctcatttgtttcggtaaggtcatcatatcaccgtccttggtgaaagtaaacaccttttttaaattgcttcgacaactaccgtttgtttctggaagtccattttgcatgaaatagccaaaatgtggttatcaattttaaatgggacaattgcaattgctgcaccaggcgtgagttgaacagtgattgcatcaactgcatccgggaacatgatttccagaatagcagacaaacgaccatgcacctttagttcagtcgacgtgtcgacgggttcgtataggtaatcagatacaatctgactaaaaactactttaacaatttcagaataagtagggaacataattacctcagtgtacagtatggaccttcacgttaacaataaaccggtcaacgacttcagtcagaggaacgaactcaacatagtactcgcctttgtaacgttcattgaggtcattacgaagggctgctagtgagttaatgagggtaggagacatattctgacctaccagtttctgaagctctttataagcttcttcttcaacttcgtggtgtttgttatacataatgttcttccaagaaggcaaggagttcaggagcggatttaaaaataccaccatcgaccttgtcttcatctttatagtccataacatccaggccaatacgtccatcagttaaaggccatacgccgaagaaaaagcatttacgtttttcaatttcttcgattgtacgaaaaatcttttcgatattattcataggttttccatggtaatgggattttagtttgctttactgttaattcaatacctgggttcttggcttttaatttaaggcattcttcccaggctttagattgactagtgaatacacagaactgcccattgttggttccgactaaaccgccgtccacatgaacaacggcccaggtttcatggtgccaggccattaaaagtccccatgagcgacttgccaacattcaacaccgatacgccgccacatttcaaccacttgggtgcggtcgtcaatagctaatttaacatcaaagtgtggagcaattttttcccagaagatttcttccttaacaatatcatctttacggtcgtcgccttgttcgcgttggcactgcatgaccaatggtacaccagcaaagtcctcaacccatttacgagtcatacgataatatttcattgggtcttctttagtaccactttcacggccacttactacgataatctgataacccatatgggcatacatcttagtcagttcaaccaccattgggttgatgacgtcggtatcacacttctcaaggtcgtatggactacggtccgccattttggctagtgtaccatcaacgtcaaagataaccgctttaggtttgccaggagtccctgtataaaccggaagtccaagataagcccgcatatgactatacatggaacgcagaacgtcaataggtactgcttttgaaccgcgtttgttgttccgcttcacgagttcggtccaaggaacatcgaatactttatattcaactttccaaccgtattctttagcaaaggtttcccacatcaaacgacgttcaggattcaagttggtgtctgaaataattacacccttaacagaatcaccgccgtataaaatacccttcgccgcatcgaactgcatacaggtcacgataccttctttcttcttagagtatttgtattggtcgcgctcttcatgacccataattgattggcgatagtcatcacggttgatgttaaaatagccagggttcttagcgatgaattcacgagtccaagtgctcttgcctgagccaggacaaccaacagtcaaaataattttcttcatcatttaattcctaacagaattttaaggaggcgaatacgtaattcagtacgctcttcacctaatttggctacggccttattatttgatcggcgagaggtattggcagagatgaacataatcaaatgtttctttagttcacccatatcaacaccttgtgccttagccgctttacgtagagctttacctgcattatctaagatttgtccagcgtcttcatcatggtcacctaatttcaatccataacacaaatccacgtaattatctgagcacttgatataattctctaataactctttcatacaccaagttccttataaagttcttcacggcaagttttaagggttttacctgattcgtaagcaacactttcaggaacatcaccgagggttactgcggattgcatttgtccatggcgtttagccgcatattcaaaactttttactagctcgcgaatacgttctttttcattgtactcttcaatgaattcagggtattcccaaaccgggcgcatcatacgataccactgttggatggtgatataattacttccattcaaattaataatctgcgaaggctcaatagaccctggagcataaaaagttacctgtcttactacatcaataccgtccacaataacccaagcaaaattgaaagttgccttcttttcaagcggtgtacttgcacaggaccctaattttaagagcttttgtaatacaggagatttaacgcctgaaatgtattcaggcttagccacaaaactgttatcacgtaaagtcataataatttcctcaaattttataatccgtaggagcattatactctgctcccaagagtttgtaaactactttccgaaaagaccgccaatacatatactaatcagaattccaaaacaaaagcagacaaaaccaaatctaacaatatcccatccatcagtacacgcttcaatcatttgcacttctcctcttttagaccggaacgataataacataacatggatttctggtcttgtacatatctttttacgtcgttcaaccaaatacgatgttcttgggaatcttcaaatggcattccaacccaggccttaccgtcgattaccttaacctgccatttaacattatgttcggcgataggttgtggccacgaaggatgtagttgttgcttaggcactacagggatgtcctgggcacatccaactaacaagccaatagataatactactacagataatttaatcattctgtaatgctcctgaagtcttctgtaaaggaatcgaaggacttgttgatttgtttttcgaccaatcctggcttacttgccaccacgtgcgccttcttcgaatctttacggagcttttcattttctaccttaattttatccattcgggcattcatttcagtagtacggaattcaatatcagagtattggccatgtaggtcatctacggcttcggcattctgtttggccgtttgctgggttgttttcagttcttcagtaagggtatcaatacgacttgattgatatgaaataaaaccataagcacctactgcaatggctccagctaaaaggtaaatacttaatttagacatttggtaataatctcgatgatgtcatcacgtgacagggaattaataagaaccgttttaggattttcacactgaattttatacgtttcaaacataaaacataattcttcagcagtatggtaaggacttgaaatgccaaggcgattaaacttgtcgcttaatgggtcgcaaatcaaatagaacgtgatgcctgagattttaacattaggttggctaatattaataaacacctcggcatcgtatttggaaaggttgttttggagaaactcgaccatagagttaacagcttgaggcattgcttcacgcttttcttcagcgtaacgggtagagtattctttttgcttgattttctttttagcatttttagctaaagtaacacgaagatcggtcaggtaacctactgcacgagaacctttaaaaacttggatgccgtcagtagagtcaccaaaagccttaacaaccatttcgttagtaatcatttgcatattcattttgttttctcctcattagttggtaagtctatactaacacgtcatgaggagatgtaaactactctaccacaatttctttcaaatatttttcagggatttgggccttatgatttttcaagaacacagagttaatctggtccatgaccgtatcataattaataccgcctacgtacgcctgcataagaatagagaacaaccctgggaagtccttaaggattagctgtccagtaacggcatagtctttacggtcgcgacctttgagttgagagtaagctgcttctaacaaggctaatgattgttctaggtaatctaaatggatgcgttcaaaggcatcgattttctcgatagcaaaggaatctgtactgaacagaccacgaaggtcatcagttccaccagccactacaacttcaaacaaacgttcgttgttgttaatggaatctttggtatgatgcagtgcactgtaccaggcggttttgagtttaaagaacgtaccatctttcagtacaaagatgaaaccttcaataccttcttgtttacggatgttttctacgaaatcaccttcagcgaggtcatagctttcaaccaaatgcttacgcagggccccatctttaaacaattcagcatacggaatatattcacctgtttcattattacgaacgtttaacaggatgaggtttgtttcttggtaagccagcacgatacggttggtaggtgctacatattcaaggttgcaggtatacccagctttggtgatttcttctagacgtgcggcaaaagcctcgttctcagggagacgaaggaaccgtaaagaatcatgcaccattgatgaatggatagagcctttagatttaacagaaagatactgtcggtccatgaatgtagaaatcagagaaccatcttccttagccattacgaggtcgatattttctggcgacaaatctagaccgatagtcatagggttttcgtcaaggttaaagaacttttgcataggacgagcagcaatacgtactggaccgttctcgtccatttcaaacataatgcctcggcactctagtgcgccgtcttccaaccaatcactgtacgatgcatagttataactaaagatgcgatagttgactcctagcgcactctgaaagtctttaaagaagaacttagatttagtcgagtttttaaccagggccatcaagttatcatataattcaatcattgctttatcctatgttgggtattccaaggtggattaaatttctttatgaacattggctcttcaagagacatggtctcaactgacatagttccaagttcgttagtcatcgacagattaaagcactgccgtgcatagaactctacctttttacctgccattaatgcttcatgaatcagaatggacttggtcgaatctgacgtttggtccttacgattaatagcggttcggtagtagttgatgcgcttacgaagatttttagtcttcccgatgtagactagtatatcatcaaccgctatagcatatatgacattttgtttatttggtaccgtaagtggagctatggtggcgtcatcttggagttctagggtgacgtacttgataaagctaaattcgtctgcgatttctttcatagcaataaggggccgaagccccattccttaaaaatatttcttatacgatgccattactttttcatcaacatcgttatcaatttgtgctacaagataagaactgatttccacttcctgaggagcagcctgtacagcatcagagttcaggtattcgcgaatccaaggataaggatggcgggcaggagcatcagtaataggacacggtaagccacattgcttcatacgagaaactgtcaggtaatcgacaaaagcacccatgttctgagtatttaatccagggcaagtaccatctttgaacaggtgagcagcccattctttttcttgacggttaacttccatgaaaatatcaactgcttcttgttcacactcttgagcaattttaacccattcgtcaccatcagtaccaagttgaagttgacgaataatgtactgggtacccttaaggtgaagctgttcatcacgtgcaatgaacttcataatcttagcattaccttccatgatttccatgtttttatggaagttaaaggtgcatgcgaaagatacataaaaacgaatagcttccaatgcgttgattacatgaaggcaaaggtaaagggatttcattagctcacgcttccaatacatctcatgctcaatagcatcttcaatatcgtcttcgtctgcattaatttctttttggtattcgatatcagctttagcattctgccaatagcgagttttctcaataacgtcgtcgtaataacgaccaatagattcagcacgtttcataatagcgtcatctaacagaatttcatcaaatacctttgacgggtctgtatagaggttacgcatgatatgggtatatgaacgagagtgaatagtctcactaaaggtccatgtagccacccatgtatcaaggctagggtctgaaatcaaggcttgaagtgcagcagaaggagcacgtccttggatactatccagaagtgattgatacttcaggttattggtaaaaatattttgttggaattgtggaagcttattaaattgagcagcatccatcatcaagttgacttcttctggacgccagaaaaaactcaactgcttttcacaaagctcttcgaatactttatgacgttggatatcataacgagcaatacccaatcctgaaccaaagaacatcggttcggctaaaacatcaactggggtggtattaaaaactgtagacatgttattctcatttgttagtgactcatccatgagtcaattataatcagattttattaaagcttacaagctgcacaatcgtcggctttaggagtttcgatttcatagtcatcagtaccagagccatcacgggtattatgatagtaaaggttcttaccaccgtagtaccagaaatacagcaggtcatcaagcattaccgacatcggaacttttccttttggaaaaatctgtgggtcataatatgtattagctgatgccgattgacacacccatttcaacgctattgccacttgggtaagataaggtttattacctttcttagcgaggctccaagcgtaatcgtagagtccttggttatgttctacattaggaactacctgacggaagttaccttctttagattctttaatacttaccggaccacgtggaggttcgataccgtttgtagagttggaaacctggctgcttgattcacacggcataagtgctgataatgtgctattacggatgccatgtttagccaagtcttcccgcaacgacgtccagtcacaaacatagttaggggctgcgatttggtcaatctttttattgtaccagtcgataggtaattcgcctcgagaccatttagtgtctgaataatactcgcaatgtcctttttcttcggccagcttgatggatgctcggataagtccatattgtaatctctcaaacaattcatgagttaaatcgttagcgtcttcataagaagcaaagttgcttgctaaccaagcggcgtagttcgtaacaccaatacccaggttacgacgtttcttagccttcagagcttcaggaacaggataatcttggtagtccaacaggttatcaagtgcacgtacctggacttcagcaagttcgttgattttgtcttggtcctgccaatcgaagttatccagcacaaatgcagacaacgtacacaatccgatttcagcgtccggactattcacatcagtagttgggatagcaatttcacaacacaagttgctctggcgaataggagctttctcacgaataaatggtgtgaagttgttagtgttatcaacgaattgaggataaattcgtgcagtgcctgaacgttcagtcatgaacaattcaaagaggtcacgtgccttaatacgtttcttacgaatactagggtctttttctgcggcttcatacaattcacggaaacggtcttggtcttcgaaataagaatagtaaagctcaccacccatttcatgaggactaaacagagtaatgtaatcattcttaccgaaacgttccatcatcaggtcgttcaactggattccatagtccatatgacgaatacggttctcatcgacacccttgttgtttttcagaacgagcagattttcaacttccaaatgccaaataggataataagcagtagcagcgccgccacggattccgccttgtgaacatgatttaacagcagtctggaaatgtttccagaatggaataacaccggtatgcttgacttcgcccatgccaatacgagaaccttcagcacgaatcataccaacgttgataccaataccggcacgtttagaaatgtattcaattattgagttagcagttttgttaatagatttcagtgagtcgcctgcttcaataaccacacaagaactaaattgacgggttggtgtacgtgctccagccataataggagttggtaatgaaacctgacgggtacttacagcatcataaaaacgaataatatgtgctaaacgattacccggctcgtcttggtgtaaggccataccaatacacatgatagcgaactgaggggtttcgtagattttaccggttgttttatctttaaccagatatttctctttaagctgcatcgcaccagcataagtcaattcgaaatcgcgttcatgctttatatgagattctaagaaagtaatttcttctgcagaatatcgagacaacaattcagggtcatatttaccttcgttaacacaataggaaatatggtcgataaagctacgtggttcgaactggccgtaaacttctttacgcagtgcaaacatcaattgctttgcagcaacatactgatagtcaggttcttcaaccgaaataaggttggctgcgaccttaacagtcagattctggatatctttggtagtcataccatcacgaaggtgagatttgatttcttcgtataattcataggggtcgatttgggttccttcacagccccaagtcagaactttaataattttttgtgcgtcaaaatcttgggatacaccactacttttttgtacttgcataatttcctcaatgtgttaggttctacaattattctatcatagaacctgttaagcatggactgatatttatagaatgaaattcagtccaaccataataaccaaaaacagagtacagattatttgaattttcatacagccattttagccttaatagtagggtgtgattcgtaacctttaagaacgaaatcagacggcttcattgaatcaatccaggatagttgagtcttggtgtcccaaagaataaactcttccggtaaatcaatctcgagttcacaaagctctttaggctcacggcgtaatacttcttggcattgttcaatatggttagaatagatgtgcgtattgccgcctgagaacactaaatcgcctggaataagattacacattttagctacaatatgcactagagcggcgtaagaggcgatattaaatggcaatcctaagaacacgtcaacagaacgttggtaccactggaggtcaagatgaccattacgaacgttgaactgataaaaacagtggcatggaggaagagccatcttattaatttctgccgggttccatgctgatacgatttgacgacggtcattaggcattttcttaatgcgttcgacaatctctacaacctggtcgataccaccaaaatctcgccattgtttcccgtacacaggacccagttcgccatcagaataccccagagaaattgcctgattttcatagttttcgtcccaaatagttttaccttcagtacgcgtgccatgagtgcgccagcgaaggtcattaacattagtcgaacctgaaaggaaccaaaggagctcagcaatacaggctttccatgctaattttttagttgttaccgccgggaagcctttagttaaatcaaaacgtaatttagtaccgaacagtgcaattgtaccggtgccagtacggtcgtcagtttcgtagccattttccaggatatctttaattaaaaattggtattgtttcatttgtatactgtttccgtcagtgtagtaagttcgtctattttataccaatgggtttcaagcatttcacgttgacgaatttcatgaaggaagttttcttccaattgaaccgtagagttaacccgatggcatttctcgatacgagaaacaactacttcatcggcataaggtagtgcggcatataacaaagcaggaccaccgattacgcttactttagagcttggtccaagcataggttcaaagaacgtattaggacttgatacttggatttcaccacctgtaataaaggttacgtactgtgcccatgtgatatagaaatgggcgaaatcaccatctttagtttcaggataatcacggtcaaggtcacaaactacaatatgactacgcccagggagtaatccaggcaatgattggaatgtcttagcacccataatcatgattgtgtcttcagtacgtgctttaaaattctgaaggtcttttttaactcgtccccatggaagcccgtcacctaaaccaaatgcattttgttttgtgccatcaaccgtttcagttggagaataagcgaacactaatttaatcataatttcctcacgctttcttagcgattttccagtcagctttaaattggtcgacatcagagcggtgaatccagaagccagatgagctaccgtcttcataaagtgggcagccatcacactcatctttccaacccatcgcacacaaagcttgttcagctttttccagagcttccgggttattaccttggattgtgaagtaccatttgcctttaacttcagaatcgttgattgattcacgttgtaatttcattttattctccttagttgataaggctatagtatcactaccatagcctggtgtaaacttatttttgaattaggcccatataaaatttagcgtcttccgggtgcataccgtcacaatactcgtcagccataaagcgggtaaggtcttcaagaggaccttggacttcaatttgcatactacagaattgagtatctttaatatgggtcataactaaagaaggataacgattacggataacttcgtaagtgtattcaaaatcaacgatatcaatattaaccttagccattttattttcctcactcattagttgataggtctatagtatcatgtttaaaggcgttgtaaacatttatttttgaattttatcaagccatttaccaagtttaatcatttctttggtagctttttccatacttctaaatttaaccagtaaaggttgggcatcaacaccccataactaaggtggttacaagactatgttcacctacaagccataatgaataagtttggatatcgagcccgtaatttcggtctttatgaactcgtacacccatcacttcaaatttctcactggctttttctactgcatccaggaaatcatctttagtcatattaggccttaaaagttttttgcaaaagttcaatgatttggtcaacgttctgttcggtgacaatgcaatggatttgagtcacaccggccttagcaataggctcatcgatttctttatcttccacaacatattcacagaagcaatagaactcatcttcatgcaactcaaaataatttggcaccaacccaaatgcattataaatctcgccgttagcgcattcgatttcagtcacaaatttgtcgccatccatagtcaacatatcctttacttcaaaccaacctccgttgtcttggataaggtcgaccatgcttttattattttcatattcgtccatttcaataaagtctttaatgcattcaggacgaagttcataagttttaccgatttccatttttatttcctcatgtagttgataggtctatagtatcatgtttaaaggcgttgtaaaccattaaatgccaaaaagggaagaccgaagtcttcccattataaatcaataacttatagaccagctaacaggtcgtccagaccatcgtcatcagaaggacttactgacggctcaggagtagtggaacgagtcggtgtagatggtttagaatcatatgcatcaaggtctgcactgaatgcgtccaggtcatcaccaatcttatcagcggctgcagaagctttagcggcagcaccaccaagagcagctgtaccaacaactttcttaaacttggcttcgttagtttcgaatgatttgaaatcgagcagtttagaaaggtcgtgcatttcttccatcaatttagcttggtaagcttcatcattgatgttaggaatttcagactgacccatgaatttggaatcgtcatagttcttgaagtcgccaactttcttagatttcagtacgaagttcgcaccatcaaacggacatgttacgtcaaccggcacttcaccaatatcggtatcaacttcaaccatctggttgattttatccataattttctgaccgaaacggaatttaaacactttaccttcgttagcaggcactgcactatccttaataacaaggatgttagcccagaaggaagttttacgtttcatcagtttgtattcggcattattagtattaaaggtatcattctggttcatgtatttacatacaggacatgaatcgaaatcaccgtgtgtagacgtacagttttcaatgtaccattgaccatttttcttaaagccgtggttaacgagcttaatgaatggagatggattttcttcgtttttcgaaggtaggaaacgaattaccgcagtaccaacgccattgtcatctttcaatttccattcagctttatcatcggaagagaaagaagaaccacctttcattgcagacagttgagcagccagttgggaagggtctttacgtttaaacatattatttaccttagcagatttagcagttatattttattaacagtttttaacagattgagttagtatattaacacagttggtttgaagcattaaaacttacaagatttgatagtttcaatgaacaatttacgagcttctaaattatcgattataagaattttcttataagcatttaatttagtcgaatacttagaccatactaaatcgttggtctgttcatcatgtttatttattatatccataaatgaatcaagcaaaataaatgtttcgaatgaaatcacattcgattgaaggagcttaaaaatatagctcgagttaacttttttattataatcaaaaatttcagaaagcgcttgaacttccactttcttactaaaataataaatgtttttgatatcatcctcaaaaacttgttttattcttttaagtctaccgatatattctcggtaaaagactaaggcgtcggcatcactgatgtcgccaatccatgcgtcttggttagccaccaagttactcatgaaaataagagcaagctctttcaaagtgtatttatcactcaatttctcaaagaaatatttgtcacgacgtttttgataagccgtatcagagattcgcatgacccagttatattttataacgtcgtatttggcattgaagtgatgtttgagcattaagtatagtgaatatacgctcttaccattcaccatacggttattgtttggtggcatgcgaatcttaatcataacaagaaatccagagtattagttttttgcgttcgagccattgaaggtcgaagcaagttatcatcaatggcttcgttcataattttatcaataattcctgcaggcaaataacgagcaaagttaccttcagggatgctattctcttccaaccatgcggtagccgcttcgaggtaactacaaccttcagcttcaacaaaggcctcaatatcaaggccattctgttgtttgtttacgagcacatggacaggttcggaagcggtattaaccgctccatcaaaatcattcaaagattgtgtcatacagttctaccacttcagttttttcgtcttcgaaacgttcacgggtgcctttatggtacagagagaacagttggttaaacattttaccgtctacaccaagttcagtcttagcacggtctttgatatctttaatttcgtcaccgtaagcttccatttttaatttagtatcggaagcagacttaatcagttgtgccaatgtgttgccatgttcttcttgattgaattcaactttcactttttctttagccattatattcaccttaataaaaatcagctactgtagcggttagtttagacaaacccgatttaacgaaataaggataaactttagatttcgaaggtttgttatacgtattatatctttcagtaattaaagcaacaatatcatctggaataaagtccatatcaattaagatttggttttcacagaaacgttcatattgttcttcagtaagaagtgttttaattatatcatggtcgtaataattcagagcaatcgcttcaagttccttggcacgagtgctaggagtacgttcgccttcaaccatcgtcaaccagtaatcaccacgaactttaatactcgcgacgttatctttacggtcacctttaacaaccttagtcacgcaatcaagcaatgaatcgccagattttgttttgacgaattttttctgcattggagaccattgttttaccccagggaatttatggagttgggtaaagtcaccatcagaagaaccaatcataacagggtgacctaaagccgtgaggattcgggttaaaacagcaatatggtcatcggcctcgacagtatcgatgttcataacaatataaggcatgttatgttcaagctcatcaacaataatatgcattgccgtaaataagccttcccaatcaaataatgattcttcacgagccttagcacggtttttcttataataaggtgaatagcgacgacgccaataacctgatttagagttgtcaacacaaataaccagttggctgtaaccttgttttttaaagtctttaatgtttttcttaattgaattcaacacgaggtgtcgaagcattgctgtagttactttaggaaatccagcattctcaccaaactcttggaaagctgcagccataatgatttggctgaaatctaggagtaaaaatccatctttttgttggtcttcttcaggaagtaaaaaatctaaatcgttcatatgaacctctgtccaattagtgtagaggtccattatatcatgggttttaaggaagtaaacatcttgctataaatagttctataccctgaaaacgaaaaggaaataaaatggccgatattttaaaacctgccttccgtgctacatccggactcgatgctgcaggcgagaaagttatcaatgttgccaaagccgattacaatgtattagacgacggcgtcaacgttgaattctttatagatgagaacaccatccaggcgtacgacgagacgcgcggatataagaaagggtttgccgtaatccatgaccaacgtatctgggttgctcaacgtgatattgatgctccagcaggaacctttgtaccgggttattggactgctacccgtactgaccctaaatggattaccgtagcatctcctacacgccagctggcttccggtgaatatattgctgtggattctgctgctagctttactacatttaccctgcctccgaaccctactgatggtgataccatcgtaatcaaggatattggtggacgtgttggttataatgaaatcaaggttcagtctagttctgctccgggcggtggtaaccagaaaattgtccgtttcggtaaccagttcactgagaccttaattacgaagcctttttcctataatatgattatctttgccaaccgtttatggcatttctgggaagcagctaatgaagaacgtggtattcgtgtagaaccgaacaccgcccagttccaatcacaagcgggtgataacgttttacgtcgttatacttcaggtgcagtaattaagtttactcttcctaagtatgcgaaccaaggtgatattattaaaaccgttgatatcgatggtttaggaagtaaattccacttaatcgttgaaacatttgatgcgtcatcttcattaggtaagcctggccagcatagcatggaattccgtacttcaggtgatggattctttgtttataactctaccgaaaaattatggtatgtttgggacggcgaccgacaaactcgtttacgtgtaattcgtgacgatgttgaactcttggctaacgaaagtgttattgtttttggtcctaataacacgacaccccagacaattaatatcacattacctaccggtgtggcccagggtgttgtcgttaagattgctctgaactatctccgtaaagctcagacagtaaatattaaggctgccgtaggagataagattgcttcatccgtccagttgcttcaattccctaaacgttcagaatatccaccagaaaccgaatgggtattgaatgacgtactgacctttaatggcaatataagttatactccggttattgaactgagttatatcgaagacaccactacaggtggcaaatattgggttgttgcccagaacgttcctactatagaacgtgtggattctaaagatgatttaactcgtgctcgtttaggtgttattgcccttgcgtcccagactcaagcaaacgttgaccatgaaaataatcctgaaaaagaactggcaattactccgcagactttagctaatcgtgtggcgactgaatctcgtcgtggtattgctcgtattgctactactgctcaggtgaaccaggacacaaccttcgcattccaggacgatttgattatttctcctaagaaattaaacgaacgtactgcaaccgaaactcgccgtggtgttgctgaaattgctacgcaagttgaaactaacacgggtacagatgatactacaatcatcactcctaagaagctacaagcacgccagggttcggaaagtctttcaggtattgtaacatatacctctactgtaggaaccactcctgcgactgctagagacactgtaggtactaacgtttataataagaacgtaggcaatttggttatttctcctaaagctctcgaccagtataaagctacccaagttcaacagggtacagtatatctttctaaccaatctgaagttaacgcaggtcaatcggcaagtggatttgccaacagtgctgtttctcctgaaacattacatgctcgtgtggctcttgatactcgtacagggttaattgaaattgctacgcaaacagagactgatactggaacagattatactcgtgcggtgacgcctaagacgttaaatgataggaaagctacggaaggattgactggtattgctagaattgcaacacaggtagaatttgatgcaggtgtattagataatgttatttcaactccgttgaaaattaaaacaagatttaatgatactgctagaacttctgtctcagtagccagtggtttggttgaatcaggaaccttatggaaccattatacactagatattagagaagcaaatgagactcaacgtggtactgctcgcctggcgacccagaccgaagtcaacgttggtactgatgacaaaaccatcatcactcctttgaaattacactctaaaaaatctactgaaagttctgaaggtattattcgtgttgcaaccaataccgaaacaaccgcaggaacttctaaagttttggctgtaagcccttctggtttaaaatatgtagtacagaccgaaactacttgggaagctactgcacttcgtcgtggatttgttaaattaaccgaaggtgctttaacccattcaggaaataaagttactggttctggtgttaaattcaactcaggtacaggcctttatgagaacgatgatactgttctgaacgcagcgaactatcctaaaacgggttatgcggtttcatcttacgagatgaataaaactttacagaactttttacctataaatgctacggctgtgaactccgagaaattggatggcctagattcactccagttcattcgtagagacgttgaccaaacggttaatggttctttaacgttgacaaaacaattgaacctggccgctcctctggtgtcttctagtacggctaatattaccggcaacactattttaggttctctggaagtaaccggaaattctacttttaaaaatgatgtatctgttagctcaggtaaatctattaaatttgtaggaccccagtctggcgcaggttcttgggattctcaggcaactaattttgcacctattttctctgagataaattctactgttgatgctagttatcaccctattgttaagcaacgattagggcagggtactttctctttaggtactttaaatgacggttccggcgattttaaaatccatcatattagcagtgcttctggtgctttaaaatcttcctactggacctttaatacgaccggtgattttgctgttaatagtggttctattagtatttctaagaatgctaatatcacaggtataaccacttctaacggtgtttctacaaccacactaaatgcttctgctctgtcttcgttgcaaaacgtaactacttcaggtactatcgtttccaccggacaggtatcggcaaataatggtttggttgctcaaaaatacgtgcgctctgttggtgttaaacctacattagcatcgcaggcccctactgcagaaacagttggcttctggtctgtcgatatcaatgattcggctacatttaacctattcccaggttattggacgatgaaaactaaacgtcaggttaatattgatacggtccaaactaaacctgccggtgtttctgatgagatatggaatgcttctggttggttgacagaaacgggtgcatttagttctccggctattcgttatcgtaacgaagacggtagttttggtgacgaagttctcagtacgacgggtcagaaattacgtggtacttggtttgattattctgttcgtgataaggaagttaaatatcctggtacgttaactcagtttggtaatacattggattcatgttatcaggattgggtgtgctatcctacaggactgaatggtggtactattcgttatacacgtacctggcagaaaaataaaaacgcatggactacgttctctatggtctatacggcagataaccctccttctgcggaagaggttggtgcattgcctgctgataacgctacaatgggtaacattacaatccttgattggttacgtattggtaacgttcgtattattcctgacccggtcactaaatccgttaagtttgagtggattgaataagaggtattatggaaagatttatggcagaatttggacaaggatatgtccaggttcctacattatctgaaaacaatgctgtaaggtataaacttagtatagcgggtagttgtactaagtctaccacaaaagcatatgttaaatttcaagatgggaacttcggttcccagaattttcaaaatggattaaaccttatagaaattgatgttagtgctgaacctaaaatagtggctaacaaaacttatagttttacaaaagattttgatgttatttctgaagcttttataacgtatataaattctataccggccaatagaatagtttgtttagtatcttctggtagattaaatgcttcacaaaaacttatcgattggttccgtgcagcaggaagtaccgcattcccgtctaaatggttgatagaccggtttgagccgtcttattctgcattttatgtttcaggaaggaatgctatagtaatggaacatgtgctttataatgatggggtattggtcgaagatgtttctactccattagaagtggtatttgatgatatcagtgatgtcggtggtacaggatatcctgtcagaattgttgaagacgaaagcacttatctaagcaatgatggagatgaaattaagcgatttcctaccgaatctcctaccaccccattaacagattataacatgaagccaggtgaattcttttaccttaagtttcaattaatgcgcgaccaagctttaaaagacgtcgggacctctcagatgtctgttagattttttaatgcctcaggtgctttaaccgggacagttaatatggacgttccttccaacgttcctgctggtgcatggatgacatttgaacggctagtaatggttcctgaaggtactacagactttaccctttatgccagaaaaacagcttcggccggacaaggtggagttcgaaatgttatgttcggtgagatatctgaatcagaacctcagccaaaacccgctgaatttggtgttaacggtattcgtatgaactttggtacagaaactaaaaatatgggtactaccatagcccagctatatgataaaacaggcactaaacctggtcaggtttgggtcgctgaatttagagaaaaatattaaggaaccttcgggttcctttttcgttttctacggccataaatatataaaaggctataactcccaaaggaaactcaaatggcagatttaaaattaggttctacagcaggaggttcagtattatggcaccaaggtaatttccccttaacgcctgtatcaaatgaccttctttacaaaacgtataaagtttacaccgaatataataaaccacaagccgctgataacgactttgtttcaaaagcaaatggtggtaattataagaataacgtgtattttgaaaaaggcctgacctttaatgataccaatggatatggtattaaattaggagcaagaactggcggagccccgttcacggcttctttccgtattaaaggtgcttttggatatgaaacggaagacggtacaccgttcgttatatttgacccaagtacagtagtgggtgctaaacgcctcacagtaatgggtgattcattatcccgtcaagtttatgacgaatcaggtcgtgtattcagcccaggcaacacccctactaaagcccaagtcggattgccattagtagataacgcaaaacaagtccaaataaataatactaacatgcaaacaatgaccggagtacttgctgctcctaactttatttcgctgaatccggcctctgacgcaggacacgttcctcgttttgaccagattgttattaaagattctattcaagattttggttattattaagaggcattatggctactttaaagcaaatccaatttaaaagaagtaaagtagccggtgtacgtccagcaccggcccagttggctgaaggcgaactggctattaacttaaaggaccgtttactttttactaaagacgatactggagcgattatcgaccttggctttgctaaaggtggtaatattgacggcaatgttattcataccggtaactacaaccagactggcgattacaccctaaatggtacctttacccaaacaggtgattttaatttaaccggtattgctcgtgtaactcgtgacattattgccgctggccagataatgaccgaaggtggcgagcttatttctaagagtgcatcgacgtcccatttgagattttttgacggcgcatcccgcgaacgtggcattatcttttcgccaaataatgctggagcgaccactcaggtagttaatattcgcgtacaagattatgcgacaagtggcgaaagcacttatgcgttttcaggcaatggtgtgttttcttctcctgaagtttttggatggaaatctgtatcaactcccgtaatttatactaataaagttattactaataaaaaggttaaaggtgattatgatatctattcaatggccgataataacccattggcagaaagtgaaacagctattaaccaccttcgtgttatgcgaaatgccgttagttcgagcattttccatgaagttaaagataatgacggaataacctggtatgccggcgacggcttagaagcttatctttggtcatttacctggtccggcggattgaaagcgggtcattctatttctgtaggtcttccaggtggctctaaaggatattctgaattaggaacggcttcaattgctcttggcgataatgacaccgggttaaaatggcatcaggatggatattatttcagcgttaataacggcacgagaactttcctgtacggccctgcagaaaccaccagtcttagaaaaatggttatgggttattctgtaaacggtaccgatttaaccactcctccgtcggaaaactatgctttggcgacggttgtcacttatcatgataataacgcgtatggcgacggtcaaactcttttaggttattatcaaggtggcaattatcaccactatttccgtggtaagggtactacaaacgttaacaccgctggtggtttgttagttactcctggtaatattgatgttgttggtggttcggttaatattgatggccgaaataacaactcggttttgctttttaaaggttataccactggtcagagctctgttgataatatgtctattgccgtatggggtaacacctttaatacagtagatggcacccgtaaaaacgtaatggaaatatctgatgctactagctggatgcaatatattcaacgaacaactgctggtaaagtcgaatcggttctaaatggcacccagattgttaatgaaaacttgactgtagtaaaaaatgccacatttgatggtacaatcagcgctgccggtgaaatcgcgacaaatgccgtaaatggtcttcgtatttggaacaatgattacggtgccatttttagacgttcagaaggaagtcttcatattattcctacagcatttggcgaaggacagaatggtgatatcggcccacttcgtccatttagtatatctttagatacaggtaaggttgttattcctgacttggatttgagttatgcttcttttgcagcaaacggctatattaaattcggtggacatggtgcaggtgcaggcggttacgatattcaatatgcacaagcagctcctgttttccaagaaattgatgatgacgcggtaagtaaatattatcctattgttaagcagaaattcttacaaggaaaagctgtttggtctttaggtactgaaattaattccgggacttttgttttgcatcattacaaagaagacgggacccaaggtcatacatcaagatttaatgctgatggtacagttaatttcccggataacgtccaagttggtggtggtgaagctactattgctaaaaatggcaatattttctctgatatttggaaaacatttacttcagctggcgatgtaactaatattcgagacgctattgccacccgtgttgccaaagaaggtgatacgatgacaggccgtttaactctgaatgcaaactcggatgctattgttattaacagtgctgcaaccgaatctggttatgtgaaaggacaaaaagcaggcgttaataactggtatgttggtaatggcggcgctgataacaacttatcgttttatagtttccaaactaattcaggcgttaatattcataatagtggagaagttggtttagctcctcaaggggcggatactttttattttaatagggaccgtctttatataaagggttcacaatgggctgcacaccaagccggcgattggggtaatcaatggcgacaagaagctccggtgtttgtagattttggtaatgttggtaatgatagttattatccaattatcaaaggaaaatctggtattactaacgaaggatacgtatcgggtgtagattttggtatgcgacgcattactaatacctgggcacaaggtattattcgtgtaggtaaccaggaaaatggtcaagacccgcaagctgtctatgaattccatcatagcggcactttttatgctcctagtcttcttaagagtactagagtatcggctggtggtggtgacccagcatggactggaccatgtattgttatcggtgataacgacactggattggtatgggaagcggacggtattttcaacgcgtatgcaaacggtcaaggtgtattcagtttccgtgctgggcttgctcagacattcgccaacgtcgcccttaacgttaacgcagggatgtatgttcgtgataatattgatgttaacgacgtttatatccgttctgatattcgttgtaagtcggaaattaagcttatcgataacgctcaagagaaatccaaactcttaggtggttatacttatctgcttaaaaactctgtcacagatgaagttaaaccatctgcaggtttaattgcccaggaagttcaaaaagtattgcctgaacttgtgactgaagataaagagaccggcttacttcgtttaaactataacggtattatcggtttaaatactgctactatcaacgagcatactgacgaaatcaaggaattgaaatctgaaattgctgaattgaaagcattaattaaatcattattataagaaagggccttcgggccctggaggtttatatggcagtagtaggaattcctggttggattgggacttcagcggttgctgaaaccgggcaaagatggatgtcggccgcttcgagggaacttcgtttaggaaacccatcttggatgtcccaattcgctggccgctcaagagaaattattcacaccataacggcaaaccataactttaatggacaatggtttagagaccgttgctttgaagcaggtggtgctcctattgtgtttaatatcacaggtgatatagtatcttaccacagagatgttccactgttctttatgaacggggatactcctaacgaatatgttactttgaatattcacggcggagttcacatgtggggacgcggcgggcaaggtggttggacacactccggcggcgacggcaacgggcagtggggcggtgattgtattgttaaccatataggcacccgtttacgtatatggaactacggtgttatctgtggcggtggcggcggcggcggcggtatcgcttatcgtcctcactctggtgctaactggcaggatattggcggtggcggcggaagaccatttggcccaggaggtggaggtggctattctggtggtggagcttcttatgaaggcccgggtggtggatataactacggtaacgctcactctgggtctggtggcgatgcaggcggcgcaggtcaaaacgcctggtctgatggcgggaaagtgcttaaagtaggagcaggtggcggttctggtgcagctgttgcagtgtcatccccgatgtggggagcaacaggtactatctatggcccatggctataatacgaaagtattaaattataaatatctttaaaggagaaaagtatggaaccaaaagtaggattttcattaacagacctactttttggacttcttgatagaatttttaaagatacttcttccgggaaagtagttttttcccgggtcctagtcgtaatattattgttctttatggcattggtttggtataaaggcgagtatattctaaacttttataaagagactacttatgcctcttatactgaaatgattagacaagaccaggacaatagatttaaaattgtggctatcgagcagctccgaatagtgcattcttcttcaggcgcagacttcacagcagtatattcttttagacctaccaacatgaattattttgtggatatggtggcttatgagggtaaattaccggaaacggtagacgcaaaaaacacgggagggtttccaattgacaaaacgtcagtagagtatatggcgggagttaacgggaactattttgaatcaagtaccgaaactgtattccttcctacaaagaagaaaacacaattcacgtatatgttttcgtgcccgttttttaatttggataacgtctacgccggctcgatatcgttgtactggtatgatatcaaaccggatttaggatttcctagactttcgtctatgtgtggtcaggctgggaggacattaggtcgaacacgttagaaattggaggtatacatcattaagtaacggtgtatatcttcatacccttcattaaattgctcaataagagtatcacgttcatcttcagttaatgacttaaataatttgttataagacaaaccgttaagttcctttccatgttcattacgaatacccaactcattcaaaaaggcaataaactcatcacgacgttgcatgatgtcttcacaatccgttttaatcaaaatggaaacaatagtagcaatttcggaaacgatttcaattttagtcataatattctcttcaattcagtacgtcattatctgatagggctatactaacatatccttagggattgtaaacatgttcttcgttctttttaacatattcctgatacatctcttctattggttcctggaacttaaaatcagctcccaggaattcctcaaagcactcctgctcacgtgtacgcatgcctgttacggtattctctaagttatgactcatagcctttacccttatgtttctgtttacgtttagactctttaaagtttttcttcttatccttatggacagaagccttattgaaatcgtgcttagctaccagattgttcacgtaatttccttaattgatattcaagagagctgataatttctttattagttgcaatatacatgtcacgtaggaaaggcttcaacccttccatattaccatggattgtcttagaactaatattctttatatattcatggtctaaggcatcccaagccggctggttgacataagttccccagttgtcttccaccatgacattcagtcgtttaacatgattaatatgggcttcgattgcatcgatttgaagttgtttaagattcattagtaaaggtcctcagagtaaagttctttttcactaccaccacgttcaatacaaacttgtccagcgtaagtcgcaataatcattgcttcttcgcgagtccaatagtttgaatattggtcaataaatccttggtcatcaccacaaacatgggctgacataagtttatcacttacttggtcaagcacttctgccatatctttagaataatgacgagcgccaggaataaccagagtcccaccgtcttttaacttaaagcggttggctgcacacacaatcctgcgctgatatttttcattattgttccaataggcaatctgccaacatatttcaggaacctcttctaaaacatcctcttctgtatattcggtgtaatcaccatatgcccgtaatttagctgctagactttcaggcgtctcacgagaaagagctttatctaataaagccatacggtctttaaaggataatgctttaccttttaatggattcatttgaaaatcaccttatggccgttatctttagcaaattcttgaattttggtggcagtttcaattaaatcacctttataataggatgataatttaatatcaactgtttggccttcaccatatgaagatatgtttactttttctacaaaaataatttcaagaaatcgcaataaccgcataccaaattcaagatgaactttatcaatctggagattgagttgataaattttcttaataccatttaccagagccacacgctcatcccaatcattacgttgttcttcaatcaatttaagggaatgaccttcaccgtcccagttaagttccatcggaatcatttgaaccatcctttaacacgttgccataaagttttctgttgagctttattaacaccaattgaacgaataacaggttgtgattcctggtattctttgtagtccgctttatagacttcataagcggctggaataaaggtgctgattgccgccataaagtttttacgaattcccatagaagcttcagtaccaccacggatgattaggtatttaccggctttaatcttaacaatagttccaagataagcgccatggtaccaaatatcccaaccttcttgagtaggttctgcacaacgacgaagttcattaacaatattcagcttgttcataataatttcctcagattgcgttggttacggttttgataacttcagatgatacattttggaagtcgatataagtattcttaccaccggtcttaatcttaacatcaagattcaaggaagtaaacacttgtttttctttatcggtcatattataaccgaagatgcgcatcattccgtcacgacggacttcaatttgacgaataccattggtacgtttggcgaatcgaacttcaaggttgctacggttttcagcaatttcacgaatctcgatacggtcttctaataaagctttaacttcatcagccagtgttaccatttcaggagtaacaccacgtgaactacgcgttttacgtttttccaacatctctggagcattttcagaagcgaacaagtcagcagctttttgaactaggtccattgcttcacctgtagccactagtccgtcaccagatttttcgatgaatcctttcttaattaatacaccgatattagagttaactaccgcagcactaaattgctcactcagggcttcacggacttcgcctgaagtgatgaagttatgcttgatgatatgtactaagatcgaagccgttttttcattcaggacgtcttcagaagctttgatggtataagtaattttagacattttaatctccgataaccatttatttgataggtctatagtatcatgtttaaagcagaagtaaactttattttgagctctttttcaagagctctaataaagtacttacttaatgttcagattacgaacttcgatttcgtcttcaggggcaaaatcaaactgtttgaattctgtgtcacctttaaatttaaaaatcattgtgaagaaagtcagaacaccgggtttttcttcacgaactccacatatatcatattcaataccatctacaaccagtttgttagcagtcagagcatttttagctttaacgatttcgttttcgattttaaatttcatttttgtatctccgggttgtttgtttcagttcatttatttgataggtctatagtatcatgtttaaagcagatgtaaacacttttttgctaaacccaaaaaaggaacccgaaggttccttactttttaaagtgggctgctattaaacctatagctaagcctgttgccaggcctagaataacagcaaagatacagagtaacaagaactcgactccaaggctcatagagcctccaaatctttaacatactcagttaccacatcagtggttttccagtattgatgctcttctttcttagccttggcttcgagggccagtttcttggcttcatcagaagtgatatggaaaatgttcattgcaaccagtttatcagcgtattcgccatagactttattaccagccaattcctcagttaaaaccttacgagtcttaccttggataactacagtcccatcaataacatctttgatgaatgtagctttagccaatgatagtttgaaagcttcttcggtttcgatgattttaccatcaatacgtttctgtacaaaggtcttacggacctcaacgaaatcacgaatcagatcaactgcatcttcgtaaaccttaagtttacctttctcattaatgacagtcaggttttgtgaacgacgttcaattaacccgaagtccttcatgagtttttcgtgtttcttatcttcatcagtaggcaattcatattctttacgaatcttaaccttgaagccgaaaccattctcatcacagtcatcatcatatgtgatgtaccctttgtcttccagagggtctaataccttagccacatatgtttcacggtcatatttgtatgggatttccgtgatatgcatttgggttcgagatgtgaacttatacgttccacgaatctcataactacctggttcaatttcaacaacttcaccacggaattccggataagccactttaggcttggttacacgtttttcctgaagaacttgcaatacagctttcttaacagaatcaaaactatgaggaagaatattagttgcataaccagttgcaataccggaaacaccattaagaagaacagtaggaataataggcagataaaaagccggtggcttatgttcgacatccgcatgaaccggagcatattctgtgtccttataaacttttgcaaagttacttccaatacgagcaaaagtataacgagaggccgcagctttttgaaccaatcgggaaccaaagttaccttgaccatctaacaatgggtagttgttattccatgtgttagccattagtgctaaagcttcttgggccgaattctcaccatgatgataacccaagtcggcaacaccaccggcaatagaagctagtttatggaatttgtctttatttcctttacccatttccaaagctctacaaacaccgaaacgttggactggtttaaagccgtcaatcatattaggaatggctcggttttcaaccgtatacattgcataggccagggcttcgttgtcaataatgctttttaaatcacgagttgttaattccatagcaatcctctttaaattgatttatcaatctagtataactaatattatcatatcccataggaataataacttttttaaaggctttatcacccggtttatttaatttaatccataaattgtaaagcgtattataattttcccaatggttaccttttctaaatgctttctttaatgctttagaatgtcgttctttaactttagggtccttaaaagcctttttaacagaatcggataactttttaactgattccaggttttgccacgtgtcttttgctcttaaagaagcttctaatctttcttcttcgccccaccattcttttacagatttcgataatttatctcttttttcttgagagctccaaacagatttagaattcaacgatatttttagtctaacttcaggtgaattcatggcctctaaatggttctttacatattccgggttcttaaaaagagctttagtagcatcagactttttctttctggttttatctgtattggcttgtctttttattcctttggagtgcgattctttatttattgggtctgcccaataaattctcattttttcagatagaattttagaagccttttctttagctatagaatatcctatagaattcaaccttattcctttaggactgcctgaagtataaaatgaccaatatgctaaataaagaccattagaattgggataaatctttgttaatatccaatgggctatataatgctctctagcgcttaaaagaactttattttcaggagtatcggggcctcctatgcattccgggattatatgatgaacttccgaataaaaatccaatttgccttttttgagccctcttcctttacccctatcaattattgctttgtacaaattatgataattcatttataattttaccatactagtgaatgaatagccataataacatcggaaataaaaagcacaacttggataagtccgaacattactccataatacagtgctactaataatgcagcaagggctactgagtagcccaagattttcttaatcatttttaatcatcttaagtaaaccgacagaagtagaaagaatccagccaataaacagaaaacttaagaataccggaccaggggtccacacacctaaaaagaagcaaaccgaacagacaatagccataataagctcaataaaaactagaataaccatattttcctcattagcgtccgaagacgcctttagttttaagattgttacgatagaactgcatcacatgttcgttatggaaattgctcattagtacgcctgcagaatgaatttaaagttatcagccaacatgcggttcatttcttccagtgtctggaggtcggaactatgattacgagtgaaagccattgcaatttgacccttaccaaaacctgtagtcagaggtttcatcttagaagccggtacataaagaacttcatacacaacaccgttcactgccatagtgcgagctgattgagaacgtttcttacgaatgttagccacgataccgtcgagcccttgggccgaacgttgattaccgacataaaaacgagccgctacgacacgagaatcagctccgcctttaacaaagaagtagaagcctggctgagcagagatttctttagaaggtttaccattttggtattcaccgttcttaacataagcaacagtagtagcaccagcagacagaacgttacggcgagtcatataagtattcatatcaatttcctcagtagattaatgttttgttatccagtcaacgagaaccattataacatgattctcgaggttgtaaactatttttgtagctgttctaaaataaatccgctggtgtaaaggcttgcattatacaggcggtcaagagataacgaatccaatccataagcttcacgaattgcattgataacactttcataacttgtataataaacgtcacgataatcgcggtccatagtcatgcggaacttaataaatttgtagaaaccagtttcagggtcctgatagaatgcaaattctgcagacgctaaatttttaaggttaacagcttttgtgtcgcctgaataacttaaatcaaatgtttctgacatgctaatctgtttaaagaacataatgttgcgattaccaaaaaataatttagacataatattttccttattcagcgtcaacagaaatagccatcagttcatcaacagtaaggcattgcacactagggcctacacaaaaacgcttagttgaatcataaaggtctgtagcattaacaggttgtaattcggtcccaacttgcaaaggagaaatgcgaatcagttgttggccattatgcaatacaaagctctcgccgactaccacatctttaaaaagtttcataatattttcctcagaagttaaagaatacacgtacatggtcaatcataaaaacgattgggaaaatgctcaataccattaacaacacaaacatgttccaaattgctttaagtaagtttttcataatcatctccattagttgataggtctataatatcatgattaatggagatgtatactgatttatgccaatttccacaacaataaactaaaacacacgcaaatcactgggatacaggccatccaaataaggcaccacgttttgctactcaaaacaccacctcttttatctcaatcaatcccctgtacaatgccgtgcggaggtcataaagaatatctatgccgtcaacattatccagttttccatcaataagcttttctaaatcttcctttgatgcgattaagggacggagaaatttacattcagaaagagataactctgtagtaacatcatcaccttcacctgatgcatcatacatagcggcaacaaccatacctgtaactttgtgtttagcgtaatataatttgatatccattttgttctcctcattagttgataggaagatagtaacaccatccatggcgtatgtaaacacttattttaaaaaattataaggcgagataccagccgttgtaattgctcttacggactagctttgtgatggcttctctgtcaccagagaacttaggagtgaacaggacatctcctgcctcatttactgaagtgtcgaatatgattatacagtctgcaactttatgattcaagagcggacccaggttaatccctgttccataagggaagtcaccagagtatcctgtagtacaggaaatccacttagaatctgattgatgggtcttaacctctacacggagtccacaatacataggatgagctaaaacatcccatgcataggtataagggtcgtcatggtcttccagaccactgttaacatatcctttcaaccaatcggcaaccatgtactcggcgtacgttgcaatgacacaccgagtcaatacttctttcttatcttgggacgggtcttgacttaaggaatacaatacggtatccttaatcttgaccttcatttcgcctgttaaatcagatgtcttcagggtaaatgtcggcatcgctgccaatcggagtagtcccgggttcgtcttcaccataaatgcctcgaatatgaagttcaccgtaataaattcggtcgtcgggttctaaagtatcagaatctgctaaaggaaattcgccttcgaccacctcatcgcattctagaaaagcgtaatgaacatcacccgggtgtttaacgagcttagcacaataaacagtacctgctttatggaatccacgcaaattagaaatcttgatatcacgttcaccgacattcaggtaattaatcattttactcaccgaaataagaaatacgaacctctaaacaatgagcataagcgcccatcgcatccagttgtgcaatcagtaacccttgttgacggatatcaagagtttcaaaaacaccaccttcaataaaggtttctagtgcgttaattttaagaaccaactggtcgtattcttcaactacacgtgcttggtaacctaacataattcctcattaggaggccgaagcctccgttattgatttagtatttgtattcgtttgcgaactgttcggtgacgtcttctagaacttcataataacatacacgcattttagcatcaccgtaatcgaccggaatactaacaacatcacgtgggttaactttacatgaaaccactttacagcttgagttaccaaaatgaccgatataactacgagagcaaacgtgcagaccacttgaacaggttacttcatcatcgtcatttacacgagaacgaggcattttaaccggtttgcctggtgagttatcaaacgtaccggtacggcagtcggtgtaatcggagttaaccaccttccacgtaataaagtgaccatcttcagtaattttgatgtcgtttgccaccaagaagtcgaacaaacgttgtacagctttttcgcttgggttttctaacaggttctcaaggaacggcaggtagaattcgaagtcttcaccgttttccattgaagtgataatacggtcaatcaaccctgaacgcaattcaatgccttggtaaaccagacgtccaccttcaatacgaacgttgcctttaacaaaggccttaacggcttctttaatggaaatcagtttaatcgcgtcatcgaaacgagattctttaagagcctgtacgatggcatcaaaatgtttgttcttattagtagtgttccatactgtacgaccttcagtgatggatacaaatttagtgctcgcgttccaaataatttccggacgagagccgccaatagtaacttcaacgggaacttcacgaggctcgttaggaactgttactttgatatttccggtaataactacctgggcctgtccagctcctttagcatttttcaggactttacggattgtatcaactgatacactgtaccagtcagccaactcattctgagtataattaccagaaatatataacttaacgatttcaacttgctcagcggaggtcaaacacttaatattgtacataatatttccttagattaagccgcttccacggctttcatgaatttaacaatttgagctacagaagcctcggtaatggatgttccacgacgatacatgtagtccgaaactaaatggtaatcagattcaaactgtacagtcattttatcattgttgcttgaagcattatcagtcaacttaaaaaaagtattgttacaaattttcttgataacggaaagcttatcatcagtgatataaccatggaaattcatataacggaatatatcatagaaattactcagacgagtatatgcttcagttaccggcttatcactgaaatacttggtcatgaaattaagctgagggaacttagcaatgatttcaaggtaataccgagctcgagtattgctaccaaggtagtcatcaacatctaccgcgtctaaggcttcggcataagcttctaatgtagcttccatcaagcattcgcattggcctaactttttaatctttttggcaatctgagggcgaatgatatggaattcggtagcaccaatcaaattagccatacgacacatggtagtggtattgatgtcaaagataccataagcttcatccattcccataatatcagaacgactgccaaacagaacataacctgtaatttcttctgcttcggcagcagtcaaatacatggtctcttgttgccagcgcccgtctttaatgaaccaacgataagcactcggtgttttaggacgcggttctgatgaacggacagtaaccggaatccatggcttaacaattttattcagttcagagactttataaaaatgaattgtgtcacctttaaaaagttctttaaccttttcaagttgttgcatttgcaacattgaatttgggtcgacaaaaataaggtcagttccgtatttaggaatattgttctctttaacaattttcttagccgaagcactgttgtccattgccagagcccaaagacctcgaactaatggcacacgacctttttcatcatcataaacaacatggatttctttcttattaatgcctaataaattactaagtcctgctaccgaagaagtattaccacttgacttaattcgtttcaaacgtgggtctgaaacgacttcgtaaaccacacctaaattaataaggtcgttttgaagggtataacgctggtataatttctcatatgtcaatttttctgtagtaaacaggctagttccaccttttttggtaagatagtcacgagcactgtaaccaaggttagaaaggtcacgataaacatggcgtggattatcagattcaacccattcctgtgtatcgtttttaaagaccactgcatccagtgcttcgatacgggttgcaatattttccatcgtacgtttatcaagagacaacacttcacgagacggagcaatatccagtgaacccatagggaacttaatataaactacatcatggcgagtacgcatccatgtgcctttattataggcagaatccaatggataaacaataccaccataaactgcataaagtcctgaacgttcgaagctgccataatttgtagtggttacaggatggtaatcgtcaaattcagggaaataatcaacttcaacaccgtctacatcaccaagaccaatgaaaggccgcatgatataacgaacttcagtttcaaacttacggaaatcttcttcatcaacaggaaccgtgatttcgatacctgttttatcacctggctgcataggttctacgaaagtaggtttaatctgcgggccatcaccatccatatatgctacataaccgcgaacttcgccattgtgccatgaggtgatattaaacgtttcggtataactgaacggagattttgaaccaaggccaaagccaccgatgaaatcgttagaagccgttttggatgatgcgaaataagagttgtacaaacctgtttcgttttcatcaccacgaatttggaaatcactcatacccggaccgaaatcacgacatacaaagcgagggtctagtttaccaggaacctgtactttccaacgttctttattaccatttagaatatgggcatcaatcatgttggtaattagttcacgaactacggcacgtactttattactataaaggtctgatgacaaaattttaaagaccttaggcgatgcctgaatagtaaagcctgtggacttagcaccattaccaatgatttgttctttttcggtttcaataatcatatttttctcaattcaggttacgtttaaaaatgtctgccacttcaaggagctcgtccttagtagcgatgtcgttgagtattttatatctgatttctttaaagcgttctttaaaatcctcagccgcattgatatcaaaaaatcgttggattaaccggaattctttatggacggctttatcgaacaaatcaatattcactttaaagtttgtcatttttaactacctcatgttgaacatattctctggtagaacctagttcagccagaattcttctcatagaacccattgtacttttgtgctctctgtggcgatacattatctctaaaaccttttcctggacaacaggagagagcgcctggttatctttaatctttaaggcaatagattttacagccttaaggtattcaagtcccttaccgcttgtagtcactactccttcgtccttacagttacgaatggctgtttccataaaggatagagccaggttgtcagtgttcactatactgttatcttgcataatcatattctcacctctaaataatcctatcataaccacaggtctttgtaaaccccgaaaagggcccgaaggcccttattagtttagttacttgaatcgaccttatagacttgtccgcgggtttggtaaacttcgccgtcccatgtctcgactgtaatagtcacgtattctgcaaactgaggtctagtatcagtccagatataaccgtattcaccggtgacgagcgtaacccagtactttctcataaagtctccttttgtatggcaccaattagtaccatacatatttattacgacatccaggccttacggagttgagggtcattaccaaggagcatttcgaactgttctttccaatcttcaggcaattgaacgacatcaaatttagggtcttgaatcattcgacggtattcagccttctcaagagaacccagtcctttgatataacgaatggagtgttttggtagagagtccttagctttggtataactaggcacatcatagaaccattcctgttctttaccaacctgagcaataatcaccggagttttacagaaccgtactcggccttgttcgaacaattcgggccattgactaaagaaggctagcaatgatggataaatcgaaccagtaccatccacatcggcatcggtcataatagcaatattacgatagttggttttctctgcgggttcaccaataaccaatccagtgattgcacagatatcaaatagttccttgttcttcatgatatctgttgctgtcattccccaggtattcataaccttaccacgcaatgggtaaccaccttgaaggtctttattacgaacttcaatgaaaggacccatagcggaatcaccttcggttaggaacagggttgtatcagcatctttgccgtataggttagctttaatatgcttatggaccttggctttagaagctttcttagcggctttagtttcggcagccttttcagctgctaatttacgtgctaaagcagcttcaacgataggcataatcaacccatcaactttaagaatggcttgagcaattttcttagcatcaatttggatatgattgcgaatctcaccaaaaggagaggtcaaacgttctttagtctgtgaatcaaaacgcatgttgctcatatcacgaatgaacatcaccatcgtaaggcattctttaacacgagctttagttacttcaattccacggtatttctttttaatgcctggcagaaggtgttcacaaatatcatcgaatacacattcaacgtggtggccaccattcttggtgtggatattgtttacataagtcagttgacggaatccatccggagaaggagtaaatgccatcgaaacattatcggtttcttggattacaaagtcttcaccaaattgcttagcatactttttaaagttgccatctacttttttaccattaaaagtaaattgaatatcaggataaactacggccagagtttgcaatcggtctaatgtaatatccagataaatttgtgacaggctattttcttcgaaatgattaaagtctggggtgaatataaccgaagtacccttacctttagatttcttagtagaccaacctttgttttccattccgtttgaacagttaacagtaatctcattctcaccatcagaggtgatgcctgtgaacaaaacagagaagatattagttaaactactaccgacaccattcatgccgcctgtcttacgctcagcgtcatctccaaagttaccacctgcctttggaatagtccatgcagctacaggacctggaatctgttcaccattttggtcggtgaccattgcttgtggaataccacgaccattatcagaaactgaaacctggttattcttaatttgaacatcaattttatttgcgaatttaaaattggtacgaatagcttcatcgacagagttatcaatgatttcatcaattaatttaaccagtccaggaacatagtttacctgtgtaaaattaccaaacaggaatcgaccgtgagcttcattagcacttgagccaatatacatcccactacgttttttgatatgttcaatgtcggacagtactttaatttcattcttaatcatgttatttcctcatgtagtaggagaatattatcccatttcacttaaagcataaaagggccgaagcccttaatcaaatcgaatggtcgactttttaaagaataatccagaacaaacagttccttcaacccttttacctgtcggacccacagcaataaagcctgtacgttggaaatcatcttcagagcagccaaataggttgtatcctgtgatttggatttgttcgtagccatttgcatccaatacacgggtagcattatcggcatcagtacacccgaccaacgaaacggctaatacaagagctgcaatagaacgattaatatatttcataatttctcacttagtcagcaggtcgtaaaaaccgccattaacatgtttaggagccgagactaaccgaacagccagccgatggcaatcaggacaaacatcattatctctttcagagattttcttgattttttcgtattcttttgcacagtcttcagattggcatttgtaatcataaagtggcatattattccttaaagtgagctttcaacatctggaaaactgaccaggcttcagaattattagagatagtgattttagttaaaggaaaatcactcggttcgaatggagctgcatcttcagacgtgtcttcgtcttcagagaaaccatcttcggcccattcgtcttcactgtcaactacaaccatttccgtaaagaatttacgctcgcttggatataaaaccatatcagtgttatcaccataagccaagtccacgttcatcacataacctgccgctaatctaacagggcaaaaaccttcagaattgacaatgatatctgctatagaagaattattaggattcctaatattatgggaattcagcttacggaattcagcttctgccgcatcatctttaaaatagtaccatttacctttttcaaattcaagttcttgattaagcattataagtttccttccagaagtcggtgccttcagcagtgatttcacggaacaccgcatagatagggttttcatcaccttggttttcgtatacataaaccgacgataaatgagaaaacgtatcagaatgttccttttgaaccacgattaaatcagggttgaacagaacatcttcaaattcttcacgagtcgagttcacagtaactttagccattttattttcctctcatttgttgatagggtaatagtatcacactactaccctgttgtatactgtttttaaactttatgcaaaatgaatatcagcgtactcaacaataaaactttcaggaactactttaaaggtgccaaggaacacgatgttatacagcttaacaccttcttcaacccattggtctgtgatgtaaccggacatactagtggtttcataagtcggaccatacttgcaattgtattcaaacggtttaggtgaaacgaaaaagacacctttacctaatttccatttgaaatcaacactaacatgagattggtcaatagtttcaacgtcttgagctactacgccacggatatcattgctttcacatacatacccatcatgggattcaacttcttcaactacaggagcgatgtgtccagtgaattcagttgattccaggaatttaggatgcacataagcgaattgagtttcagtctggccatttttaggaataatacgcactttaacttctttaattccacctactaaattagtacgaataccagcaacttcaacaaaacgacccgcggcttttgagcgagattctttggatacacgaacaatttcaccgatagtaatcataattttctctcttggttaataagtttattctccatgagagccattataacatggctctcgataaagtaaactactaattcaatacattaaccactgcactacgaggtactacgctaaaatcaccagcatgtacaacgttcagcagctcaacaccgtcttcaacccactggtctgttacccaaccacagataggattatcaaaaggacgacggatagacacagcagcacacagaaggtcggtagggtcttgttcttcaacttcttggaacaggatgaactcatcttcataaaccaagattttctctattttgttattatctaatcgacggccgtggatgacgtaagatttagtaaaccagtcacttttggtaaattcttcaacaataaattcgccttcgccaaaaacctcagtcagagttttatggccagaaatcaaggccttagttttaatttcaggttcaaccagtttgtaggttttgccgatttcgatagtctgagtattcatagcaggttccttaatttccagtggtttaacagggcatacataagtgcttaaaacatcaaaatcaatcagtttagctgccggattcggggtgtatttagggttgtaattaaatttcatattgttctcaattcaataaaatctacgagttcagcatgggatttgcggaacattacttggcggccaccaatgacaacctcatcttcagggatttcgtaaacggcaagatagaatcctttagaagataattcttcacgctcttcacgagtgaaccagcgcatcatatcatactcactggcaaaagcaaaatggtagagattaacaaaccaacctggaatataatcatcacagccttcataatcaggctggttccacttagttcgaatggttttattagaattttccaccaacaacttgtcttgacctggtagtggaatatttttattattggtatggtggtgtctaaaattaggtttgtcgaaacctacttctaataaccaaccttcgctccattcatcaaacgagcctctatacggtgttaattggcggcactgttggtgagtgattgctataacatcgctgttatctaagatactgaacgatgactccactcgataaattttcattttgttctcctcatgttgatagggtagataatatcatgtcatgaggagaagtaaacacttttatcgattttttatacttaatgggtcaggattctcagggacatcttccagacccaaggcgtatcgttgggcatatttcagcatcaagatatccttagcacagtcatggatggagtcatgagcaacaaagccgttcaatgttccgttaggcagaggacacatgctcaatccacgagttagtgaatatgcttcaatagctgtacggatgtcacgttggttccagaatttaaccggttctaatttactggtatcaatttcattctcaggaacaccttcagaacgataagcatcacggattaggtctactaagataggaaagtcaaaggacattccacggcaccacatctgagatttccattggtccacttcgtttttacggcagtattccaggaaattaccgagaccaatagaagtggacacatcaatttcagatggagccaggtttttacgcgcttcaggcccttgctctttccaccactgcaacgtgcttttagaaaacagtcgtttatcacgttgagaagcgaggtcaaatttaatacgaaggcctcgttgagtaagctcttcaaacgtttctacaacctctggattagggtcgtaagcaattacggctaggtcgataaccgctgcattttgagtagtggcaaaggtttcaaagtcaataattatatctttcatttaacgtacctcataaggtctcggatttggccaacggtgtagtcttcaatataaaccgaagagatattgtcgtccatcagattttgtactgcaataaaatcactttcaatctctttaagagagttcaggacagtatgggccttttgcctaatgctgatattattttggttgactttaataatatgttcggtttcgaatttcaacttataaaattggtctttagttactttaatcatattttcctcaaacgtagtaggcgtcagtacgagcacgagtaatactaacataagccagctgtgaagctaaattcgcatcagccatatgcatgcatggagtatagatgaaactgttttggactgtaagtccttgggatttatgaacagtgctcacaggaagagctcgaaccttactgaacattcgcttggctttccagaaatcagcccacttaggtttcttaccactaccacgcatggctttgtactctgtagcaaccttagccaagaaataatggaacttctcaactgaagcctcatcgataacctttaaatgctctacatagtactcgtcgtcttcatcaacagattctacttgcaggtcccagtaattaatcatttgacgagtgcctacatccttagcagacaaaaacaacgaggtatggttcacatccagaatacgaaccatttgtccattattaaaaatggtttcagagaatttcttaccatcgtattcaagttccttcataaaaggctcttgcatcactaggatttcgcccttgatataaggtgcatcggtttcataaagctttttacgaataatgctattcagcttttcaaccgatttattggtataagcaaacatcctattctcaaacagggcatcagcatcttttacaatggaaaaataattcatcataaaatcttttaatgctgtttgggatttaaaaccatggacaccatgtccttcgaatacacaatctctaaaccacccaccattacggatttcagtagccacctcaatgataggagcattactacgcatcacttcagtcaaatgtaattgtttgatttttggatgtgtaaagaatggagacaactgagggctaccatcacttccaggttccactggctgtagctgagctctgtcgccaatccctaatacagtacaccatggtggcacggaggattcaataatcttaaacagcttaccgtcaatcatcgagccttcgtcaacaactagaacattacatttgctcaagtcaggagcttcgcgttgttcaaagatgtcctggtcttcgtacgtagtagggttaatttttagaattctatgaattgttgatgcttcttgacctgcgagtttcgacaatacctttttggccgcatgagtaggcgcagtcaaaataactccgagttcaccattcttgactagatggtcaagaataaatttggtaagggttgttttacctgtaccagcaggaccgttcaatgtaatccattcacccttacgtcgtttaatagcttcaatgatttctttaaaggccgtcctctggccgttgttcaagtcttcaaatgtaatcatgccaattttactcgcttaacatataaagtgtctaaaactaatttaagttctcgggctcgttcttcggtaggatatactgttttagtttcccacttatcaaaccaccattttctaggtgtgcacaccgtttcaaggcgtccaagccgaagatatctttttgttgacatttcataaacggatagagcggtatcggctccaatctttgtcgaatacaaagtcacttcaccggcctcttctaatggaatttcgtacccgtctttgtccttgtgaactaatacgtatgcatagtacatcacgttaacctctaatcagtgaaaaaattgaagcattcagcggaagaccttttttcaacttcattttgtcaataaaagaaaggtgttctaaacgctccagaccttgaataattttatcatacatatcgtaacgcgtttctgcttcagacaatttaaacttgacacgccaatcaggcccaccaattaaagatttaagacccttttccatagtacctattgaagcgttagaaccatggatacgggccttaaccgcgatgacagaaggggtattatcagtggctcctgatttaataaggtccttaagacgtttttcacgctttttaagacctctttgggtatctttaatatttttaactattttacgaattttataataattatctggggtaactttaaaactattaggcattttagaaccacctgaaatacgggacgctaaacgagtctgtgcacgtttcaattcatctaaagacaaatcagctcgcaacccgttgtacttaactttaaccgggattacattaccttcgatataacctatatcgttgttaaagcgttcaaacgaaatcttatctttatctgaattctcatcaaagcgctcgcctgaatatgcacacactttttgttcaagaagtctacgaacgtacttactagacaggttaaagtccttaccacgttttttggcagaggctttagtgtgttcgcgacgtttgtaaacctttaattcaaattcaggggtcatggtatttttctcatcttacggacgattagttgataggtgtctatagtatcatgttgcttgataaagtaaacacttttttgctttaaattttcgacggtataatgaatcaaggactttgcctttcaattaaaccgggtggttcagtaagaaagaacggaaagattccataatgtataatcttgccatccataaaccttctcaatagagtctacgcgcagcgtagttcccgcagggaacatcatctcatcctcatcattcactagttgtaagtttgaagttcgagttatttcaggatacggcccgttgaactcttcgggaggagcgccacaaatcattttaaagattgcttcctgataatcaaatgcaaagggggcatcgttaatacagaaaatatttttagttccgtaaaaattatatgaagcaaaattacgggcaatcttaaaatctttagagaagctcattaccctgtcaaattcaatagtagcgccgacacatcctaccgattcaaggtatttcaaagttttcttagaaattccacggtacagcttgtcaggcactacagaagtcagattcttacggataattttattcagagtttcttggatgcaatccggtttattttccatacacagccagagggtactctgttctaaatcagaatactgctggtcgatttcacactgaatgttttcacggaaatcatcgcacttaacattgtcatagaactctgataatctgtggttagggtataacatattattctcctcagttgatagaaagatagtaccacaagcttccttgcctgtaaactaaaaatccaacatttttaaatgaattgttttgtactcgatttcgtacgggtcccttttgatagtttcgatttccacaatctcaaatcgtgattggctggagaccatgaactcacattcagtttcgaccatatcgtagaggtctatacgggtttcatctatttcaagctcatctacattccctgcaagaacaaggtcgatagcatggttatagtagtcgaaaatgaacggtgcattcctgagacttaaaatggttctggttccatattcccatgcccctgcgaactgacgagcctgtgagtattgtgtactaaaagaagtaacccggccaggagaccactggcacccaacagaaagaacttcaagttgctcaagttccatagcggtaatcccacgataaagctctaccggaaccgctgaagtaacatgcttacgaactagcttatcaaggtcgtaatggaagttagggtcctttttagcatctagacatttttctaaaagattctgttcgtgttttgagaatttggaattgattcggtcttgataaagacatttttgttcgatgttcatatgacctccagtgatttagaggtcattataacatgaagggaggaggtgtaaaactttattttacccaaggggcccatggaggagggtctaagtaataagaagctaggtcactaagaacatctttaggcaacttaaaaccatgcttctgtataatcatatcaagttcgttgacaaggtcaacaggcggctcctgagttgtttcaggctcagggtccggaatgacaaacatatcaaataagtccattagtaaccaccgataggaccgtactcgtacatacgagctcgtaccttagcatcacgaatagcgtcttcagtcatggtaaagcgcaatccaatatcaaagtgcttccaaatctgacgttcaacttcaataaggtcttcggtagcggaaataagataagtacgacctttaagacgttcgttggacattctatcggtatctttatagaaaatgtccattgttccttcgccatacgggtccggatggcgataacccttgatatgtaatgcttcagccaggctaaaaggacaatcttcagcaacatcaacatttttgttatggtaagccttcatcataatattttctggaagcttaatatcttttaatcgtgtttctaactgggttatagaattcgtaccattgtcgacaaagataagacacactgtagcatcataaggacgtgtctgtccagatgaatcacgtacatggaattctagttcataaactttcattatgatttcctcttcttagtttacctactaaaggaccatccggaattttattttcttggatgtatttctcgttttctttcatcattttactaccaattttaagaagcaaatccagtgcctctttagcttgtttttcggcctcttcagtagtcatgatttatccccatagatgtcacgcataattctaagagcttcgcgttctaatttcttttcgcgttcttcacggatacctttaagaatccattcttcggactcgcgtttcatttctgcattagcttggtccaaccacccgtcatcaagataatcaccaggacggtccagccaatctttaagccatgataaaggtttcattaatcacacgagccggacgatgagtcacagcttcctgagtcataagacgaataagaagaatcaccagtccaagaactgacagcagccgcaaccataataggagtagtatcaatatggcttgtgcgacgagcttctagatgctctttaaactttttagaattcaaaggaagggcacccgggcctacattacctgctttttcaggttgacggataacttcttccatcataccatcgcccacataaacatattccttcagacctgagataggaaccaccccttcaccaggtttggtcttgaaaaaattcttaagccaacgaatcataggaaacctcgtttaaattcaactttatcgatatcatcagtctcgtgacggatttcggcattaaattcgatagaaccgtcttcatgcatcataaatgaatggacaataacttcggtataccaaggagtataaaagtactttttcaatacatgattagcgataatttcatctaaagttttatttggtttaatccaacgatttaacatagcattctcctctataagataagaccatcttaacataaccttcttagaaagtaaacccttaaaaccaaaaaaggaacccgaaggttccttataattaaactactggggtaggcgtaaacatcgccgcgttcttagttcgccaatcggctgcatcagttactacagtagtgtatgccgccttttcagaaggaaatgtctgatagtgtgcattcgcaatacgatgctcgtttgaatagatttcaaacgggacagatacttcaacacctttaacttctttaccttcaccagccggatgcgtaaaggttttaatattaacgaaaccacccataattaactcctttgttgtttaattacaggtgtatttataacttaataacctcggtcctggcgagcaaagttctcggcatttttcaggtaatacagtttaaagatttcttcagcagtcagtccaagaccttggaacatattcagaacaaagtgcagaatatcaatcatttcgaatttaatttcgagctggtcttcaggagacaaatcgttaatcagggtttcacgacgttcagcatgttgagctttccaaggcttccatacagcgctcgcatctttttcgccattgctcatgccaccaagagaagtcagaagttcgcggaattcatcatcaatataatctttctgattgcgcaaccaatcaacaacttcacctgcagtagccaagtcatcaggatgacggttatattcaggtttatctttagccaaacggacttgtaatgatttctgcatatcaagcataacctgcagagggtctttatcttcgtgaatcagagcattaaaataagcttcctcagctttatcaacaccagcaataagttgtgagcattcgttaaagtgtgccattatattttttccttttcaattcattagtaagttagataattataaactgttagattaaagcgaataaatattattttaacaggaggataacatgggcagtattttttaccaaatctggaaattggccgaaaagaaagacaagaaaatgatgttaggttttcttgcgctagacgtattcctttggaatcttctagtagtccctgtagccgctagccaagggataattttaccagcggttacaatggaacacgtattaagcataattggattctttagcggagttcctgcctaaattttagaatattttgaaagtctcatttttgccattaaaccttgggctatattagctttcatatatgccagtacatcatttatatcagctttatctttcataatcatatcatttatatctttagaaggccatggagccttgtcccagaatagaaccctttcgccagcatcaactaatcgttgcatacgcttaattgtgtcaggatggcggggttcattgtccattacccaggcacgagtttctttacatggaaccatagccaagtccaacgacccgccagtaattgctattgcattcggaacaaacaaagagtcaatagggccttccattacccacaccaactgacgttcgtcaactgtatccattccatatatttttgtagcttggtcatgagcttttattgtaatatatttttgtggagcatctttacgtaaggctcgaccctgaaaactttcaatttgtttattcttattgaaaattggaataaccaaacgaggctcaggcatttctttagaataggtccctggattgacagagttcaccaatgccggccattctttagtaaaccacagccggttccatttgttttcaggaatgcaacgtaacgtcacatatttgataataggatggtcctttggcattctatccagacgttcacagaaattaagcttttcgatgacaggcatcttggctttaatcttttctgatatctccaccttaggtgcagcttgtctcccgaacgattgctctttatgtttctcaagaatatattctcgatataaatcaggctcatattcgtatagatacttcttaattcctgctgaatagtcacagttaaaacagtgcagcattacggagccgtcattggccggataggcccaaaaacgagctttgttctcatcttttagggagtcgccacatacacgacaacgacagtttaatttaaaatcactaccagttacttgtctgaatttaggttgataattcaaggcacgtacagcaaattctctatcgacatatgacattatttttccttgggctctaaattaatagagccattatatcattcgttttcggatttttctttacgctttttagatgggatttgttcaggccctttgttgacgactgcgcctgaggtagttccggaggcaatattagatgggtttccacctgcatcgcctgcgaccatatcttcgttcataacttctttaaaagatttcataggctcctggccttatttatattacgaaaatagctttatcaccatttgcatcagtgacttcgtacgtatcttcgtggtaaagtggaataatccaagtcacaccatcaccggcaataatatggatagcttcttggtcctttgatacgatttcatactcttcgaataattcgaatacagaaatcttagagcccgtacacattgcactcatattgttcccttctctcaatcagttggcgatgggcctttttaagtttacgaagctggcgcttagtcggccgtgcgacataagcttgagtagttactcgaccaaaaacaccgtacttaggtgaaggagaatcgataaagacttcccactgacaagagtaactatacacggctttagagaattgagttaagacaaacatattaacctcgattcataaaggcattaaaaatctggtcatctattgaataaaccggagcttccagaattttcaacagactgtttttgatatacttgctagggatgtccatattaacgcggtcgttcaattcgttgtctgggaggatgtctttaaattcgaatccatcaaactcaaccttgtcaggaataccttcggcgaaaaaataaaccaattggtgcattgtattgcgagaaaataatttagacctcaccgcaataagttcttgccaatggtttaattctctgttaagaagtttatgagccattgtaattcgatcatcgctatcaacaagaaaataacctaggtattggtggtcgtcgctccaaaacatcctgtatgcttgtgcatttggatttttacaacaaagttttttgataactaaatttctgttaatcttattcacctgtcacctctttaacgatatttttgttatcgaaattggcatcacaatacaaaacatagttatattgcataacaccacctgaagctaattggtctgacacttctttagccatatcagggcggtcacgtttagtgatgttcatgatatcagcataaatctgatgttcgactgattcttggtctgcagtcatagaccattcacaaaggtctttatccaatccggcagttaccggagctgtgccacatgatgctacggtaagaattgctgcgattaataactttttcatttcaatctcctcgttagttgataggtccatagtatcactaccatagaccgttgtaaactttattttaatgaatcttccaaagaaattttacggaatttacgttttgtctgacgaatctgacgcttagtgggcttcacaggaaattcgaagaactctacgtattcttgttcataatcgttgcggcccactgaaagaactagttcccagttgtttacggtacgttggataaacatattatgcttaccgaaagatttattccaaaaagagctaggagttggtttcattagtacgatattcatttattcctcgccttcatgtttatgagcaatttcttcgaattcgctgtcacagtctaaacaggttgcgttgtcccaagcatcaaataccgcttggtcttcatagactgaacaaccacatactacacattcaaattcttccatttagatttcctcaatgcgagcatcatgttcataaacttctacgtcgtcgacataggccttgactagaatactattgacttcagcgaattgggtagccacccacacaatatcgttttcacgcactgaagcttctttggtagcggtatcaccgttggcgaaatggccgacaaattttactttaattgattcagacatttagatttcctcgcagaaggcccattcagcatgataaaccgtagcgcctttagtatcatttaaacaaaccacatccaccggagcaattacacgataaagacggggttctcctcccactgaacgagctgcacgtccagcataaatcttagccaaaccgatatcttcagtaaagaacacacgatttaggtttttcttacgaccggtttcagacagaactcctgtttcctcaggaggacaaagcatattaccgatattagcgacactacaacttccatggtaatacactttatattctgctttacagtcgatggttttcattttgttctccaagttgataggtctatagtatcacgcctacaggagatgtaaacccttaaaaacaaaaaaggagccgaagctccttaaaatttgatagatgctgctaaatcgtccaaatcacttctattaacacgcgtctgtcgattgacctcggcctggcgattcatctcacctgtagcctcacgaacagtgttcactgggcctgggttggaatcatcttcaacttcgtaccaacgttgatttcctttcttaacgccaatcttaaatttgttgtagtagctcttatcgccataacgagatttaagctgcttaaccatctgcatacccatctgagcgaactcttctgtctcgaccacacccaacatgaagtctgcagtatgtgcaataccaaaggattcagcaatatcggccatatcgatttcggctgcaacgttcgcaccacgagtagtctgggctgcagtccacaacagtaatttcttctctactgcaagtccacgtagttcttcagcaaccatcttaatcaatccgtaactgttttcagagaaaactttcgtacgagacgatgcacagatagccaagtagtcaacgataacaacctgagggacaaagttttgtttgagcttgtattcgtttaataatgcacggaatgtatcggcattagcaccgccagtagggtactgtttaatctttaaacgacccaaggtagcagttgaacgccatttatccatcttagctttatattcaggccacgagacgtgaccatcatcgatatcatccagcgacacgtccagaaggttggcatcgatacgcttagcacatacttcctctgccatctccatggagatataaagaacatcgtaaccagattgaaggtaatcagcagccaatgaacaaagaccaagagacttacctacgtttgttcctgccaacaatacgttttcagtaccaaactcagcaccacctttggtaatcttattcagaatattaagacggaacggaaccttacgtgctttatcagaataacttttgaaacgttcttcatagtcatccatccagtcatgacctaattcagaatcgaaacaaatcgataatgcatcacgcatgatatctggaatagcaccaatacctggaagttttctattttgttgctcaaccggaaggtcggcattagtttggatttcaatgatttttgaagttgcattatacatcgctgctttctgaacgtatttctccgtctctttaaccaaccattcttggtcttcaggtccggcattcagcgaacttaaaagctctttagcgccttggtgttcaacttctgaaagcgtactgttatctaatgcaatgctcaatgcgttcttagaaggcactgcattatattcattgacatgttttttaatttctttgaaaagggtctttgcaggaccctggtcaaaataagaatcattcatataaggccagaccttagtgaaataatcactattgcctagcagttgagccaaaatagtttctaccacttccaccacctcttagatttaattttatccagttcttcttgtatttgcattgtaacacatttttctacatgaagcgccagctcttcttttcggtcttcggaaggtgttccgaaatcaaccgacacttttccatctttctcaataacaatattcatcacataaacgatgtgagcagtgccatcgggtaaagtaagcataatttcctgcttaaccgatcccattgacttacggattatatctaatgatttctcataataacgagggtcactaggaccctcttcggtatctttaacgaaattatctaaatcagataaatcagtcatctaaatccatctcttccaaatcgttttcgatatcagcggcgctttgggcattaccacctaatttaacagcaacgttcttagagacacgagagttaataaggtcgttcactgcatcgtcaacttctttaatagaattaattgcaccgagcttatacttattctcgattgcttcacggaacggggcatgtttaaacagcggtccccagaactcgacacaatcggtagctttagcacgccatgctttttcttcttgaaccatttcgcctgtggtttcgtcaaggaatgcacgattataccagccagctttaggtttcacgacaaagccaatatcagtagccatttcaagcaatccactgaatgggtcgataccgccttcgaagttcactgtaatcgggaacgttgatttctctttaaccgtacgagatttctcggccttcagtgtgaagtcataaccagtgagctcagtaccatctttaacctgacgtttagagataaagaacacggtagaagcagagtacagaataccagtaccaccacccataatctctttagggtacattccaccaatttccatagccgtgtggttaattgctacacaagggatatctttgatagtcagataaggtgttacgatacggaacagagatttcagtgacttagcacgggtcatatcacctacaactttctcgttcaaagcatcttcggtttctttcttagaagcagtgttaccgatggagtcgataaagataataaccttttcgccacgagtaatttcttctaattggttggtcatatcaactttaagctgttcgactgactggattggtgtatgaaccacacgttctaaatcaacacccatcgaacggaaataagattctgaagcaccaaactcagagtcatagaacaaacaaattgcgtctggatatttcttcatatatgccgcaaccatggtaagtccaaacaacgttttaaagtgtttagatggagcagcaaagattgtcaaacctgattgtaagcctgcattcaacgcaccgcccaatgcaatattcagcatagggatacgagtaggaacttcgtcacgaccattaaacaatttagatttggtcaggtcggcggtcattttagaagtagaagctttaatcaaacgggattttaaatcagacattatatttttccataggcatcattatattttactcacgttttaagatagggtaattatatcacttcacatttacagcgttaaaggaccacgtcctcataacttggcatttcgtgctcagaatggatgtgggcaccgaaataaatgaattcagccagaccaggatggaatactaaaccgggattctcatgataaatgatatgaggtcttgatttcagaatctgataatattcaaccttactcggtttgaatttaataatctctacatcaggacgatagtcttcacgcttaaatgaatcattcggatcggtgatataaaggcgagaaccttcagccgcagcttggtctacaactctttcgaattgataacatttatcagagatacggaatggatggaaaataccatcaattttaataggcgctaggccttcagagtaacgctcaattactgccggattaattaccttttggtctacaaaaatcttatcagaggacgcacctcgtgacaccaggacgtctttctggcattgattcaggactgtggtataaatcgaacgttcaactgaggacacgtcggtatcaataaactcgtcgatataataacgaggaacttcagggtccattgtaatgttaaagttgaattgtacagtctgagtgccatcataacctgtgatatcggttaccaatcctgagcagtcatagtattcgattaacgaatcaacaacgaactcgttttcagaccaaaaatgtttacgagtttcataagcattttctttataccaaagcggtacaaaattcagttcaggaaataattcaatgcattctttgatatcgctcgaatttctaggataagccagataatcacctgggcaagcacggtttaaatggagttgaaaattaccgtccttaaggacggcatattcacctgtttcgtaactacgcatactgaaaataggaacgataaacaaactcatttcaggaatcctcgaacgtagtcaaaatcacgttcaaatacgtgtgcactaaccatagtatgggaatacgtacccagaccaacaccacactgttcagcaataaaggccatcagtttaccctgcagatagaaatccagctgcataacaatagcacagttctgtgaacgcatatgggtatgtgcataaagacgtccatcacgaatataatatgtcactgaatcagtacatggatattctaaggattcgtcagaatcaaggagggcttgatcttgttcttggagaatttggaacacaactcgtcttgagttaggcttctctttaagctctttaagtaaggctgggagttgggccacaattctaggtccatagaaagtgttgaagtttgcaggcaatacgtcacttttcggcttatcaatgaacttagcaacattagggtattccttaaatgcttcggcggcgtcagtaccaccagaaatcataaacttccagaaagattcggcataatcatagttgatgcgattaatacgagggtcggtgaatttataggtgcttgcatccagtacttctaccgaagcagaaccaatttcataacaacggccgatacgagaatcaactgcaaactgtggagcttccaggatttcttcgttcatttgcttaaacgcgttttcaaaactaacagcggtaatgtgtttcatttattcaccttattttcaatatattcattcagacgttttaattctaccatatcgacgttaagcaagttattatggccgtcgtgatttaagattttaaacacgttttcaaaacatgtttcgtattggcggatagttaggttgaactcatctttggttaatttaataaggtcatcttcaaagtctttatccagtggattacgggttaaaataacctcaataatattgaattcagatttaaaccttttccaatcttccagttctacataagggtccatttcaccacgaaggaatcctgagtaaacaatattactaggatatccacggtctaagatgtagacaaaattagggtctaaaaacttatacaacgtctcgactaaagccttgtcattatcagtccctatcgaaatgcacttaccattaatctttttagggaaatcaataagacgatatttcttatcagataaaagtgattcaattaaagtagacttcccggaattatccgggccgtcgataacaatgatttttggtttcacggatgatatgccttataggtttcaagagttccttcacgaaccatttctttaaagtggtcaggacggattgctcggtcatcgatgataaaagtataactcggcttatgtgtaagcagattgtgatatttcaatccaatcttttcaaggttcttaactaatgcaggaactacttcaaccaagattcgacctggaccgcatgaagtcataccacgggcagtgaacaaggtaatctcgcatccttcatcataaagcttattaatcatggacaccatttcggtgtccggtttaaagttttcgtaatcacggtcatcttgccagtgagtaatggtattatcgatatcaaaacacagatgcattaaattttcttccattgtttgtggagttcggtagaacctgtaggtttatattttacaccagtttcctggtcaagcaaaacccacttatcaggacaacgagtgataatttgagccgtgatagggtcgcgaacttcatcaacgaattcacctgtgataagcttacgcttacgaggatgccgcttcagcagcacactcagttgatatagcccattgtaataagcgcccagagctttcagagggttatttttaaagtaacctgccaatgccatccagataacagcaatccagagcttgtgcttaaatgtacacatcggaatatcatctaaaggcataatcttttcaatatcaacgaatacacgagttccgttacgagttaagccaccccatagagggtcagagttaaatttgtcataaccatcgatagaataaagcaccttagcttcatcataaatcgcagggcctttagaactattaccaaaataaccacgtgggtcgatgattttaatattaccttcgtccgacaacataatattactgtagtgcgggtcgccatgaataagttggtacggttctttatgttcagacagaatttctaaggcgtgacgaagaagtttttctgggtcgcctaccttgaagtcgttaacatgggtaataccctgtggagcaaagccttcaatcaatccggcaatagaagcattacgaataaggaccttgtccaatacttctttcttaacatcagaataccattgctcatcggacggattatcgatagttccaccgaacgaacgtaatgcactaataaccttataaaccattaggactttagtttctttagacataaacctgtaggcatctgccatggttcgaccaaagatacgttccattttaatgaattcgcctggagcaaagtctacaatgctaggaacgaattcggaatcaatagaattataccaattgatttctttagattggatttctttacccaattcgttagttggtactttaatagctagattctcggtgaactctaatttattaaattcacggttaatttcagaatcttcatgcgccttagccagtttcagtttgtcaccaacatcaactacaaagtctaacttacgttcagtcaaatggaccattgaatccaggttgtcagcaaggtcttcaccataattagaacggtcgaaacctgtccaattagccacctgatacaagccaactacgccaccaccggtgccaatttcacgcaagtacggttcttcaaatgtaaaacgacagtcagtcccataggtataacagtagtcgttatcccactcaactttatgaccttcaggaataatatcacaccagttaaacaagacattgtgcccaatgatatcttcggcaatgcaatcgatagcatgagccgaaccattggcaacatcaacgttacgaatagtgaatttaggcttatcactattaatcatgttaatggatttaatatagcctttaacgaggtcgttaaatttgctgtgaataaccagaataatttcatctgattgattactatacaaatcatacaaatgttttaatacagtatgttgtttgtagttaaccagtaccttcgggatttcgttggtaattggatacaaccgtgagccaagacccgcgcctaaaataacaacctttttcattatctgttcctcaagtgaatgtaggtacattatacactatttttaataaattggtattgcttaaatcttatctttaccgatttcaatacactgttctattgccgccggtactttggtcttgagcttatcgatttgtttcttataatcacgagctttaccgaagctctcggtttcgagcatttcgtaataacgagcctcgtggatggaaatctgtagattgatatggtttacgcacatcgcatacagtttctgctttttgtacaaatcatcttgacgcttcatttctgcctggtgtttggctagtaccgcttcacgcttggactcttgttcacgttggaattcgatttcttgttgagcatattttgcacagttattaccgcattgattattagctcgggtgtacacaagtccagaacctgcacggaatttcatttcgccatcgaattgtttctgttcagctgcgatacgagctttaccaacttcatcggccgaaactgtatcaccatattggaccgcgcaacctgataggagcatactcattgcgataattaactttttcataatatcctcaattaaaacagttatacttaatttgtgctataagaataatccatccaatgatgagtgtcggaatcattggcggaattgccactgcccaataaacggtaaaggcagccattataagaaataaaacaattattttcattgtttaacaataatgatttgtgcgtttgatttacgttcagcgacgatagcccagattaaagccactacccaaccaatcatcgtccagcctaacaggagattaaggaagaaaattcctacattactacgagtgcctcgcagaagagccagaatccatggtaaaaagtaaccgatgaacataataaccagagaaccgaatcctaaaacaccagcactaacgattaaagcttccattgtaatttcctcatgtagttgataggaaggatactaccacgttccttgtggtatgtaaacacttaaaagtcgaacatatcaaataatgttgcttttttctcgtagtcgattttagcagactcagtaaaaccggtcagaggtttgataaaggtcttttggaacagtacgttgtagtccatccaacggaggacttggtcacgaatctgaaccggaagttcaatacctgacggccatgccatacaagcttcaccaaacgggttgccttctttaagtggcagtacatataccttttcaccatcaacgatacgaggcatagtcaaatcacctgcagaagcacgcatgtaagctaagcaacctttgatgtggtatggacatttagaacccgggaatccgccttcattatatttctcgatgttgttagcactggatactgctgcaatgcttacataatcgagttcgttaaattccttattaaactgtttgaaatattcttgcaaagatgcctcgccttcctgaagcatacgacggatacattccttcagagctttctgaactgctttaggtgtacttgatttctgagtttcgagacccatgattttcaagtgtggttcagcataacgagtaccttccatgtcccaaacgttaagtgcataacgtttcttgcctgtccagaatccaccaaggcctttagaaccaagtggaggacctgcgatagcttctcggtccatgaacatcaagtgttgtttgttgttcatgtactcgcacatctcacggaagcccgcatcaatagccggttccatacgttcacgtgcaaatttatctaagaagtcaacccagtggttagtatcacggaatttgtcttcgcctactttattgatgattgcatccgccttaacataaatggagtcagtatcaccatagagcacgaacttctgattttcagtcttacacacgctattcagatattcgttaaccttacgttcaatccattggagggccatttgaccaaacaatgtgattgcagttgcgttcctgaggtcatagtaacggaaccatacgttaccaagtgcaccataaagggagttgataagcaacttacggttaatctgagcagtgttacctgcaacttcagtgagctcggctttcttcaacatttctcttaaagaaggcgctgacagtgctttaatctgggctttgatttcgtcagagaagtcaaaacgataatcgatatccagtggactatcaactgagagattaggattttccaatgcttctttaattaactcaccattacgttgagctgcaagcatgtaacctttatgttctttacgctgcaagaataccttggtgatttctgtcggaatcacaccttcacggtctttatagtacatcatgccgttaggagagcaactgtaggtgtcgctaggacgctgagcagttccggcaatatattcatgtatcggtgcgttagcgaatgtccctgcgatggtctctgggcttatattcacttgtcgaatgatactcggatacagagatgtaaggtcgaaactcattacatatttgtaagcgttaggaatcggttccttaacgaaagcaccaggataaggttggaccacgtgtgagcgagcttgtggaattaccttgccttgttctttaaggctattaaagataatagcgtcccaagtcttaattgggctgaacaccgactgaatctgcatcttggcataataacccatgtccaaactcagaagaatgaactgacgcttcatatcaatctgcactacacgatatacgtcgataatgttataggaaatatatcgttggtggttcgtctcacgtaacttggagattgggccatcatatttcaacttacctactttcaattcatattcagaaacataatccagagaataagaaggctggttggtgaagctgaattttttatagaggtcgatataatccagaacagagataccgaacaatgtaatgatttcacgagcaccgtacatgttctcaataactttaacacgagttttacgatgtgggcttaatcgcttagcagtgttctcaccgaacagatttttcagacggttataaacgtacggtacgtcaaacgactcaacgttccatccagtcaaaatcacaggagttttctgttgccagaaattcaagtactcaagcatcatttcttcttcagaattaaacggaagataaacgattttgtcaatgatttcttgtggaacttcgtcaccgccttcgtcttggagtttctcagcgattttaatcgaccactcttcgacagtaccataaggcgaaactaaaaggtcgaatacatagaatttatcgtcaatcgagtcgtagtgggtaatggcatcgataggatgtttagcctgagctggttcagggaatccatcaggagatgttacctcgatgtcgaagttagcaatacgaatcttagaagaatcatatctgatttctttacgataggtatcagacaaataggctaatttatagtcgtccatacccagggcttcgagacccatatcgtccatacgtttcatccattgggatgcatcacgcatagagtcgaattctttcttaacacaacccttaccatagatatcaatgtattttacggcttgctctggattagcatgcataaacattgtaggcttgtaaggaacttcacgactacgttcgttaccatttttatcgatgtaacgttcgagaatattatcaccgatttgttcgactgtcaaatagaattcttgcatttcatttcctttatagacgagtgattgtcttttgtttgttgatgaatcattatactccaaaagggaccgaagtccctttgcttaaatttctattgtctgacgtttaatagttgaattaccatcttcgtctttagttttaatcatagcctggaagacttgctggccaggatgtagtaacttttggaggtccttttgaaattctatttggagctcttcggaaaggtcaaaaatcgtttgagttggagaaagtccgtatacctctttaagacgttcacacgtttcaatttcaagaatcatattaattaccaatggtatacttagacagtagttcccagtcatttttctgcttaaaggaaatgacacggaaattattagtgatttcgaacagctcagagtcgtctactatatcaatcagtccccactccttaagaagctgggcaattgaatcacgacgttggtagtcttcaccatcgatatcaacttggcggccatccatacgcaacatctctttaaagtggacgatatagtatagcccttgcttttgcagaatgtggcaggattgatatagtttcttttctttattattagcgatacccatacgagttagggtctctttcactttcaagaagtcttcaggttgtttcagagtaatttcaatcattttaatttaccattccaatgctttctttttcaagtctttttgttctttaacatttttagttacggatttcaggaattcgtccgtaaccaaccctttcatcttcttaagcactgcaggaagatggcctttaattttataagtctcgagataacgataagcgtcatcattattaattgaatggtatttcatcaataaacgagtaataaaaactacactaacttcatcatcatgggccttagcccatttaccaaacctcttacccttaggaacagcgtgtaaaagatagttgaaatgactttggtcatcaagtttcagacagttaaccattgcagcctgcataatacaatccacatgttggctcaaactattatcgagccaaaattgattgtagttttccgactgagccaagttacgttggttcttaccatatgtgatatcgttcataatggcgaacagttcgttttcagccttttctttaaatgaatcggccaaggcttgaattgcagcgtcgttacgttgtttccaagcaacttcatgttcgttcagttcaacgtcatcatcaaaaagacttatagccattggagctccagagcaagttggatgaacagatgagtcatgtgaatttctgggttagccgcaataccgtggtattggttattttcaccgacaatttcgtacattctaacaatgcttggcccaggcaatttaccatagagttcgttagccagcgacataataaagttggaataatcgttgacatgacgtggagctaatgcacggagttctttaaagtttttatctttaagtgcagccactacttcatcgataggcgaattggtattcattacaatactcaaaatgcctgtatcgattttaccactggatgagtaacggtccagttggttaactgttttacggaagtcaggaaagttttgtttaactaaggcagcaataactttaaggtcttcgacttcgatattttcgtttttacagattgctacagcacgatgaatcatttctttcatcatggatgtttggtcggccggagtggcttcaccaaatttaataacacgacaacgggattgaagtgggccgataataccatcaatattgtttgctgtaataattacagagcagtttgaggaataggcttctaagaacgaacgaaggtgacgttgagcttcagcaacaccggcgcggtcgaattcgtcgataacaattaccttacgcttaccttcgatagatttggaagatgcaaaacgagtaagttcattacgaacgaaatcaatacggcagtcagaaccgttaacaaacaacatgtctgaatttgtatcagcacacaatgctttagctacggtagttttacctgtgcctggtgaagcagagactaggataatgttagggattaggcccttattaacaatggcttggagggtttctttatcatgcgcaggcagaatacactcagataaagtacctggacgatatttctgttcccacatgaattcattattgtttactgtaagcatattaatttcctcaggtttgtttttacattatactccaagggaggaatttcctccctatgctttagaacgagtggcttgagcctgcttccatagccaatacataagaagcttgtgaaccttcaaacttggctgcgaaacgagcgtcctggccttcaccacgggcccataacaatacatggtaatcggcaggcatcattttcatattagttttgttgataatgaatttgaattcagggccatcatggtctgcaaccactaaggaatacaatggacgggccaggtccttatcatcaacttgtttgtagccattgattacaattttaccattgtctacagtaatagcaaatgtatcaatactcagtccagaggacacacgcatcaactgctggtaatcttcggctttaaggtcaaaaataacttcagccaccgggaatggaatagctttgcttgggaatgcaattgtacttgggtcggcaataggccacttaatagttgaacgttggtctttaataattaaagtggtttggtcttcacttaccgaaacttcagcactttcagataccaatgacagaatacttaagaagccgttcaggtcgtagattgcggcttcgatatcaaaggtgtcatttacagtagcttcaccataacttgcacccgttactgaacgagttagaatagtgttaccaggtttaagcatgatacctgggttaataccggagaagtttttcagaatgttcagagtttctttagagaatttcataatgtttccttatcaagtcaaaaattaattaagcaataacgatcatttgtttacgaatggattcaggcagagattcaatatactctggaatctgggaagcaacaatagcaccagcttcaagcagttgttcgtcaaaatctacacaataatcatcttcgagacgttcagaaccatcacggtcgataaccagtttagcacctgcggccagtgaatcattatagtggcgacgcataatttctacccacttatcggatacgtcgttatcaatgataccgtagagcatgaacttagtttcttgtggaagagactgcagacgacgtgcagagtcggtatcaatattcagtacccatgatttacggatacggttttgattatgtgggttggaatcagtacgaatggttttaacttggatatctttaacagtaatagcgttagcaaacataatattttctctcatttggttggtagatgtattataaatcaatattttaaagcacttaatttaatcaaagtattcataaacgaaccaggcagggttcctgttcgacatgattctatcatactctgacttaaaagcatttcggagataatcttcagtaacaagatgttcgtctccagagaagttgttaactaaaacataccgctttagttcaggaacggccaacaaatgctggcctgttataaaattagaagccatataaatatctttatcggtcgctgtatcaaataaggatttgataatgaattataaatcaatatacgaaaagcttattcaacgcgcagttaatagaaatttaactacctataaagaacgtcatcacattataccacaatgtatgggtggaacggatgacgctttaaacttggtagacttaacacctgaagaacattacttggctcatcagttgttagttaaaatccatccggataatgtatcattagtctatgcggcaagaatgatgacaattagctcaccaaaagctgataggtctaaaaataaattattcggatggcttcgtcgtaagaattcagaagcccaaaaggataaagaattctcggaagaaaccagaaagaaaatgtcaatttctgctttaaaaaagcctagagttacttgtccatactgtggtaaaaccggattggttggtaatatgaacaggtggcatttcgataactgtcctaaaggccctaataaagtggttcatactataccaaaagaacaaaaagataaaatatcaaacacttttaagaataaagtatttgaattggttaattgccagttttgtggtatagaaggtaagaagagcgttatagtaacccatcaatatttttgcaaattaaaccctaaccgtaaaaagaaagaggaccctaaaataaagtgtcctcattgcgataaagtaggaatacctgccaatatgaaacgttggcattttgataattgcaaattaaagcctcaataagaggcttattccaatacggtaaatctaccgaccttcttcatttgaaggtgttgtccatacgattgagggtcatggtccttatgagaaattataaagatattagaatcttccaaagaatttataatattagatacacctttaataccctctgcatcaaaacttccatcaaaaacttcatctaaaattaaagtgcttatatgtattcccgagactcgagaagcaatatcacgccatgtaaacaataaagccacatctattctagacttttcaccttcactaaatgaagcataactaaagtcttcacgtccacgtgatttaatcgtctcgttgaattcttcgtctagggtaaagacgtagtcggcttccataatcttcaaataagaatttatctgcttattaaagataggaatgtatttcttaataatggaacctttaataccggtatccttcaacatttctgtcagaattccacgatgatatttttccattactaaggacgatttggtagagacgattttatcaagctctgcttgaagcgtggcaatctcttcggcattacttacgaactcagcagcggcttggtctattaatactttaacttttttagctttctctacggcagtaatggcttgttgcttatgagtagctatctgagatttaatagccagcgctttattacgttgttcggttacttggtccttaatgagcttgagttcttggtactgctcattaatcttatccaaagatttttgaagttcaaagttcttgtccttaattttagtaaggatgttcccatgctcttctaacccttgcatacacgtaggacagctgccgccagtttcgtataatttcacgaccttagtaaaggttgccatatcattcttgattgcaaatcctttattgctcaggtcactcatagagttgctagggtcatcatcgacgatgacattgagtaattcatcagttagtttttctatattgcccttcgcagtcctggcttctttaactagctcgtcatacattacttgtagacgtgctgcgttctcgccggataatttacgctgacgttcttcgttgtcattataaattttaatctgttgggtaatagaatcctgcttaacgtcgattacttggatttggctattagtctcgcgaatcaaagatttgttcaacttatccatatccgctaatacagaaacctctaagaggtcttccacaagctttcggcgcgcaggggtcgacaaacccatgaaaggggtataccctgctgtaccaagtacgacaatctgtttgaagcttgcataggacattccgataagctgttcaaattctgcttggaagtctttactgctggcagattcatcaagacgttcaccgccacaagagatttcaaaaacgttcggtttttgcccacgtttgatgtagtattctttgccatcatattccatccacagttcgaccaaaaggtctttcttattacttgagttaatcaactgccctttcttaacatcacgaaaaggcttaccgaacagagcaaatgtaacggcttcaaggaacgtagatttaccagcgccgtttttaccggtgactaaggtcttttggaccttatcaagttggattgtaataggttgctggcctaccgacataatatttttatacgttactttctttaacttaaacgttttcatgtattgttctcacgaattgtttgttcagcatattctagcatttcttcggaagaagcaaacacgtcgtcaagttccatggcccatgaaacaccttcagaatatccagaagtgacatacatagttccggtataccaagaaccatccacgtcccattctacattaccgaaccagccatcgccaatatgaaaatcatgtttatacattttcatcattataagcatccttgatgcatgattcagccatatgaattaatgtttctggagtatcatctaccattacattaaagctaaattccacagcccaatcagtagcaacataaactttaataagctcgttggtatcgcgagtgctcacggcttcaaaccagaacttaataatactcgtttgtccgtcgtcatcaataactgtgcagtcgtgttctagttcaagtcccgattttttgaattcatctaaagtcatcgtgtaacctcattataaagttgtgcagccatggtcttaagggctttaacatcgtcttcagtgtggccatcaggaagggcatcgatataatcatacatcatatccaagagagacttaacttcatcttcctctccagaatcatcgatatcaacgctgttatctaccttagacacaatacgtaaagagtgaacaaccttttcaagttcagattcgaacttggtaagcccgtcatcaattttatcgactataacacgaaccgcaatatttgtaaaatctttgtaatcgatagtcgcattcggataatgaatcttacgatgccaacaagtttcattgatgatgaaatccattttatgggtttctgtatcgaaaatccagaagccacgagggtcgttctcatcacctgcagtcagggtccatggcgtaccaatatacttgacgtttgctgcatcagaaatggtgtggaagtgaccagaccatacttgcttatacttcttaaggaaatcaggttctaaaccatgtgatttcattcctttatagaaatagaaaccatttaattcccagtggccaatgcagaaatctgctgtagtatttttgatatggtccatgatatcggtcgtgttttcttcacacatccatggaatcaaatcaatttctgtaccatcaaaattaaccgtagtaggtttctcaataaccttgatatggtcgtatttacccagaacttcagaagcagcgttcggtgtcaaggtatttttgtagtgtgcatcatggttaccaacaacagtatacatggtaatgccattttctttaagcaaatctgaaatatgtctggcaaattccatgcacttatgagtaattgctttacgaacatcaaaaatatcaccatactgaatccagacagtgataccatttgctttagaataattgatggcgtctttaatgcctgccaattgaatattttgcacccaagggtcgtcgttcttcactccaaggtgccagtcacccgtattaagaattttcattacgtatccgttcccacattttggaggctgctttagaagcagagccaggaagtttacctttgacccacccatcaggaatattagatgggttaatcagtttatgttctattccgttattataccacttcctgcccttattatgactagatgctttataattaggtgaacgaccttctacatatccttcggggactgtaggtgcaaaggtttgttctaatgtaataggattataggaatgaatataccctttagcattatgagagccgtaaagagggtgttgctctttaggtagcgaaagcccaaagaatcctttaggagctgcgacagccctattaaagaatagaggattttgggccgcatccgttcttaactggtacattctttcagcttctaaagcctcttctcttgtagggtgttcacttacaatacatgagtcaaataattctggatgctctaaaagctcatttttatagatttctttatatgctttagaaaggacactcccgtgatatccttttgaatgcttctctaaagtggtagaccctatataaaacggtggaagcttagtcccggaatatattgtcaggtatgtgatgtatttcatagatttattttatcatccgaatataaagcaaaaaaggagcctaagctcctttaccaactaatacaccgtacagaggttcgtgattagacctgaacttgataggcttataggtaatagtaccttcattttctgctttaatacgagcggcttcaaattgaagtatcatctcatttttgtcagatttaatcttatcaaaatccatcgaattcgtcattcatacaacctcttaaactttttcgtattcgtctttcattagccgcctgtccacgttatcatcgttgccaccatttcttaagttgatgagaatctacccaaaccttggctacgggctcaatccgaaaaattccatcggaatactggccgaccattttatattcggtttcggactgcttaatacagatattaccgtatgagcgaagtctaaaggcggctccaataagaagccgtttaaagggtttatttactagggccattgacgatttcccaaatttgtttgcgggtagattcccacatcaattgaacaagttcatcagtaacaggttgacggtaaataccacgtaatttaattaaagcgtacttatatgcttcaaagttgttttcaagtacagcgccttgggcatggagatttaaacgacggatttcacgagcattcttcttaagaatcttagccgcttgagaattagcttctttaatattgtgctcttctaaacgttgctgggcttcttcaatttgctcatcagtcaattgagaaatgtcatggctttgcatattaatcctttggagtcaattcaatagtgaagtagaaattagcgttctcaacatgataacggtaatctacgttattgtcaggagaagtgaattcaatattcctgacgttaagtgggtcaatatcaataggaagacctttaacatcccgtaatatcaatttaataaaataagggagtgcttcgaagtcttccattccatctaaaagtggagtgatattaatctgatgttccatataaaaaatccagttcaccaactttaggttcggcactcttatcagaccctggtgctttagttaaagaggtttcatactgagtcattttgtcgtagatatcttggataaaggtttcatctgcaatacctaccatgtcgtcatcattactgtcatagacattatggacgaagtagctatatttctttgccatttctttacgttcttttttgatacgctgaacgaaggcattaaaacaagccatagtgatatatgcatgtgggttgtcgtattttgtttcgtcgaagttgtgaagacctttaatcgaagcttcgattccatcagcaatcatttcttgcttccaagattgggtatatcctgagaagttgaaacgtttacttagtccttcagcaatgagcataatagccaagccgataacgtcgttctggcgaactattttattaggatcggtattttctctgagttctgttttccattgggtaatagctttcagaagctccttattatttacatagttatttttagtcagtttaatttcggtcattgttacctcagataactcaaatcataggtctattatatcatagtatttgaagacccttttaaagcatcaacggagtaagcaataagcctgaaatactgtttcaaggatttgtgtgaactcggaataagaaattgtatcagtacacccgtgttcagacatatatccacaaaattctttaaaaagacttggatattcacgatggttgtatttggaaatatgagacttccatactaaagaagtctcaccacaaacaaactcaacatccatacagttatctattaagaaaaatccgagaccttcgtaggcgagggtggtggatatgggtttcattgtaggaatcgagctccttccaaggcatcatctaggttatcgaactcgtcgacgtaatcaacaccgccaacctcatcttttgcatacagccaatactgtttaaattcgtattcgatgataaagtggtcaccctcaatctggagagtcccatcaccattaaattgaactgcataacctgtaaagcggacatcattcaagagttcttctttcatagcaatcatttccaagtttttatcgtaattagagagttttattttaatcatttcgctgccttaacaattttcaggtcaacgaattttttcttacgttggtttttcatacgacggatggttttatccgtgatttcaccaggggcccaagctttagattctacaccaaaggcagcgacatcgaattcatcgaggatatattgaaccaggatttcacgaataccgttcttaccaattttctggtctttagagtgcatgataggtaacagttcagcaacccattggtcaagaacctgaggagttacaaaaccggttttcatcagttcgtttactttatcgaaagcgaaagaattcagtacgtttttaatagcttgtgacataataatttcctcagttttaaagttataatccgtaggaccattatactctggtcccaagagtttgtaaactatttttgtgctttggcgcctttccaaccttcatacatcatcgcggcggaaattaacaaagcgcctgaacaacttgaatatttgtgattccaaaaccagttcagaaaaacttcgtcatcaataccttgggctatcatattttcaaagaactgacgacgagcttcagcaattcgctgtgataatttagattcaggattcattttaaattttccagtttccgtgtttatcaatgaatttaatccagtcatttactgaccacgtggttgtatcgccctttggtctgatatttaaagtatacaacccttgcttaaaaagcattcgtttaatattcatattttcctcagctataacgataacattcgtttgatttacgttttgcaactcgatgagaagtattgtaatcaggttcatcgtcattgtaaacatcttttttcagctttctcacttctttacgaagctggcggttcatttcgttcttaacttcagaatcaacaccgcgcatacgtttccacttgtcagaacggaagatattttcttcaaccagttcctgacttacgccgtccggtgctttacgacgtccggaataataaaaatcttttacagacaattctttacgacgaatagttttacccatagttacctcagcagtttgtatccaataagatttttaatgtattggacatctttgacatccaaatctaacttaatatctttcaggcgttcggtcagagtaagaaatgatacacgtttccaattcttaacaggacagcaataagttttcgggccgttggcgatttcaatattcttatcagtgacggtgagaaaaatcaggcgctcatcatccagattaagggtgacgacatttttcattgaatgtaatttcaggctcatgatttaatttccttagctactgaacaaaataaaggacggtcgcacaccatcattggaatatttctatggtccagtacacgataccatacgtctgaatcgctagcagcaattacacgaaccgcacgcccattcaccaaataatactggtcggctttaatttctttatcttggatagtcataatgttctcctcatgtgttgataggatagactataacacgtgaggagaggaagtaaatactaatcttcaattaaatcttggtcataaccaagttcaatcaaaagcgatttgaaggcaggaatattttctattttcttattatcgacaaatatgacaggatagcgtatcgctaagctcttgaagcctgcacgtttggccaatgatactataagaggcttgtcatatactgcgcctgacggcgtctgattaatcacaggatagaaagtatgtgggatagaaagggaatttaggagcgatagaacagcaatgcaccctggacagcgcatgactgtctcagggataccgtaaatctcaattttagttaacttttggtccacaggaaataactccttggtagtcccaggtttttagaacttcttcacaaacagcttcgtcatcaacagtttcataaggaacataaatctgtacaaggaacccggtatcatcaaaagagaaatagacagtaggtttaataccatgaatctctgataaagcgtagatgtccttgaggtcttcttccttacctttaaagaattccgggttcaggtcacagtcatggaagtaccaatcatcaccaaacttgtcccaagcggtccaattcaaagctacatattcttcaaaacgtttcattctttcaccttcatcatttttgcaataacactatgaacagcctggattcgtttttcgaactcagacccttcaagacctttttcagtactcaatgcaccaataatcatgaacagcaatccaaacggaatagccaggattaaaaggcatacgataaacagaactaatgtaatattggccaggatatcagaaacagcattacgaaatttgttcattaaagaacccacatgttagttacaacaaataaccattgagcaggatactcaacacccataatacgaaccgcatcgttcagagattcggctaaagcataaaatgcgtagccataaaaattaatcatttaagcgatttcctcagttgttttttgaatgaatccaccatttgtttcttagtggcagattcattataagtcattccgtgtgaaagcatttcagcaatcatttcttccttacccaacctgctgaactctttggttttatcaggaacgaaattaggatggatattgttttcagtataatcagctttcagatagaccagcaaattctctaaccattcgaggtagtcaacgttttgacctttaagaccagaacggttgaacttatgcttcatttgtccttctgcggcattgcacagattacatagtaaaccacgaaccttaccggcttttggcccgttcaattcatggtcgtggtcaaggtggttactttgaacatcagggtttaattcacgtttacaaatcaaacacttaccacattgtgcatcataaagtttttgtttttcttctttgtataatttgccggtcaacaacataataaacccttaccattattagataagggtatttattaatatcctaatagtttagcagtgcaacttagcactaacaacaatccgaataaaacaactcctacccaaaataccgtaataagagcctccatatcagaccccatagaatgaacggtgcaaacgtttaaattgccgaatcatctttttagtaggacgggtatataatcctatacaggtggccataaactggtcagttggacttcctttgataagaagtttccagaccttaccgccatttaatttttcggtatagactaatacagttttcatgcgacctcaaattcattatcatcgttagtccaaaaacaccagaatgaagctttagtatcttcaaacatttctttagtgtattcgtataccttaccattaaattcgatagcagttacgccgatgatttcagggtcgccccagggagaaatctccaccttaaggattttaacttcggcgccttcacaaagctcgcctgattcaaagccgcgattgccgtttaattcaggccagtcaacatagtggtcgacatcttcttcagtaatacgaacagttttaccttcaaattcaaataaattcatcagaaggcctcatcggaaaagcgaagttgagcttcaagccaatgaatataatcggctgcagatttaatcaaatcggattctaggtcaggtaaagaacccgaatccgacaactcgtaaagcgaatgttcaatcagacggcctttatgacggccaacttcaattttggtactcatatccaaactccatatcgattaaatcattgtttgaaggttcattatactctatttcggaatcgttgtaaacaggttcctctggctcggtagttttccaccgagcgacataccatggcttaacggtcacaccaccaactacttacttcaaaatcaggttcaccgtgttcccagtaccaaggaccgactggatgccaatcaccgtgttcatcttcttcaaattcttcagattcaaggccaacgtattgccattggacttcataagcagtgccaccgattacaacggtgttctcgccatatggatgagctacagcaaagtctacaccttctgctttagccagccaaaccatatattcgtatagtttatattctaggtcatcttcggtaccatcacctagaaaaatggtttgttcgtttaattcaatcatttgaagttccagaatgaagcaccaaccagaaataaaggccaacaaatcatagacgtcagccatgaacaaaagtcacctgaatcatctaatttagctagggtcttagcataaccaataccgatgataagatacaaaacaaccaacattaattcaatcatttgaaataagctcgcagttggtcaaagccaccaatagaagttccgtccggagcaaatacctgaggcatagtcaaacctacctgagattcgcgtccaagagcagccaggagttcggcaatcttctcatcatcaaatacacctttttccggcatcacgttaatgaattcgtaaggttgtttcttaacatcaagcagtcgtttggcattatcacagaaaacacaacggtgaatatttgaatcataaccataaactttaaacattttaaattcctaatatttgtttgaatgcttcagaacggtcgagttctgttccgtatttttccatgtgctcatattttaaattatacacatcagatagtatattattatacgagcgagttaaagcagatttcaatactgaataactgtccggaaatttaccgtgctctttataataagctagagtaagttcgcggactgccttatcggcagcctctacatattctttacgctttgccattttcttctcgctcaaatttatgtttacaatggcggcatttgtaacgaagattactagtctgccaatggaccaattgaacctgttctgtgccgcacttaggacagttaggaacattcttagaagcttgttctcgtcgtgcgaccatagccattacagcatcccaattaacggcatcatcataatcatcacaaccatgaattttaccaaccaattcaacttcaacatccgcggctttaataaatttcaataaactggtattagatgctgaagcaatatcttcagctaaacgttgtttcatttcagcagctccagagcctgttcaagacggtctaaacgattggtagactcttcccaaagtttcttggcggcggtatattggccagtcagttttttgttgatagcaagggcgtctttatacgctttttccaaggcaacgacttccggtaacttggatttagtaattggtgtaggggccatgatagggctgttcaagtcgttaatcaagtcttctaatgtagcaggctctttatcagtgttcacaatttcctcacatttttcttggtaaatttcagcgtcagtttttggaacggtacatttgatttcgcgaactgttactaaaacttcatatcctttccaacctaacgggtgtttgatttcttgaatctcatatttctctaccgtatgcatcaaagctaaagcctgttctacagtattcaaggtattgtaggaaatatcgtggtatttcgagacttcaacttcatctttaggtttccaaaccggggaccaaataatagaaatatgcaccctaccatttttagcacaggctttaatcatctgaggcgctattggatggttagtacggcaatcaccctttacaaaagttttggctgctgctttaagaattaaagcactatttgtgtgaaattcaccagcccaacgtaaaggaaataggctcttagggtcagtacctttaattttgacatacccttttaaaacatcaccaaaccatttgtagttaacaacacggctggaacctggatatttctctttgccaaactctgaaaggatgtccttattgaccagtcgcgaaagcagtcgagaacctttaaatgttttaatgatatcatgaatgcacaaacggcctgcaatcttttcgatttcggctttgaaacagcgcgataatgcatcatcaatttggtcgacccatttattgatattagaaactattaccacatatggggttaatggaggggtgttggcagtgatatacgtagtaaaggcattaatgtattcagtacgagtcatgatattctcctcagtagatttaaaaagattatactccatccgtccttggatgtaaacattattttagagctaatactgccgcgcggagcttgtcacgctggagttccatgttcttgatgcgaatcaatacgtcttggatactctttttctcatcttcgatctggccgtttaaacggtggattgattcctggaggtggtcctcatgatacttctcgataggtttcatcgtagggttagtaacaaccaaagaattatcaggtttaattttccaatgatacggttcagaattgaatggactcggtacagccgtggttttgaatctgtcataggctgcatactggcctacgctgtcacatgatactgcagagatacgacgttccatttgtggttccttttgttgggattgataaggggcataagacaaaagatattcacgagttagtttaatattaaaataaactgcatcagcccgctcaaaacaatcagcatattcatcggttgtaactttatatgattctactgccttaatacgggtcattgcctctctgaataaggtttcgaatgcttcacgaagggccttattaccttttgaggtaggacggaaacgaacttgaataccgtcaggcagaatattaatgactaggttacgagccgtaaaattaatattcttgatattgacaggaaccgtagaaatacgtcctgcggtagccaagaggtctttgatattagctcgcagtgttgcaccaaataaatgagcagggcaacggcaataatcgttcaaagaactaatataagtccctttacgacctacaccataagtataattaccattacaaatatggccgaagtcggccagccgatcgatagcgatacgacgagtcgtgtcatggtcatagatggaatattctttacgtgttttaatgttcatatcagagtccaaataatttttcatagagtttagcgataggccacagaattagcatacataaccaggcaaagcaaaatactggccatacaaatgtaatgaataccgcatcatagcttgattcaattttaaccgggttccacgcgcctgttttatgcgcaatcaaagcagtaataaatcctatcacaagataagcaagaataaaaccaataatttccataattaatccttaagaagatttaggatatcgatatatttttgacgttcagccttggctttagcattcagaccagagagtcggaaaatctcatcatcttgttgttgaattgtaacattcaagcaagtaagcaaattgctaaaatactcaatctgggcttgatgcttctcattgctgcgcactggcacaggttccggtttaggagcttgttctgaatgctcttcagccaggtctttaattttataaagtttaatacgctgacccaccccagtttcggcatcaccaaaactaagaacaccgtgctgttctaattcggacaaggctaatcggagatggaacttccagttgtcatattgacaaccactaaaagttgaaatggtatactcattttcatttccggggtggttaacaatattaaagataatccaatcgcctgaaccattggtcttaaaggtcatttgtttatcaagaccttttgcaaggcgagcgccaagagccagtagacgtcgttggttggcatgaaggtcttgaaccacttcgtcaaatgacatcgccgggattaaacgaccatagaggtcgtagcctttgttataatttttaagaataattttggcattagcacgagacaacatacctgttttacgaagagttttcatgacccggtcttctaaggtaaacgacctggtcttgtcaaagattttagtgaagtcatctttaacagtacaaacgttgaacttgtcccacatcatatatagaaccttttcaaccacttctttagaactcggaatacgaccaaatttaacaacttttttaacttcagaacgaatttgattaattgcctgtgacataataatttcctcagtaagtaattaagaacctagaaccattataccatccttggtataaagcgtttatgcgagaaccgtctttaaacgctcttcaaatttctgaagcagagcttggcgttcagctcgttgtgatttgtactgctcgatacgacctgaagtgagggcgtactgttcgtttactgattcccgcatgaattcaggaatctctttacaagctttgatttcgtcaaacttatcaataacagcttgttgttcagcaatcagattatcgaaataagcgatatcagatttaacgtttgccaggtcagattcggtaggcattaaacgtttgttacgttcagcttgataagcttgattggtttcacgactccagtgaagagtacgttttttgttagtgtttttatagagctctacaataccaactgaatcgatgacaacaatccagttccaacggcttttgtaaatctctcctccagatacagtaatctcattaccacaagcaacgtcgttaaagaacttgctttgtttttcggatttgaaattaccattgttataattgatgagtgaaaaaatatctttagcgttcatgttaacctccagtagttgataggtctatagtatcatttctactggagatgtaaacaactaatagaaacttttttcaccggcttgaccactaaaccatgcggattgagtgttctctttccgttggtgttcaatacgaatgcgatattcattcctgatggcgcagagttcatctcggaagtcgcctgccaactttacctgcttgcggtctagatttattaaggcctgggtgttaacggccaagcgcagtctcctgaagtctcctccactacacggatttttatagaatttctcagaaaacttagtactacattcattaatatagtcttcaacagactgtttcatagctttggaaaaagtctgacctgcgttataaagattgtaaataaattgttcgaacataatttcacctttatttcagaagtgtaacttcagcgatttcgctccagtcatttttatcggtggcaatgaagtccgccagataaagagctgtacgtaatgatacgttacgaagacgagatacattagccttcatccatgctaaagcttggtaagtctcggcatcagtcagaccacggttttgcatcatatcagtggacaggataacgtcttcaacacggaccataatctcttcgttagagtgaactccgaggtctaagtaaactgaacgagatactaaagcctggaggtgtggagcaagtttagttccacgctctaattcacggtcaatatcaacgttggtgatgaacacgatggtgccttcatactcaaattctttatcgatatttttatcatcaagataagaacttgaagtgctccagcacaccttacgtttttcaccagtatccaatgctgcttttaacaggttcaggatatccatatcagagaatacatcaacatcatcaataagaagaacactattagggccgcggttattccaaagctgctcgtaaagaccgattccactaatctttccgttgattgatttatattcgatagtttcattttcgtgggcattctgtaatgctttatctaaagaatacgttttaccaatacctgcggcaccagagatgataagggaacgaattttaccatcgatgattccgttggtcatcatgttcattactttaaaacgtttgttgatgcgatgtttcatttcttcagcggattcagtaacaaccgcaggagcttcagcaccttcggtttcgatatcagatttgaacacccatacaccacgttcaacaccatcaatctgtacgaataccttgccatcaccgaggtgagcttcggattcatgaattttgttagggaaccaggttttacctgaactcatgaacgtaccagagatttcattaccgcgatagatacctttgttgattttgatagttaacattatattctccatttcactcagtagatttgataggtccataataacatgctctacgagagtgtaaactctttttttgcactaaacccaaaaaggaacccgaaggttcctaaattgcattccaataattatggaagcggatattattaatggaccactcaacaaatcgtcttatctgtttaggcgtaggtttgcacacgtacttgatattgactcgacgtccggtttctttacagacagcttcaagataccaacgtcgggttttatggggtcttccatatgataaaaagaccttcatttcttcgttatcgataataagagttgtggttgtcaaggtatacctcttcaacaaacttgtcccagaacttcatatctaccttctcaggcataccgttcttagatgcctggatggctaggacttcaaccaaatcaacagtatcttcaagaagttcttgaacttctttaaatggtaattcaccggctttaatcagcttaatgatagaggcttctcgcaatgggaataccaggtcgcctgtttggtagatttccaacaattgatatccagcccgataagcatggctcagagctttccaatcgataccttcattagcttcagccttacgagcacgttcgccatattcagcatcaagcttattcagagattgcttgagctcgattaaagacaaagtagtttggtacttacgtcctagaacagtatagaacgtttgagggcctgttttctcatggttatggaatacccattcacagaactcattttcagggagtctgtgtttgatatcttctaccttagtacgacgaagtctatcagggattccttcttgatagtcaacccactgttcaggaatctggttaacaatagccagtacaccacgcagtgcagctagtcgagaacccttaacaccatatttagaagcttgcttacggacgtaccctaaataggctttcatgttagtcgtatagaaccgagaacgattgtcttggataaatttccatacaccaggtaaatcagatttaaccaccatttcaggtggagtgtggagcatatccagagcaacggtttcgccatctgccgccagtttaaagaaatatttcaggctgtaaagctcgtggtcaacatcatctttagtgtttttggaagcagtgttattcgtattcaggttggtatggttcatagccgtacctaacagaatatcacgcggatgtggaacaaagatttctttaaaatcaacatcagattctggagtacttgttccataaaggtgggagccaaaatatcccttcataactgttctcattattcacctctttcatagtcttcaataaattgcataattaaacgttggtagttagatttggggtatcctaatttactaatataagtaccaaaagccccacgcttaggcctatttaatttaatccataaagaataaagcaaatcataatcttgccaatgttttcctattctttgctttgctttagaagcatcagattgcctctttttagtctccggattatttagagatttcttaacagcattcgaatgcctttctctaacatcagggcgtttaaatgcttctttaatagctttagaaattttctctttaacctcaggacggttttgagcttctatttgggcggcagacattttatcttttatttccggtagactcatagttatagaacgtttatttctatactcttcagtcttccatatttctttcatcacatttgaatggatttctgaaaatttttctctaactaattggtatcctctagaagttagtttaagatttcttcctagagaatcctcgccgaagctataaaacgaccaccaagcataaattagtccagaagaatcgggatgaattctagctagaagccaatgtgctataaaatgttctctggctgtcaacagaactaaattattaggttcatcactcccaccaatacatgatgggagtatatgatgggactctgtataaaaatttaatttggatttgtctaatcctctaagtttacctctttggattagactatcataaagcttggtataattcattatgggtttgttttgttctcaaaatggattacaggacagaccttagatttacgagctttaatgtattgaataacgatattttctttagtttctcggccttcacgctcagcttgaatacgttgccattccttttcttctctacgggcatcataccatgcgtgtaaattcatcgcaccgaatgccaaaccaatggatagcgcaataataagagctattgcaaccaatcctaaaacaaaccctagactcaacagaacaggggtacttaatacaaagaaatgctctaatacaccaacacctgcaacagttaatccaaaaagcgtactacctgcaacaacagcacaagcaaaacaagcccaaaccattttccagaagtaagcacataaagagtgcggtcgagaatgactgtcataaaaacggtcatgaagtttagcgtgccaagagtttgcattgataatcataatcataatattttccttaagagttcatagttgggataacagagttcagataagagactaaaacttttagttcgtctttagtaaataccacttcactttcaccatcgtgtctttgggtcaaggataacaaatcacggccctgatgttgatacacggttaattcagtatcataattcagttcttcttcatcaccttcaaaggtttcactagaacgaatcacggcatcttggccagggactttccattcaacttccggcttgcattcttcctggaacagtttgaaaatacaatcaaagaatttatcagaatcgctgatgctcagacattcaataccattttccagattaaacccggtttcatttttatagatataggcaaacatatcatcattgatatcgataggagcactagcccgaccgttaagataatcgtgtctatctaaaaccattaaatcataaagcggtttaatatcagcgatagtcagtacgattttatcgtcttcttgtgaaagctcaattgcgttattaactacttcagcggacagttcgccaaacaattcagttgtttcaataatcattttctattcctcaacggttatgttttaaaatactataaagctcttcgacttggtctgcattcagacaaatcatatcattttcttgttggagcgtgattccacctttttcttcccaatctttaacaaagacgtcatcgtcagattcttcaacatctgctaaaagggcaatcacaccatcttcagaacaaccatttggatcgtataacatttacaatttcctcactaaccatgaaaagaataaaccgattaaaatagggcctataatcattgttgaccaagcccagggttctaagtaataaatcatcttcatgctcctgtgccatcagccattatgctttcaactcattaagatactcaaccaatgccgctttagagttatccaaatctcgtttacactgctctattgcggaatatgaatagccttcgcaatgttctactgcactatcataagaatcacgttcaatagcagtagctagtttaaggatttgttcaatctgttcagtagttaacataatatcaccagtatttgttgatagtagaaattaattcttgggcttgggtagtcttcagtttacatccacaaccctttaatgtgtctttaaggagccacggttccttgagctcgtccttttctagacgaattctgtatcctcgataatcagcgaagatacttcggtcgtcgaatatcttaatctcaaggatacgaccgttgatttcatattctaatgaaaccgtagtacttgtaagtttcatactgttctcctcattagttgataggtctatagtatcatgttcctagaggatgtaaacacctaaacgaaaaaaggtcccaccgaagtgagacctttgattattctaacgtcagcaaatacttagtctggtaaaagacgccagtgatatcgtccaaagtcgactggatggccttaggaagggtgtcatagattttatcagatgctttaagaagctcgtcaagaaaatctaccgggtccttaggcaagtctgaagcagacggtaatgatgctttatattctttgccactgaatccaagatattgctcactaaattggtccagtggtccttgaacttctacataatagaagtcatacgctttgtgtcttgcatagcttttggtttctaaatgggctgacttaaaataggctaaagaaaccagtagccaaccaatataagaatccacttcagaccctcgactgggtacgaaatcattgaacttcatcttccaccttcattagttttacataacgctctccgatggcccgaccttcaattgagcacgcttctatagtccgacaacttgaaatcttccaggaagccgtaacataggcccaatagtcttcggaggcctttacgctgggtctactcatttgcgcataaacaggcatcgcactactagcaaatgcatccatcaatttatcattggcaccatttgctagtgaaactgtagggcttaaacatcccgccataaggatacaagccgctgtacggaaaatatccatacaaaagtcctttgttgttttatactatttgcctttcggccttaaccgatagcgattaccaaaagctaaagctctacggttagtattattatttatagctttttaagcttacgacaataagaatagaacacgtcgttaaaattatattcaacccaattcctctgtataggcgaggtaatggaaagcatataatgcgctttaattaaatccatcccatttttattaggacattctttattattagcattatacgtcgctgctacaacctctatctctcttttgtaagccacatcatccatgataggcgaaagaacaatataagaaatagccacagcgaacgctagaattaaaatctttgaatttaggtccataataccctcaactcgttatttctatccagtgcttcctgcacaatgacacgtaagaatcgttgccacctatagaaacttgggcgccgtccttaattgcgataccatcctggaccctagcagtcatagtagctttacggccacaatggcacacacctttgtactcaacgagtttatctgccgtagcgagtaattcagcagagccaggaaacagtttaccctgaaaatcagttcttagcccatagcacataaccggaacattataattgtctactatctttgccagttgttttatctgtgcaggttctaagaattgtgcttcatccacaaacacacagtggatatctttttgagattcagcccaacgatagaactcgtataggtccatatccggagtcactgcattagcctcttggctaatccctatacgagacgaaatgctatggcttgattctctattgtctatcgcaggctttaaaaggagtacgcccataccgcgttctttgtagttatgagcggccgttagcaatgaagcagttttcccggaattcatcgccgcatagtgaaaataaagttgagccatattaccttcttaaagactatttacataagcaattaattcattttcctttttagaaaactcatcctcttcaccacctctccaatcccaatccagagagttatcaaattcacattctatgttgagttccataagctcatggataagctcaaacaatttatctttctgttctttactcagactcataaccattgcacctttaagcaatattcttctacatgctgtttacgtttatttttatctataaaagtatattcaacatattcaccaatataccatttatcggtgttgtgttgactttttatagggcatttagttactcgtgtttcggtccagcgtcgaataatttccgctttgtttttagggtcaaacggatgcgggtaatgggctttcataatctaccaccactaaattaatatcaggagtaaacaaattaatcaattggtaaaccttgtcccaatcaccaccagcaataccacaaccaatgcgagggatataaattcttggtttaaacaaaagaccttttgcttgttgatttaattctatcatacagtttactaaagcaccataatcaagattagggcctggttcgtattgggtatataaattatagcaaatttggccattattacctgtagcttgagtaaacgtgccaagttttgccaaattgcctaaataagtagttttatcgatagcgagaataggcggataagccttagccaattgcccagctacacctgaacccattgtgtggaaacagttgcacccgtgtgcaacattattaccttgaagaaacagggcgacgatatcgcccttaatataatcaataatcatttagagtttaatcctcgattgtatgagtcaacgagtctgtctaccatagacgcgcacatttctttgtactttttatcagatggaatacattcagtaacgtttagacgttgctcgtatcttttagaaagagttttctctttcattcggcgatgctctacgtcattctggccatctttaaaagcagctgtgatttttgaactgaattcgataatgcattcagtattgctcggatgacaataatcttttgctgtacgggtagcatactcgacaattgaattattactatcatcaacttgtgacgctaatactcccggagcaatcaacataagcgctatagtcatctgcttaatcatttaatacaccgcctcaaacatctttttagattttaggtaattggccttttctagaacttcagaagcatatttactgcctgctttggcgttccagcccgcattataagaagcaatcgcttttctcaggtcacctttgtgaacatcaatccaataagacagttcaatgtaggcccaagaggcactgttctgtcgtttttggaccatacgaattatttctttgtcagacatcttccaacctacctgttgaacacgacttcttaacgtaggcaagtaattttggaacatgccataagcatggtgcttatctttatttaaaccctgattaattccggcagatgattcctgccatagtaatccggccatgatatatcctaatcctttttgattaggggtttctttgaactttcccgacttttggtattgttcaccgaaagcatacgcataatgtaaattatcgagttgttcattactgaaagtaggctctacgctatgggcagacatactaactgtcaatagtaaagtggctaatacttttttcatgagacctcattattaaagatagattactttcgtgctggttttaccttctaaacgtttagagttaacaaatgccatacgacatttaagggaatatcctttatcaggatgtttacggtctacagtcatacctagccataaggttttatcggtaatttcgagacgcaatgggcgatacactttaccaggaatgatttcggcttctacatcaggcagaggttcctggattaaaaattcatgaatttctttaacatggttatggagttgcttgaataaagcaaaaacgtatttttcgtcgatttcacgttggatagcacggtccaacaagtgattagagtacttaataaagaaggctgggactccgctcttaatggcggcttttttgatggacgcattcagttcacggaattcggtttcgaactgacgacgtaatttattgcggcggatgaatacttctgaattaatttctgacattttgtaatctcctgtagttgataggtttatagtatcatacctacaggagatgtaaactgctttattcttggaatggggtaagttttccagcagctgaacaaatttctaccagtacagggtaaaactctttcacttgttcaaggcgttgggctgcatactgtacttcaccttcttcgagacaagccatttggtcgtcaagcaagtatttgtggtagccagtacaggcttcaccgatgatacgctggaaatcttgtaaactttcaattttcatcagtatttttcctcgggttggaaaacggaacgacacgcccacatgcttgcttctttcagacggtcaattgcattacgaatctgggtgatgcgttcatgagcctggtctagttcttgttcagaaacctcttcggtatctaagttcatataatgagtaacatgttcttcttccagagctttaaacattaacccaagacgaacttcagcatctttgatagcgtttactttaccaattttatcgtcggtatgcggcttataacccttgatatcttcaatcatttcacttcctcgccggttgcgatatcatattctaccaaacgaaggccttcagtccaaccttgcacggagatataggtagtcgggtaaatcatttctttaccattccaccgaccgccatcccagacttccagaaagtcttgttcacctggtccattaagccattcaacaaatcttttcagagcttcttcagaaccttcaattgtcaatttagacatattttttccaatcagaaatcatatgaatctcttggtcataagtcaagagactacgagaaataatacccttacaaggccctgagatgaactcgagagtgaagtaaggaacctgtttcattaatcggatactaggagcatgacatctaaaacgagagcccttaaagggccctgtcatgaatacatattccaatgggtagaaataagcatattcgaaatttgcagtaaggtcctctcttcgaaccttacgtgagaaataacagaactcaaaaagttcttcatcagtcatcattgcattcctatcacaaagaacagaggcaaaggcttgtcgccttggcacataaatttattaatcattacctggtaagcttcatagaacttatccatcgctggaaggcgcattggctcttcgataataatcaataatcgagtaacagatagtccacgatacttatggaaattgtcttcatcaaggaaactgcgcacagtatcatagacaacaaaaccaggaccttcgacttggagatgtgggtgtgccttagaaacctgttttattacattacaaatttctcgcgagcgatgcgaagaactcgacataacaatcacatcattacccttggaaacccaatcagcggcgaactgagcaagggcacttgttttacctgtttggcgtccgccatcaagtcgaagagtaccaaactcttgcattcttgaagcgggttcataccatgtgtattggtctgagtctaaacgttcaatggcgcgttcagcgaaggcgtgcattaaggttagataaatgggagttaaaaatttcatagtagtctcttagtggtggggccattccttggcacataattcgtccatgtatccgtatgtaaaccctttaccgcacttgggctcgaccttattacaggtagggaaaggtccatcactcagaggacgcgacgttcatgaggagagggccggcttgcctttattagaaagaaccagaacctctaattgtgttctggcgacctttattttctaattcggagtggtcgatttcatatgcttgtgctacgccaaaggcctttttaactttagctaaagaacctttagatgtaacaatattaaaagtattacctttggtaaaatcaacaaaatcgacttgtacgccctgtttaccgaggcttgctacaatagcatcaacatattcttggtctaaattgccttgaactccaatttgaaatgctttaggagctttggcttctgtgataaattcttgataagttttcattgttattccttaagttgatagaagtattctatcacggatttaattaagcgtaaatagccttgccataatgtttgtaccaggtaggacgctgtgcaattttttcatccaaacgggtctgagatatagcaatagaagcttcgtgtggagtatagtcaccacggaattcctgaggaatgtcactaatgtcctggacagtagtatccttgatattaaaaccacgttttaaacattcggctataagctcaatttgtcgcttacgtaaaaattcaagcttatcgtaaaagaatgtaacatggcctgtgccaaggataaaagtaggactgattttgaaatcacggacatgtttaccattagcaacatgcttacgaactgcaccgaaaacacgtggtaattcacgatattcagccattaagtgttggtcagccaattcagatactaaggtaaggttgatacgagtcattttagtgttctccatgtttgtatgagaacactatatcacaactatcgtaaaaataaaccgttatttacctttaattgctttagctgcttcggtagccgcttgctgaaggtcatccatagacataccgaacttagaagcaaagttatcaattttcttttcgacagaattcaaaggcttggcctgtttaccttcattagcgcctgggagagcgagaatacgctctttgtcaatataaaggcttacaagtttcttacggtctttatcgggcaaatcatgaaatgaatgggcctttttatttacggcggcttctaatttacccgcacttactcgcgcttcggtgataaattcttgataggttttcatatgtttcctttaaatgtaaataggtccgagtattcgctttattaattaccacgggctgcattagcaacggcgtaagcgtactgaatattagcgtctttaaacgtacctttagaggtatctagttctgccttaaagccgcctttaaccataacatcagcaaattctttacggaaagtcattgcatcaagacctttccatgcggatttatgcttggcaaattcaagaccggcgaagttaactgctttagccaatttattatcaatagtccatttacctgctttaggtacaaacaccgggcctttctgtttagagaacagttttaaattccagcgacgaaggtcaccgtcagctttaacaaaagctgcgtccaagttactagcaacaacatcttggatatgggcaaatttaagtccatcagcttcaatatttaggtcgttacgccagcgaagtccttcccaggcgaaagctttaaagtcggaagcttttgtagccaagtaccgttcaataggagctgttttagcgtcaaaaccgtttcctgggttgtcaacgccgtttcctttgtaagtccactcatctttattaatgccttggacctttcctacagaagcttcggcgataaattctttatacgttttcatacgggttccttaaaggaaaatattttaattggtctgttcaagtaactgtagatatactatcacaattctaggagatgtaaacttatttataggtcttcatccaattcttgaacaaagccgcgacgtctttctctttaacgttcagtttaatgtccaacattttaccacccgctgctctggtttggcgaatcttagcagtaccggtttcgccattccactcaacataatactgtccagtgttcattgcaataccatcaccgtagtcttcatttttagaagtggtgaatgctagcttcatagtcttagatacacgagcctgcatgcctgtctgaagggcattacgaacgcgaataacctgaggagtggcctgggtcaagttctcattcagttcttcagtgaactcttcagattcaaacatcgccaaaagttctttagatgcaggaattacattctctgcgataaattcattataagttttcatatgctttccaagtacctgttttaaatgttgaaatcacgcgcttagcacgattaggagtttgtttataccaacgggattgagccaggttaactgccgcatcgttccaacgtttctgttggagcatacgtaaagagttagtgaaccctgctacgcctgcttcacccatttggaagaccatgttaattaaagcacaacgacgaacttcgtccagtacatcataaacaggtttcaatttaggattacgcagaatagctctacgagcattttcaaccgatcggttaaagagttgttcagcttcagccatagtaatacgaccattacaaactcgacccataagcttatcaagttcagcacgagcaacatctttagaagggttcttagtaatcaattggccaataccaatagtccaataaccttcagtgtctttataaagatttaaatcaagaccttcgtcttgtcgtaacatatcaaaaatatccataatacctcctgagtataggaggtatttatatcaaaagagcgaatctaaaaccttaaacatcgacgggcccatgacatattcccattgcggacgtttaatcaaggcaaaagcatcaaattcaggaatagtacgaccgtcagggaacgtatggtaagccgtacatttgcaatccttgaactgctcgtgttccacaggcaccgtatataagaacagatgtagattcttattgcttgaatatttgaactcacccaggtctttcaggaacgcaggatcgtatgctgtgaatccaatctcttcttcggtttcgcgcattgccgcttgaatgggctcttcgcctggttcgacatgacccttaggaatgtcccatttatgacgcatattctctggattacgagagcctgttacacggcccatgaccagttctttatcaacggtcatgaataaaatacctgccgataattccttagctttcttactcatcgtctcgttcccatgattgtttaaaaatatcttgcataataatttgaagtctattttctgatgatggactttcactatcagacacttgaagcatatagtcaccaataggacagaacatatccatatcgctttctaagtcttctttaattttctcttctgatgttccggtatcataggaatacaggtaagaatcacatgactcagatttaatataaattgcaatactcatttacggcattcctcaataaactcatttaaattctgtttgattttaccttcgtcgtaaagacgttgttgacgacgtaaacgccatggcatttcaatagccaagcaccaaatacttaaagcagcgccagcggcggcaaggttcattaatccagcgccaataatagttcgttctagcgcatcattccagttggcatcgattaaaaatgaactcagcactaacattggaagtaaagtaataaaatacgctacaacatatcgtccgaacgtaagccattcagtatcaatgagcctggcctttccatcttggagacaaatatacttatcgtcagtgcgagtgattttctttactggttgccagccgtttacaatatagcccattttatattcctcaattaaaagctgtttcatttcggcagtacaacctgaccaatctattgtactggctgaaattccttcatcacagacatcgatatttcgccaggactttttaacaatcatattctcaccacttgggataataattccagcattttccgaccgacggatgaagtttgtatcaatacccatacaaccaggttcataaagggccattaccagccctccataggaaattccagatatacttgagcattaacacggatttcattagtaatctttttaacacggtcggtattacgagagacacgaccaaaccagcgccaaccgttacttactgcacgagaacctgtatgccacgtctgccaatcaaactggagcaacgtgcggtcaggagcatcccacttagttaattcattagactcaattttttccagaacttctttatgccactggcgatagataagttcgccttcaggaatctgactgaactgtgcagttccggttgcaaaatgagtaggacacacatcagcgttaacaagaccaagaatatgttcagaatggtatcgaggattatcataatcaggttgccctgcagtaataaagtgttggcccaccggaatatccgtgcgtggtacatcatcatggtggaagcctggaattgcagggtaccagccaggcattaacatgtgtacacgggaatcaaatactacatccgagtctttccaatcgtcaggaagattttggataaagctacgagtaattgggccgccattatcaaaagcaaaattcaaatcgcagttaaagaacataggctcgtttttaatctggtcgtttttaattgcatgagcaaaaccgcctactgcacgagcttgactattaaacactttagaactattcataatattttcctcacttactttttgttgaaaaagtacattttacctttaggggataaggatacacgaagtgcgttaccaataccaactgaacatttaaccaggtcagcagatttcaattcaccaaatgcttgacgaaggtcaccatcacgagtgttaaccatcaggcatttagcaccagctgcacgaacttcgtttaacatgttgattgcttggttagaaagtttcattttattctccatttcactctgttgttttgataggtctatagtatcacacctatagaccttgtacactgttttgtgcaattatttttcgaaaggacgaattaaatgttggttacgcttaaaccgttcaatgtagtcgttttcacctaaagtcttgtacatattaaccacagcttggtagttttcccatgcataagtgcggaaccaacctgaagtgattgaggtgcacactttctcaagggccatatagaaacttaatgatggtgaaatattgaagtcattaggaacctgtgaacgttctagtgccaggacacaagtttcttcatacacaccagccagtttaatagcttcaggcaaagcctcgaacttctcacgagaggtcatgacttcagaaccttccttcatataaaaggtatatgcagggcgccctgccaatgccactgcttcatggatagagtcgtggtctagggtataaatggtatcattaaagaacgatgatttgtttacatccaatttagggtgggaatagctcaacgtttctttttgacgttgcaacataatttcctggagttcttcgttaagggtgatacctttattacgaaggtatttgatgtgggacatggttttcaagaagaacggattattcttcaagaaacgatgggaggttttgatagccagacagatatcaggggttgcccaatagaaacctgtaagacggtcctttttaatatgattttcagcatatttcagaagacgataacttgaggtgaaatcttcatcttggagctcaccggtgatttctcgtacgttagtcagagcacgaacgatatatgcttcaaaataggtttctttaccgttgtacatgcatttaaaagcctggacatcaggattatccacaggaacatgggcaccaaacatccgagctttaaagtgattccatgagccttggtcggcaatgaaatcccaatcagaattttcgatatgcttactttcaatcagaccagcgtggtgcagtgcacgagaaccaataactaacatcataatattttcctcagtaaacttaaatttcagcgacgtaatcgttatgcaattcccacatatcatcagaattattcttaatgataggaattatctcattagagatttcttcagcataaaggtcattgatacagtgggcatcttcaaaacgaacaccgtaatcagacttcttataagagaagccataaatctttttaaacttggctcgagtaatgcgtaccggttcattagacttatcggacatcggagcgtaataccacatatgttctcctcatgtttgtgtagggtaatagtaacatgattttctagagttgtacatcacttctgcaatattctaaaaataatttatcattgtctactgtatcccaacgacgccaagacgggttccagaccaaagcgttgtcaccacaatcattgagcttaaaatggtcgtagtacatagctatgtgtctagtctcgtcaccagagaaccccagtataggcccaccgcgggtgtgatacatatgatggtgcattgagaggtcgcatttgtaaaacatctcacgtttaccacgaacgaacaagaaggcctgtccattcatatagaattctttatttgttttcaaaagatatttgaatactgaatctttatgcataagtcctcctaccacatccatgtggttaaattattttcctaacgaaatacgagtaggttttttaccgaaatagtcttcataagaaccatctaaacgacctgctttagaccgacaatatgaatcgtactttttgtaataagtcatctcagtattataacgcgggtgtctatcagccataataatacttaacggccaacctttggcataatcgcgaagaccatttattttacgaatgtatcttttctttaattttagcatgagctcggataccagattttaccatcggcctgagcaacgaaggtgcgaccagcttcttcgccataacacgagctattcagccaatcttcgagacgaacttcaccgtcataatcgtcgagctcaacaccaaaactttgagcagaagccatatcttttactttcttatacagtgcagccagttcaagtgcagctttttctaattcattaatatcagacattttttatcaccttagcaagacatagaggacgtaaaccagaaaccttcaccttccggaataccgtagtcatcacggacccattcgtaatcatcatattccgggttctttggagaaatgtattctccacgaccagaaacacgaaactcttcacccgtttcgtcagccacagactggcctttacgtactaattcacggatttggttttcaatttcatcaatagtcattttatttccttaacattcagaagaagaggacacccaaccaccattttctaggctggtagtgtaatcatgttggtttacaatagcgtactgagcttcaccgtattcttcccagtgggcaaggtcggctttcaaggcgccaggagaataatagtcaccgcccataccgcgagcagggtatatattaaaatgagtctcatatttgtttgcaatttcctcggcacgacgaatagctttatggatatcatttactgcttcagccaattctttatttttatggtaatcattcatcataaaatttccttagcacattgccgaagaggagatccaagcaccaactgtaacgacgccattttcaacttcaccaccgttgttttcaatttcatctttaaaccactgggagcattcataaccgacaggataatatgtacggcctgaaccataatcaccagtaccgaattggataccatacttatcggcaatagcttcacattcatgttcgatggtattcactttattcagaagagcatagatagccttttctgcagatttctcgtcattgtgttccgggatttcaatttcaattttattcatgatttacattccttaataaaggtttcaaggtcattacgtttagtttgttttacatactcattataattagccatagctaaagcatatctctttttacgtggcttgtttattttattagtttgggcaatatcaaagacccatgggataaaaaatcctattaaagccggaacccaaatccacgcgaggctcatatcttcaaacggatggcgaggcataccattaataatcccaccgacaagaaatccaattatccctgcagtcatactagtagcaatgccgaggaataatgaaatagagatatcgtaatctgctaatgcgtaaccagggtcggttttactaggcttatgcattttgaacctctttagcgtattcgcgacattcagcaataaaacgattaagcttacgttgttgtttacgactttctaatgtgtactcattagccaaaataataagctcatctttatcgtaatttttaatatcagagtaagatgggcgacggtcgaccataccaaaatggtcaccattttctaacatcaaatagcatactaaatggtaatcatcgtcggcattagtaagctgtttataatcgcttggttcatttaaagagtatactgaatagcgtagcccagcgaattccactcgttgaatagccagatttacgtcaataatttccaaagcatcttcaaaagaaaggtcttcagctaaagcaaaaataaaaggtaatttggtagtatcgccacggctagatgttctgcttaagaaatcgtttgaatagcctaggtcttggcgaattctataaagaactgaattggtttcatgggaaagaccactatttttaaaccaatcaatatttgatatcaggtcgtcatataaactcataatattctcctctcctccaaatagggagaccgaagtctcccggtaacattacttaagtgaattaatgtagtcttcgatatcagcagaagtcgtatccattccaacttgcgggcctttaaacgtttctacgcgcatcagggtgtcttcgatatcaatcttggtcagtgcagcgatttcaacaacatcgtcggcagtagcaataccaagggcagccatattacgagtttcacggatgtactcgagcttaacagccagttcctgacgagagtcatcaagttccttaaccttcagtttaatttcattacgcatttcgatataatcatcggctttcttacgaagctgggtagctgtacgacgataaaggaggccaagtttagcatgtacctggacatcagcgccttcggcaatcagtttacgaatttcacgttctttagaagcagcgagctggtctttttcattagccaatgcacgaatacgtttttcttcattcacagacttaacatgagcagtctggagttcagtgattttatcaatcagagtagaagcagctttggtgtattggtcttcgattgacaggttctgagtcatcgcggtacccagtttagaacggatgaattcaacgattttctttaaagtgttcatagtatttccttcagttgattaagatttataatccatgaggacattataccctgtcctctgaggtttgtaaacattttatttcatttttgcgaggcaaatttcattggcttcccattgagcttgcttaataatagctttggatacaggagccctttggccataagtttttgacgttgagagaacaatatgtttgtttgcttcattatgccagccccatgatttttcgccatgagtacctttaactacagctgacacctcaacagagcaaccaccatcagaaatcttggtttcgacaacccattcatttctctcagcagcttcaatttctaatctagttttttcttcatacatcgcggcccaatcagtttttgccaagttgaaagtaagagctttctctagttctttggcatatttttgttgttcaggtgttaatgaattatacaactcttgcatttctttatcttcgatattcattatgttctcctcaaattatgggctcataatatcttaatcatgagcccatgtaaacgttttatttcatattattgaaataattttctgcatcaaaatcattaccatggtaaactttggtagacgatttggcgtaaccttcagctgagaacatattaatcacaactttaattgtataccactgtccatcttcattacccattactgcataggtttcatacaccgggtgttcaggaccgataactttaatatcgttaacagtagcaccaaattcttcaggaacgcatttcataaagaaattaaacacttcaccataattatccattttactctccttcacactgttgttttgataggtctatagtatcatgttctacgaaagagtaaacatctttttttaaactttttagaaacaaaaaaggcccaacctttcggaagggcctagaatcagttcttgtagaaccggaatgggtttatgtggaaggctaacatagccttagggattttacgagacaaaagactcttaagtttccaaccacagtatacacgaaggtaaaaggtaatcccacccactttaagatacggaactgaagcaaagactccccatgcttcgtcattccacatccataaccatccatgatgagctttatcaggagaaccggattcaacgtcaggattaccacgataatggaattctgagctacaatcgcgtccaagtttatggtaagcaaagttataagctttatttcgccatagccaagctaccctctggagataaacaccgcccggcattttcctgattttagcccaacgtttaatatgacctttgtcaccgtcaattggattatcgtatgtcatcatccaatcaaagccataaggcaatttaccggtctttttattatggaaaggaactacaaaaggcgcaaggataacggccagaaccatagagatgaaatccagtggaaccaacagaacccaactcaaatattttaaaagtttcatatatttctctaagttaaccaaaaaagccccagacggggctttcgttatttgatttgtttagcagaccagatacggtctttgatgattttctgaatatcttcaacatactctaagtcgtgagcatgtggattatctttgaagctatgtgctcgtgccagtttctggccttctgttttgattactaaaagctctttaagaattgcttcatacttagaaataattcctttggcgatatttttttcttgagcggctttagggtccgcttttgacgcaggtgctttacctgtagctttctggaacaattcacctgatgcagctaggcttttaaaaactcggctaacagtattggcattagtaaaaccttcggctttaaaatctttaataaaacggaaacgttcttcatcagaggcgtctttgtaagaatatttacctgcttgaattgctgcaatcgcagcggcttttacatctgaactagattgttcagtcaaaaattcattgtaagttttcatattatttcctaagttagtttactacatatttatacaaaaaaagcccaacctttcggaagggcctttaacctagggtaaccttgtcggggttccacctgctaggcaagtgtttgtacgaaacgccgggattcgaacccggttattaagtagttgacgccactcaatattttttaaaaggccatatctcgaccatatccgaacgttccgtcaaaaacgctactcggcttacggcaaagatatttcctcgaatcgataattcggtgcgccgtttctgctgtgatgtaaggggacgttaacagatcgtaaagatttgttaatgccagtccttactcagggaacatcagtccgacgacttaccggtagcgacccggtttcttgtttgttgcgccggtgaatgctggtaatcagtcttcatacgacggcttgactatataatagtcttcatttggtatcccgccctgggatcgaaccaggaccgcaaacttagaaggatcgtatgctatccattacaccagcgggacgtagttggtgacccagaccagatttgaactggtaacctttcccttatgaggggactgctgctaaccattgagctacagggccttaaatcaaactacaaatccagcaggagcattatcatctttagccatgtgctgaattgtatgataagtcatttcttcaggagcaaccagataagccgcagcgttaactagtggaattatttttggtttagcgaatgtgctatcggcaattgccataaagggctcgccatcagtctcaacttcgccaaattgacattcatatgaaatagaacaacgtttggtagttgttgtcttggtttctgggtcgtaaaaagctaattttaatactaacataaacacctcaaataaaattaagtaaagtaagtttgattaatagaccttgtctattatgaaaggttctttgagggaagaacctttggtaatagagggtattaatgatagagtaataataacacattactcttaaagcatattactatttttaggaatagtctggtcaaatttgattcattgtggccacatattaatgtaatcaagtttaatagaagcaatcttcaaaggatttttaaagatgtcgtattcgatcaatccgttttcagttgcggtgtagaaagtaaagttaacagaattataacggcgaccattaacttttagtttaacgtcgcttgaactacgaccaatattaacctgttggacatcaagcacagcacctttgccaaagttgcgaatcagtagctctgctgcaacctggtctgaattatagccattctctggattagtaaccttaacgtatagcatttaaccctcgtctacaatagtatgggtgttggcattaacaatctgccaccattcaaagcgactggaatcataaaacgttttgttttcattttctttaataatttcgcgcagttcatcttcagtcgcagcttttgcgattaaatcagaatatccaccgcgagggtaataattaacaccagcaaagagcaaaaagtttgttttgatattcttgaattcttcaagtgtaataacggacccattgggttgaacaatatccacataactataccctaattcctgggctttatctaccgcctcaagcagggtgtcgtgtgcccacccaatttgacaatctgggttttcagatggatttgcctgataatctgcatacactttatacattttactcacctttagagattttatccataacaaaagaaattgaaccaattaaaaatgccactactaaagagattatattctcggaagttgaaagcatatcgagcatgaatcctgcaaacatactaaagccaaaagcagtaacggcgaccagtgcagtaacatttctaattaattcacaacgtttcattttattctccaatcactcatttgttttgatagggctatagtatcacggctatccaggaaagtaaacaccttttgtttagatacaaaaaggagctttgtggctccttatctgtacttagggaagttttttaacttcagcattgaattcacgggtaagaccaatcataccgtggtaaacttctttaaagaccttgtcatttaacgcgtccagttttttagccagatccgagaaaggtttcttttgctctttatcaagggtctttgtaaatttagccaggtcggacttagcttgacggatgaaatcaccaagcccgttagccatatctgaagctgcatcaaaagatgtttcaatatggtagtactcagtaccgccagctttagccggtttagggatggctacttcattaattgcttcagtttgtacaaattcgttatatgttttcattttgttcctattttaggtcttcagcccagtcgagcttcaagggttctttatattctctgtctaaaacaacaggaatctggacatctccactaaagctaagtggtcctacattataagacagggtgatatgaggggtgtaatcatcaaaatcgtgcgtagcacctaaggtacgagcatactgatggcggcatttaagatactctgaattgagaaccaaaaccaggacaggagaatcaccgtgtttccacacttcaagatgtcctgacgaagcaacttcaaaacttccggatgcaacggtgtatggaacgttgactcttgaatagcagattgtagaatggaatttttcacgaggaactggattaggaacctttaaagtgcgctgaagattttccagcgcatctaaagttaattcagagaattttgcagcaacgtatagaccttgagcaaaatcttcggttttcattattcttcttcagaatattcttcgtcagaagcttctggaaccagggctttaacggcttcaaccaggtcttcgattttaacagaatcaccggtaacgccaactactgcagcaatctcacccagtactttagtaagcatatcacaatcagctttaacacgctgtgcatggtcctgagtatcaaggatacgagatttcaggataacgatttcagactgcagtttctgttcaacggtttgttcagacatttttatttcctaataatttatcaatagtggtgtatagttcagaaagagtgccgttattttcaacaacaacgtcaccaggtaaaattggtagacccgcttcagtgatgtgcgagtcttgtacttgaccggtttcagcgcgaactacatgaataatcgtagcacccatcgctctgagcgaatcaatttcgtgtgtttgacgaacatcaggtacgacatagtatttcacatcagagtatattttatcaaaatagtctaaagcgaacaacttaacccaatacatcttatcaaattggttaacaataatatcagtcccaagggtctgcatgagacgacgtactgaccaattgttatttttatttattacttcaaacagttggtcttttgtttcttcagacagatactggactggggtaagaccataatgatatgcggtacgaacgtccattcctggaataggaaggatattattcagtttgacaatagcattttcaaagatatcaatcacatcatatggttttaaaggaatgatttcttcacggtcgtaaccgataccttcaaaacagttaaaatctagtttaggcatgtaactacggtcgaatacagggtcatcagagatgtattcataggcttcagccagatactttttaataggacctgcgagctgaaattttaccgaatccatattttcgattacatagttagcaacggtatccttaccgctacgtttgattcctacaattgatattagtttcattattttctcatagatggatgcatagacatacgagccactcgttgttcggcatacgaatcaatttgtggacgacctgtaactattgtaccatctatttctacagcaaacgatttgaagttgaatgttgctgtggcgataatcgccgggtcagaatcctctttataagagtactggatttccgagaggtcggatggccaaccaccgtagtaatgaatgctcattacgattttctgtttgttgttatcaaggatgtggagggtgatagcttccggttgacctttaggatgccaggcttctgaatcatgggttacatagttgtttaatgacaacatccacttataaacgtcaagccacgatttcaattcacggtccacaagaaagttcacaatcaatgggtcgaattctacagtagaacctggcagcttagcacgatgtatgccctgggtcgatcctgggacgtctgagaccggaatatggatacccggtagtgttacatcttgtacgttcaatttgaatgcctgtgtcattcctgcgtcactaacctctaagataaagttagtagtgttagtttggttaaataaaccgttcatagggttcctatattgcttaagtcccagacagtgtataatggtcctaggtctgttccattcaataactggctgggataatagattattttataaattcacgtagtcttactggtgtcataaaaggccatttggctatagttggttttatccagtatctttcgtggcatgtagctttaaatgcccgaaccatatccttggcctcttctatagtatccacaccaaattgttcacaagtttcctttctggctttatcccatctccgtttagaaagctccgcttggagttctttattggcaaaatggccattattcctatcatgagtggttccttttgtaggactccatcctcgtccctttacaaatccttcaggaatcggttcacccggaaacagcttaatacacttcttgccattattataataaacctttcctgtttgggttgctgtgatattctcagagtgcttacgtttaagccaaccgtaaagcttattagaacgacgagggccttgagtcattgtcatagctgcaaaagttagaccaggatgtcccggatgcattttaactaatagttgatgtgctaaataatgttcttcaggagttaaatcaactaagtttgtagattcatcgcctccacccatacatctaggtaaaatatgatgagattctgtataacaggatagtgctcgtccttgagcacgtgtaattaatgaagaatatattttctggtaattcattatgccttcttccaaactttctgagctgagtaacgcttgcctttagatacaaattgttgaagtggtaatcctattacattagcccaatcagacggttttatctctactaaaggtcccttaatatttccagggatataagccttaatcatcacgtcggctccggcgaatccttttaccttgctccaatcaatttttaatttagtcgagttcgtaatggtaggcgtactcgcgtattgcttcagcaattcttccagaaattgctgtcgtgctttaggtggaatatagtgtaagttcagtccatacattaaattatgcttacctagcccaagataaatgattaatggatatttgtcccagtacggtagggtatccttatgtttggcatcatagatatacgcataaagcttaccaggagatggtttagatacctggtgcccacgaattcctttctttaatgtttctgtaaaccatttagccgatttattgtttacagcggcgccctcgttagcaatcttatcacgaatactctttctaaaactattcaccaaaattaattgacgttctgctttggttaatttattgccaggtttcttctgaagtttttcaacctgtacagcagttttaattcgactcgagtatcgagacatcgcagatgtaaagctagaatacttgatgcctttatcttcagcgaatttcttagccgaaacacctttagccttagcgttggcatattcaacgcctaaagttatccattgttgttctgaacgagtaggcttggaaccttttgtagtttcagtagcctcgttgatgtaagaaaatatactcatcctttccatcctaattttttcagtgagttttcggtaatcaatctgaaattaattcccattttatctgctgtagctttagcagctttccatttatctttatttacactccatgtataatgttcgttgatatatctctttttagcagctgtagtcattttagcaggcgccgctggaggatgagtctctttaaaaggtttgacttcgaaaaagaattgttgaccattgtcgaacttcacccagaagtccataaaataccgacgtttctttccatcagcgttactaaaatatggaataacaacctcttccgagttccactggacgacattaggatggttgtcaagccaacgcataagccatgcttcccaagaggaacgatattggattttcttccaatcacctttatatttttgtaagtttgtaggtttaaatttccctgagtaggccatagtgcctccttataaatattaatattatttatactcggaggcactatgctcttctcatttttcgatcctatcaattatgaatcaaaaacagtcaagccggattcgggctcattaactgatgccgatgtactgagcgtaccgatgactgatatatttagaaactataaagaatattttgataaagtggctaaaaattatacacttaaaacatattatatcagtggggcccctcgtccagaagaattagcccatcaactttatggtaacgtgcaattatattgggtccttttaatgtgtaacaatatctatgacccttattacggctggattacaggccaagaatctgcgtatcaagcagctattcaacgttatgctactgcaggcggaaaccaagtcctttatcatgtcaatgaaaagggtgagaaattctggaatctagtaaatactccggaaaatccttatacttggtacgataaaggtgatacagaaaaacgttatcctcaatatgaaggtcctttggctgcagtagatatttacgaggacgccattcgtaaaaatgaatataagcgcgaaataaagattatagaccctaatgacatcgagtcctttgtttccgctttaattagagaaatggaaaaagcgctatgattaacatgtctgataatgtaagttggttcgtcggtgtagttgaagaccgaatggacccactccaacaaggccgagtacgcgtgcgcgtatggggtatgcatccatatgaaaaagtacaaggccctgtaaaaggccttcgtacagaagatttaccatggatgtcggtattaatgcctacatcttctgcctctgtttcaggtatccaaaccgctatgactggtatggtccccggtacacaagtttatggtcactttcttgataagtggaaattaaacggacttgtccttggtacatacggttccgcttcaagacagaaggctaatcctaatgaagggtttagtgaccctacaggccaatatccgctttatttaggtaacgatgctgctgctttaaaccgaggtggtgaagttggatacgatgccacttctaacgtaatacaagatgcaaacactgatgtaggtattaatcctgacgggttggatttaagtcaagtcaaaccagacgataatcctaatttcacaatagaaaacatgcttcatcgtgatgaagggcttagactgaaggtatattgggataccgaaggttatcctactataggtataggccaccttatcacaccacaacctattagagatatgaatcgaataaacaaaatattatctaatcaggtaggacgagaagttaaaggtaaccctggtgcaatatcaatggatgaggcttctaaattattccaagaagaccttaaaaaagtccaaaacgatataggtcggcatagtgttgtaggtcctgtttacaataaagaaaaccgttcaagacaaatggctcttgaaaacatggctttccaaatgggattaggtggattggctaaattccgtggaatgcttagtgcaatgctaataggcgattataaaaaggcatttgaggaagctcgtaattcagtatggtttaaccaaactaaaggtcgcgcatcaagggtgtcaatgattatcctcacaggtaacatggaatcatatggtattatggcccctaaagaaaggtcatttaatggccgttcgtatagaatgattcaaacctttgtggcccctacaaattcagaccctgccgacccgtggactccagaagacacaaggattctttttaaagaacctgattctagttataaaggcgaatatccatatgtccaaaccatgcaaactgaaggcgggcatatccaagaattcgataataccccagggcaagaacgataccgtttaatccatcctaccggtagttatgaagaagttgctcctgatggacgtaaaacttctaagacggtagccgatggttattatatgacccaaggcgattcaaatacttatgttggtggtaataataaagtcaacgttggcggtgatgaaacctattataatatggctaacgttcgccgtcagaccgatggaaacgaaaccatccatattcgtggtaacgaagagaaaactgtagaaggtaatggaacccttcgtgttaaaggtaatgtcaccgttattgttgaaggaaatgctgacgttactgttaatggggatgcgactacaatgatagaaggcaacgaaactcgcacaactaatggtaatttaaattggactgtaaatggtaccgtatcgtggacttgtgcaggtgcttggtccgagactatggcttcaatgagttctattgcatctggacaatatactattgatggttcgaggattgacattggctaatattttacctatgagcactgatttaggagactccatggaaggggcctcaatcgatgttacgtttaccgctcaattagaaacaaacgaaacattagttgaaataaatataacagaatatgagcctacagaaggcattattgtcgatggagctcatttatatggaacctacgaatcggtatttgggttctctgaagatgccttgaaatatcgattaaacgatgaatttaaaacagcaggttcatggaaagacctaccggccgacagtaacactcaattatacctctggaaagcccctagtaatctccagaagacgttttcttacacagtcacaataatctatgactttcaagaagagtcgtcaggaggtgatacagggaactcaggcggcagtaattctagggccggtagcgaaatagaccctcctccggctcctgtaagaaaaacccttactaaggtttataccaaggttattgtcggtaattggtccaaatgggcaaatcaattaagagaatacgtatatgcgaggccataaatgtcaggcttaagttataaccaatgcgtaacagcaggtcatgaagcgtggcctcctacagtaataaatgccactcaaggtaaagtatttacaggtggtattcctgtgttagttgacggggaccctattacagaacacacagaaattaaaaaaccatatgaaacccatggtggggtaacccaacctagaacatcaaaggtgtatgttacaggcaaaaaggctgtccagatggcagaccctatttcgtgcggagatacagtcgcacaagcctcatctaaagtattcataaaataggaattaaaatggctactcctacgaattaccaattaacaagaaccgttaacgctatcccaaaagtatttgtgggagctacgtttgaagagattaaaaagaatattatcgattggctttctagccaggacgaatttaaggattacgatttcgttggttcgcgaatgaatatcctgattgacatgttagcttacaacaccctgtatatgcagcagtttgctaataccgcggtatatgaatctttcatcggtactgctaacttgcgttcctccgtcgtccaggctgcacaggataacggctatttgccaagttctaaatcagcagccaaaacaagtatcatgttgacctgtacccaagccctgaatgaaaagaatattcgtatcccacgtggtactaaattcttggcctatgcccgtgatacttcagcagacccgtatgcttttgttaccacggaaaacgttattgccgtacgtgatgttaataaccaatatcttcctatcgtatctttagcacaaggtcgtattatccgtactgaacttaagtatgaccctaaaactcctattcttattcgtgacccggatattgatagacaggaagttaaactttatgtcgatggcgcagaatggactaactggactaataaatccatggttcatgctggtagtacatcaacaatttactatatgcgtgaaaccgtagatggtaatactgaattcttctttggtgaaggtgttgctgaaaaatcagttgcaggtggggtattagaagctaattatattggtggtttaaaacctgttaaagatgctaccattgttatagaataccttcgtacagatggtgaagttgctaacggggcagtggactttagttatgcggattctttggcatatattacggttgaaaaaattacagaaaactacgatgaaaacccggattatgtaggtgctgacggtggtggtgaccctgaagatattgaacgtattcgtgaacttgctgtagttaaacgtgaagcccagatgcgtgctgtaaccggtacagattatgatacattcgtttcggagcgatttggttctattgtacaagcagtacaaacctttacagacccaaataaaccaggttacgcctttgttaccattaaacctaaatcaggattgtatttgacggcagtacaacgtgaagatatccaaaattatctttcagaatttaacttggcacctattaccccttcggttatttctcctgactacttgttcttgaagcataaaattaaggtttcatatgcactgaacaaattacaggaatccgaacaatggctaacggctcaaatcctttcccaaatagaccgttattatattaacgaagttgaaatattcaaccatggatttgccaagtctaaaatgttgacttatattgataatgcagaccacagtatccttggctcttcggctacggtaacaatggttcgcgaagtattaaacttcttcaaaacacctgaagcaggtattaaatactataatcaatacaccaaccgttctgtaacttctagtgaatttgagttcgtcccaacaaacgtatctgatgttgttaaatcttacaacgtacgtattgttgccacagataaagacgaacgaggcgatggtaaaatggttataggtcctttccgacctggcgatgtaattgaaaaccaatacatccaaccttacaccggagatgacttcgataaaatggcagcgcctgcagaccaatcggtctactatgttattggcgaaattgattattactcggactttattttctgggatatcgccgcaataggccttacttccgaccgttttgaagtccagtctattgaactttatgcagggccagaccaagacaacatctttaccaaagacggttctttaatcgtatttgaagatgaccttcgtcctcagtacacaactatagagttggaaccaattacaatataagcctcttcggaggtttaaggagatttaatgtctgtacaagcgccttatgttactagtctgagaattgataaactctcggctaaccatgtgagcattctttgggatgacgtaggcgccaacttctattatttcgtagaactggcccaaacgaaggatgcgggtgtagaaattcccgacgatagattattttggagaaatttaggttacacccctaataacgaatggtttgaagaggcattcatttctcctaattcattttataaaatgcgagttgcagtggccgcccaggggtttgagcagtccgaatgggtttacactgaagaatttgaaactttctctaccaacgcatatacatttgagcatatgcgcgaattcactttgtctaataaatttattgaagaaaaattcacaaaaaataatcagaattatgtgaactttaataccgatgccattatggcttccttaatgacggaagattttaactttacgcctgcatattcgcatttgtcatctatatcaaattatgttttaaaagccgaccgattccatgaaatccaaggaagcatccaagcggtttgtaaagaccctaaacgttctattttaatggaacttggtggtgtactttaccttttagaaagattccaaagtaccgctaaggtttctaatgataaagggcagaactggcattatatccgtttgtttaatgaccgagtaggtaaccctgtttcacgtacggtacattaccaaactgaaactactacgtatgttctaggttatgaccaaatattttacggacgtaaatcaagtgatattcgttggtctgctgacgatgtccgttttagctcccaagatataacatttgctaaaataggtagtgatatcgaccttccatttgaaatcgagatatttggttcttatgcaaaacttcctttgcctatttccactattgctgaatctatatgcgcttctgacgatttcatttatgttgcaggtagagacagagtttataaagcaaaaacatctgaggctcctatagacaccgaccctagttctccgacttatggagagaagatatttgaaagcggatattcaactatcacagggaaccctaaagcagtttgttataaattagattctatccaaggccatacatttgctttaattacaggtgaagttaaagaagaaaaaatggaccctacggtcgaatccaatgtggttgattctgaatccaaaggtgtttattggttagacacttcaactgatacatggactcgggtatttggaaacaccgaagaagaacgtcgtcgtatagagcatgggtataccagcatgtctaccgacggagaggaattatttttcagttcaagcaactttagatatgaagtagaggttgattctgagcttcctttggaataccctgaaattgtcacctccgccgttaaatatgttaaagatgaacaatggattcacgataaacattatttgatgatgagttttaggtctaactctaaatctgatttcaaagaatttaaacctgggcgtatggcttattatgccgaaccattctttagttggtcccgtcgtgatggaacccgttcgtggattactactagcgaccatgcgatggttgtttataatgatgctttataccagaaaattatcgatctgaacagtggttcttcacctgaacgtattgttcatgagatttggaataaaggtttttgtaaagtcacatctcctaatatagagttcaacggctttaagaaatattcttccggaatgatgattcacaaatctacaggtgaattggttggatattttgaatttgactatcgcgtgcgtgatgaagtccgtgttatttggaagcctaaagaaattatgtttacggctgaattgcaaaaccaagaacatgaaatcccgtggaaacctaaagaggaagttggtgagcaagaccctgacctccagcctttactggttaaaatgattccagatagttatttgcttcaagatagcaactttgaaaaattctgtgaatactatctccaatttattagtgatggctcaggtacacactataataatttgttgaatcttattcgtaaccaatacccacgtgaagaagattcatgggaatatttgtggtcggaaatctataagcgtaatatctatttgtcgaaagaaaaacgcgacgaagtagttcgttttttccaggcgcgccaaactgatttttggtctacaaaaggtaccgaagcttcatataaattcctgtttaaattgctttacaacgaagatgtcgaaattgatatcgagtccaagaactctatcgaatatgatatcatcgtagaatccgacaatatcagtgaagatatcgtaggccaaacgatttatactcctacaggaagaagtaatgttacttatatagaacgaaattataaagatggtaaactgcaatggcgtttaaccattcataatcttttaggtcgttttatagtcggacaggaaattaaatctgaacgtacttcgttcaagggtatgattgttcagggcgtacgtggtaaagagcttttgagtaacaatatcgactatatcaaccgtaaccgttcttattatgtgatgactattaagtctaatctccctacctctcgttatcgcaacgatgttttgagatttgttcatccagtaggtttcggctttgtaggtataactttgctttctatgttcgttaacgtaggtttaacgctaaaacatacagaaactattattaatatccttaagaactataaatgggactcgggtttgccatctgaatggtatgatagagttgctgtaataggttttgatggtaatatagaacgagaccctagaacaggacttccggtttataacgttggacctaaagcaggagaaccgtttgatattcctgctgattatgatgcagaaaatgatttctctgtattccaaggtcaattaccacacgaacgtattaaaaagcatagtccattgtttgaccaaagtgctgtgacctttgccaattggcgtgcactggttgataagcgtcttaaagacgatattggaaatcctagagaccctaaagttccaactcaggtaaaaattaatgattaattctacagtagtttatcgttctattgttacttcaaaatttagaacggaaaaaatgtacaacttttacagaacaataggtgatggcgaagaccagaacactatgtatgtatctttcggaagggcccgaccatgggccgataacgaaaatgaccctggttttgctccgccttatcctgtagatgattctgagggcgtagaagacgtctggaccaacatgatgggttgtgttaaggtttataagagtatgttggattgtgttgttcctcgcaaagactggggcgatacctcttatcctaatccgtttactttccagattggtgaaattgtagtggcgaacagccagccgcaaaaccgtactgatgtcggtgccgggtggatggtttatcgttgtgtagatatcccagaatcaggtacatgttctattttgtcccttgataataaaaccgagtgtattaaacttggcggtaaatggacttcaaatgtacagtcggttaaagcccctgcaggacaaggcgatacggaaggtatggttgatacaggtgatggatatctctgggaatatttgtatgagattccacctgatgtaagtatcaaccgttgcactaatgaatatattgtggttccatggccagaagaaattgccgaagacccagaacgttggggatacgagaataacctaacttggcagcaagacgattatggattgatttatcgtattaaaggcaataccattcgttttaaagcattcttagattcagtttacttccctgaatttagtcttcctggtaacaaaggatttagacagctttcgataatctctaatccattagaagctaaagctcacccatccgatccgatcattaaagccgaaaaagagtactatgatgttatagacctctcccgccattccggtgaaatgatttatatggaaaaccgtcctccggttattcgttccatggaccaaacagaagaaattaatattatcttcgaattctaataagggccgcaaggccctttcgggtttaataaatacagtatatcaataatgaggcatacctatgattaagcaaactggtaaagaactaattgacgtcggtgaaattggtaatgccagcaccggcgacattctttatgatggcggtgttaaactgaacactgacttaaacaacatctataatactttcggcgaccaacgcaaaactgctttaaccggtgaattaaccggtcagaaattacacgctacaggttattatcaaaaatttggtgatatggaccaagcaagctcagtagatttaggctctttggtggatatcgatgcttctaccggttctatcgtgttaaccactgtaaaaggtgcggtcggtgaaggtattgaaataattaactctaatggaagtatttcagctaccaactatcttgaaatccgtatattggattcgtttttgaaccatcctacatcggccttaagaatagtaactccttatacacgagttcttttatggtgtgtatcagatacaaacggcattgcggtatgggattattcaattgaaagtatgtttggtgataaacgagttccattaaataagacatataatatatcttctgtcgctcgtgatattccggtggtttattccggccagtattcattggtcaaacttttagttacggcagtgaatgccaacgaaaccatttacaaagcttcagaataccttgtgtttatcgacaaccaagctagaaagatttattccaccgaatacgctgttattaaacgtggacaaacttcagatgatgacgaaatttattccctagattttaaattcgatacatcaaactatattatcgcgaccgcttcttctgtcaatcctatgaggcttgcaattaaggtcgtagaaacccaaactattggagttccagtataatgaaacaagacttaaaagtaggttccgctgttgatgacgggtccggtgattacctgcgtgcaggtggtcttaaaattaataacaacttcaatgagctttattaccaattaggtgatggcaacaacccacatgcagcaggcgcttggaaacagcattctactgcagatggtgctttgttgaacgctgtaatgggtcatagctatacccttaatactcaaggtgggcgtattaacgttcagcttcctaaaggctcccctgaagaatataactttgttatccgtgtacgtgacgtgtattcctcatggcaagctaaccctgtaaccctaatccctgccacaggtgataccattaagggttcagctactcaagtagaaattgctcgcaacttctctgaccttgaattagtttattgtgccccaggacgttgggaatatgttgaaaataagcaagtaaaccgtattccaaataacgacctcgctactgtagcaactaagcagtttattgccactgaaggtcaaacagactttctagacattttcccagggctttcttataacgtagcaagtttaagcgtttcgcaacgtggtaacaatttgttctacggtattgatgatatttttgatgcggctactgcagagttcggttctccgggtgctcaaccaggtgaattggttgccttgaatggtaaagacatccgtttaaaatatccttgtgaagcaggtgatactgttattatcaaatcatataatgacgggcttgctcaatggcgcagttcttataaccgccgtgatataacaatccaaagttcagaattgactaaaaacgtttctgttcctggttcttctttcgtggctgatttgaatacttcgcatgttatatcggccgcagatttgaatatttctgttaacagccctatcaacccaaatgcttgtcaagtcatgcttaatagcacattacttcatcaagcgggtacagcaggacttccttcgttttattgtgaaggtgctgatggtcgtactgctaccgagtgttttaatgctggtggtcaatggacccaatccaaatcagactatatttttaatttgactcctgaagacaagattgaatccatcgaatttggacgtaactttgaacatggcgatattcttacagtaatttggtacaataatgatatcggtactaccatggaaattgatgagattttggattataccaacaacatctatatttctaaaggtccatcgattgatataacagggcaggttcgtattactgatgtagataatccttttgcacctaacgttgaaccggtcgccgcgtccaatattacaatagatacagcagcaacgttttttgatttggtttatccaataggaaccatctatgagaatacggtgaaccctaataaccctaaaacttatatgggctttggttcatggaagcgtttatctgatgtgttcttggtaggttggtctcctgacgctagttctttgtttaatgcaaataacaacgatctggattctgccggtattccacagtcaactgctggcggtactggtggcgctcatgtggctaatttgaaatatgagaatatccctgaacttaataccgatgataaagtccttattgctgataacgatggccctatttttgtaggtgggtgtttagttgaccctgattcacaaggaccggcttatacaaaatatcgtgaagataaagccagtattaataaggctcaaggaaccactcctatcccggttaatactctaccaccatacttaactgttcatcgctggatgaggattgcataatgactttaactgaaatgaaaagcgggttaaaatcccgcttagccgattatttggaattatcttacactagtgacaagcctactgctgtcgctgaccaacgtcctattggtggtccttctgcaaaccaaacccagaagggtgtttattttcctacggtccaaagtgcaatagatgatattgcatttagaacagagcttcctgtgaactctgttattattaccacagaaaacagagcacctggatttatccagcaatctgataaaattacatttaccggttctatttcttcaggcggtgaacttggcgacccggttattattaaagtgttcggacttcctgtagaggtcttagttggcgattcatctgtattggttgcatctaaagtaaatgatgtgtttttagacgctattgctaatagctatattttggccgaaactgctattgatgccttagaccaatctaccttgaatattaaatacaatgactatcagaatcatattttttcaccatataaacaatcgggttgtacaatttcccatactatagtccaacagccaagggctggatacggtaagtgggaatacttaggtaactctacccaatcgttagcaggtggtacagttaacggcacgattcctttatattactataagagattatattaatgtcaacaaacacactaaaacacattagtgataaatcggaattcaaatcattcgaccctactgggtcgaatttcccgcctgatattactaatgttcaagaagcattggcaactatttcattaatcggcgtcacaggtaatgttccttcagctacagaaacgtcccaaggcattattcgtcttgccacaacacaagaagtaatggatggtctggatgcttatagtgcagtgacaccggcaactttaaaagcccgtttagatattcctactcaggcaacagaaacttatgtaggtatcacccgttatgctactaacgctgaagctatagcaggcacagagccccaggctgcaatcgtagcaacttctttgaaagcggtaatggattatacatttgagaaccgtttatcaacagagaacgctacaggcgttatcaagatttcaactacacctgccgcattagctggtaccgatgataccacagcaatgaccccgcttaaagtatctcaggcaattggtgcagcgacggcagcgttaccggtttattctacagcaacgactacaaatgaaggtttagttcgtttagcgaccaatgccgaggttggtaatggaagtctttcggtaggtatcgctatttctccagcaggattagccacattaacttccaccgaagccagaagtggtattattaaactcgctggttgggatatggtatctaatggtaccgaccataccgccgcagttacacctgcttctttgttagctcgtacaggtaataccggacgtattgggttggttcgtttatctactactgtaggccaaggcgatggtaatacggcgctggcttataatgctaacgttatttctacttcaggcggcgaaatatggggtactttaaacgttaatggcgcgttacgtcgtaacggtgttgatgttgttacacacgaccaattatcagatagtgttccggtaggtactatttgtatgtggggtggcaatgaaggtaatatccctggtaaatggcgagcttgtgtaggtgggacttatactggtggtgcatatttaaatgctgttggtgggcgttggggatggtggggtgctattccagatttccgtggattatatcctcgtggcgctaacatggtcggtggatattctgaaggcgaagttaacccgcatattgccggtaaccgaggagaagacggtaaaggtaaagcccgtttaggtaatggtgttggttctttcccgcaatcttccgttcaagcccaagcattacgttatcataaacatgctggtggttttggtgaacatgataactatggcgcttttggtaacaccgctaactccggatatgttggtactcgtaaaggccttgactgggataaccgtagttattataccaacgaaggttttgagaccaccgatccttggaaccgtgatggacataccacattgaatagtgaaggtcttattgccaacgaaacacgtccatggacaatgtccgttctttttattattaaagtagaataagggtaaaaaatgattaacaaattggaacttagtgagttaccatttgttgacggcgtacctgatgctcctcaaaagcgtatccaatggatacgcgagggtgattgtatgtctgcagcaaaaacaaaatacggcaatgaaggtaatttgaacgctgctgctttaggagttcagaaaaacgttgaagctcttgatgcgaatgatttgaaaaccgcagataaagttaacgaactggtagaaaacgttaataatatcaatgatgccttagaaatggctacggatatttccgtcatccaacaaattgagaaaaaccgtgttgatatcgtagagcttaagagagtagaaggcgaaaccactactgggctaaacaatttaaccataaatttagaccacctaaaagaagacgttggttaccatgaccctttacaagatggcccatatttaactgtacgtgaaaatattgttcttcttaaaaccgaaataggtcattatgaaaaccaggatataaatggtaatccgttgcctcctggtgaaaccagcgaagccaccggtatgaaacgtcgcatcattgataataccactcaattggtcgaccatcgtcttcgcattgatacccttgaaaggaattatgaagattctgacgtcgggcaactaggtattaaattaaatgaaattcgtgctgaactcgggccccattccgatacggtaggtaaacaacaggcttatacccgaatttctgtattagaaacggctgcaattaatttcaatacatctatcgacgaaattaagactaatattgatttctccggtatgcctataaaggaccgagtaactactttagaaagcaaaactcttaccctagaaaattcagtcaacgttgatttaaaacctcgtgtaacatcaattgaaacccaaataggttctgaatcaactcctacttctattaatggacgtttaagcggtcttcgtactgatgtaaatgaccttaaaaccatagtgggtgttagttcaagtgatggcttacgtttccaagttactgatatcaaccgccgtttaggtagtgaagtatctccggcagctgggaccattaataagcgtttaaatgacgttattatccaagcaaaccaatctacttcatctatccaggatattcaagtagaaattggaaataaccaatccggtattaagggtactttacttaaactcaccaataaggttgacgggacaaaccctaacggtactactgtagaagaacgtggtcttattaacgcggttacttctttagaaacccagatgttaggtaagttgaatgatgccccttccgatggtaagctttatgctcgtcgtaatgctacgtggaccgaagttcctaacgtttctactgaaatagggaccgttaaagctgatttagttgttaccgatggtaatgtggcagctttaacttctagagttactacagcagaagataaaatcactgcattagaaactgaacttgctaaacgtccaccagtggctccagttgctgatggacttccatatgttcttgttgataatgcgtgggtgctattgtcagattttgtgactttaaacccagcaccataataaaagggcttcggcccttttttgctataaatacggttattagaggaataaaccatggcaagtgaatcatataaccctaagcaactcaaggacgcaatcctgcgccgcctgggtgcaccgattacgaatattgaagtaactacagaccaagtatacgattgcatccagcgcgccctggagctctacggtgagtatcattataacggctataacaaaggttatcaggctttttatataggccatgatgacgaagaaaaattccgtaacggcgtatttgaccttaaaggccgtaatatatttgcagtaacacaaattttaagaactaatgtgggttctttaacatctatggatggccaagcgacttatccatggtttactgattttgtattaggcctagctggtattaacggcggtcttggaacttcttgtaacagctttgggcctaatgcctttggtgctgacctcgggtattttacacaattaatgcaatatcgttctatgatgcaggaccttttggttccattgcctgattattggtataacgatgccactgaacagttgaaggtaatgggtaactttgttaaaggcgattttattgtaattgaagtttatactcgctcttttaatggggtcgattctatggtaggaaataccgcaggatatggatatgcctctggtgggtgcgacgaaaatgaatggagccccggagctatttgggataacccggctcgtcgtatttcaggtatgagggcaggtgaagaccttggtttgcaagatggttcatataataaccgttgggtcaaagattatgcgacggcattggttaaagaagtcaatggtaatattttggccaaacaccaaggcatgcaacttgcgggtggaaccactgtagatggtattcgattgattgaagaagctcgtttagaaaaagaacgccttcgcgaagaattagatttactcgacccaccaacacctattttaattggataattatggctactttcgattcgagtttatttgccaagctggaaaataatactggctatgctaacacgaacgaaactgaaataatgaatccgttcgtcaacttctacaagcatgagaatacccaaacattggctgatgctttagttgctgagtctattcaaatgcgtggtattgagctttattatataccacgtgaatacgttaatccagaccagctatttggcgaagaccttcagaacaaatttactaaagcctggaaatttgcaggttatttggattcctttgaaggttattccggtgacaatacttatttcagtaagttcggtatgatggttaatgatgaagtaacaatcacaattaaccctaacctttttaaacatcaatgcaatggcactgaacctgtttcaggtgatttgatttatttcccaatggacaacagcctattcgaaattaactgggtacaaccttacgacccattctatcaagtaggagctaacgtccagcggcgcatcaccgctaccaagttcatttacaatggtgaagaacttcgccctgaattacagagaaatgaaggtattaatatccctgagtttagtgagcttgatttaatgcctgttaagaatatcgacggattggctgatatctccgacattcaatatgaagaggtcaatgagattaatgctgaagcggcggaattcgtacatccttatgttgtaattaatggacgaggagaggatgctcctcctacagcatttgatgatgcttttttagatgattaaataatacatggcgcaccatgcgccattttgagaggtgatttatttttggccactggtacaattcatcgctgcgtcgctacattgttttgatgggtgatttattttcccatgtccaagtagcgcgccaaagagaagatacaggacttaaatttattaaggttcctattacgtatgcttctaaagaaagatttatggcaaatttgggtaaatggacggcagtacagaatattccaaatcctaatatgtctcctaaagaacgagccgaacaaaaggctaaagtggaaacggttcttccacgtatgaaccttcaaatggttgatatgctttataactcacaatacaaaacagctcttcagaacagaacacaaatccaatttgagaatggtgacccgagaaaacgagttagccaatattctcctactccagtaaaaatgattttcgaactgggtatttacactagaacccaagatgatatgttccaaattgtggaacagattatgccttatttccaacctcactttaatacaacaatcactgaactctatacaaacgagattaaatttgaccgtgatattcgtattgtgttccagtctattgcaatggacgaacaattagaaggcgataccacttcacgtcgtcgtttagaatggtccatgatgtttgaggttaacgggtggttatatcctccagttaaagaaatggaaggcgaaattaaaaccatttatcttgatttctttgctaactcaaaggaactcgctcctgaaggtaatttcgaatcagttgatagtgaagtggttccgagaggtgtagaacaaacagaatgggatggaagctccgttcaaacatattcacaagatattccagtgcctgtcgagccagcgcctccagcaccaaggagaaacccatgagcgatttagatatcagtaaattaatggatattaccgacctccctggcttgactggggacgaggtagttccttatgaaccattagtattaaaagaagtggaaagtaatcctcagaaccgtactccggatttagaagatgactattcagtggttcgtagaaacctccattttcaacagcaaatgttaatggatgcaggtaaaatatttttagaagccgctaagaacgcagaatcaccgcgccatatggaagtatttgccacattaatgggtcagatgactaccactaacaaagagcttttaaaacttcataaagaaatgaaagatattaccgctgaacaaatcggtactaaaggtggagagcctaatcaaactaatatccaaaatgctactatttttatgggttcaccaaccgatttaatggatgaagtgggcgatgcttatgaagcccaggaagaacgtgagaaggtaattaatggaacaaccagttaacgtattaagcgatgaccatccactaaacgaaggcaagactatagtcattaagccaccgggttcgcttgaacgtaaaacagaagaaggtatcaattggattaaatcccaatgggatgacaaatggtaccctgaaaagtttagtgattatttacgtatccataaaatagttaaaattcctaataacggcgaccgtccaaacgaattccaaacgtttaaagataaaatgaataaacgtacccgttatatgggccttcctaaccttaaacgagcaaatataaaaactcaatggactcgtgaaatggttagtgaatggaagaaatgtcgtgatgacattgtctattttgccgaaacttattgtgcaattacacacattgactacggtacaattaaggttcaacttcgtgattatcagcgtgatatgcttaaaatcatgagcaagaaccgtatgacgacttgtaacctgtctcgccagttaggtaaaacaaccgttgttgctatattccttgcccactttgtttgctttaacaaagataaggcagtaggtattcttgcgcataaaggctcaatgtcagccgaagtacttgaccgtaccaaacaagctattgaattgcttccggatttcttacaacctggtatcgtagaatggaacaaaggctcaattgagttggataacggtagttctattggtgcttatgcttcgtctccagacgccgtgcgtggtaactccttcgcaatgatttatattgacgaatgtgcgtttatccctaacttcctggattcatggcttgctatccaacctgttatttcatcaggtcgtcgttcaaagattattattacaaccaccccaaatggattaaaccacttctatgatatttggactgctgcagtagaaggtaaatcaggctttgcaccatatacggccatctggaactcagttaaggaacgtctttataacgatgcagatatatttgacgatggttgggaatggtcttctcagacaatctctgcgtcctctttagcgcaatttagacaggagcactgtgcagagttccaaggcacaagtggcacattaattagtggtatgaaattggccattatggattgggtggaagttactcctgaaaatggatatttctatcgtttccatgagcctgaccctacacacaaatatattgcttcattagactgctcagagggtcgtggacaggactaccacgctttacacattattgacgttacaacggatgaatgggagcaggttgctgttttgcattctaatgaaatatcccatatgattctccctgacatagtgtataaatatctaatggagtataatgaggctcctgtatacattgaacttaacagcacaggtgtctcggttgccaaatcactttatatggaccttgaatacgaaaacgttatttgtgattcgatgcaagatttgggtatgaaacaaaccagacgaactaaacccgtaggctgttctacattaaaagaccttattgaaaaggacaaattaaaacttaatcataagcaaactataatggaattccgtacctttagccagaacaagttatcttgggctgcagaagatggtttccatgatgaccttgtgatgagtttagtgatttttgcctggttaacgacccagcaaaaatttgccgacttcattgaccgagacgaaatgcgtttagcatctgaagtctttagtcgtgagttggaagatatgaacgaagaatataatccagtcgttttcgtggatgctggcgataattcttatgaatattcaccgttgaatcatggtatttcgtttatataaataacaataaagcataaccaagaggattcaaaatgtctttattatcaccgggcattgagctcaaagaaacgtccgtacagagtactgtcgttcgtaacgcaacgggtcgtgcagcgctggttggtaaattccagtggggccctgctttccaggtaactcagattactaatgaagttgaactggtcgacttatttggaggtcctaataacgaagttgctgattacttcatgtcgggtatgaacttcctccagtatggtaacgaccttcgtactgttcgtgttgttaaccgtgaattcgctaaaaacgcgtctccggtagcgggtaacgtccaaaccactattactactgcaggttctaactatgcggtaggcgataaaattaatatcaaatataaccagactgttgttgaatctgaaggtcgtgtgacttctgtagatacggatggtaaaattctttccgtgtttatcccatcagcaaaaattattgcttatgcacgttctttaaaccagtatccgaacctcggccctgcgtggactgctgaagttacttctgcctcttccggtgtttctggtactattactgtcggtaaaattgtaaccgattccggtattctgttgactgaagcagagaacagtgaagaagctattacttccctggagttccaagcatctcttaaacagtttggtatgcctggtgtggtcgccctttatcctggtgaaattggtagtactctggaagttgaaattgtttctaaagcggcttatgatgctggttcttctaaaatgctggatatttatcctggcggtggtacccgtgcttctattgccaaggcagtatttaactacggcccgcaaacagatgaccaatacgcaattattgttcgtcgtgatggcgctatcgtagaatctgtcgtactttctaccaaagaaggtgaaaaagacgtttacggtaataacatttatcttgacgactatttcgctaaaggtacttctaactatatttttgctacctctttgaactggcctaaaggcttcagtggtatcattaatcttatgggtggtgtatctgctaacgatcaggttactgcgagtgatttgatgcagggttgggatttgtttgccgaccgtgaagcactccatattaaccttttgattgctggtgccgttgccggtgaaggtgatgaagttgcttctaccgtccagaaacacgttgttagtattgctgatgaacgtcaggattgcttggcatttatttctcctcctaaaggactgttggttaacgttccattgactcgtgcagtagataatcttatcgactggcgtaccggtgcaggtactttcgataccaacaacatgaacattagcaccacttatgctgctattgatggtaactataaatatcagtatgacaaatataatgacgtaaaccgttgggtgcctctggccgctgatatggctggtttgtgtgcacgtactgatgatgtttctcagccttggatgtctccggcaggttataaccgtggccagattcttaacgttctgaaattggcaattgaaccgcgccaagctcaacgtgaccgcatgtaccaagaagctattaacccagttgttggttttgctggtggcgatggtttcgtattgtttggtgataagactgcaaccaaagttccatctccgatggaccacattaacgttcgccgtctgttcaacatgcttaagaaaaatatcggtgatgcctctaaatataaactgtttgaattgaacgacaacttcactcgttcaagcttccgtatggaagtttctcagtacttagatggtattaaggcacttggtgggatttatgaaggacgtgtggtttgtgatactacagtgaacacccctgcggttatcgaccgtaacgagtttattgctaatatatacatcaaaccggcccgttctattaactacatcacgttgaacttcgttgcaacgagcactggtgctgattttgatgaattgattggacctttagtataatctattatcccaggctgtaatataaagaacctaaaaccattataccatgagtttggttacagcgtacatcacgtagaattgcgcctgggattgattattctttaggaatatgatttatcaactgttataaataaattaatcagaacgttcctggtgtgtccaggaactgacttaagaggcatcccatggagttgacagatatcactcgtgcgtttgagtcaggtgactttgcacgccctaaccttttcgaagtggaaattccatttctgggtaaaaactttagctttaaatgtaaagcagcacctatgccggcaggcattgtagaaaaagtaccggttggctacatgaaccgtaaaattaacgtagccggtgaccgtacgtttgatgattggaccattaccatttataacgatgatgcacatgacacccgtcaagcaattgtcgattggcagaatctctgtcacggtatgaccaatgaaattaccggtgcagcacctgcagaatataagaaacaagcagtagttcgccagttccatcgtgacggcaagactgtgaccaaagaagttacaatttacggcttatggcctactaacgttggtgaagtccagatggattgggacagcaacaacgaggtagaaactttcgaatctacgttcgctatcgattggtgggaatgagtataaatagaattatcaaggagcttcggctccttatcccattcatcggagactctaatggcaaactttaatacaatattaagttttcttaagccatgggctaatgaagacgaaaaagaatataaacaacaaattaataacaatttagagtctgtcaccgcacctaagcttgatgatggcgctcgcgaaattgagacacaagagcaaaatattccttataatgctcttatgcaacagatgtttggtagtaatgagcctgaagttaaaaataccagggaacttattgatacctaccgtaatttaatgaacaactatgaagtcgacaacgccgtacaggaaattgtgtctgacgctattgtctatgaggatgataaagaagtagttgcattgaatttagacgggacagaatttagtcaagcaattaaagataaaatcttggccgaattcagtgaagttttaaaccttttaaatttccaacgtaaaggtactgaccatttccaacgctggtatgtagactcaagaattttctttcataaaattataaaccctaaaaaaatgaaagatggcgtacaagagcttcgtcgcttagacccacgccaagtccaatatattcgtgaaatcgttacacgtatggaagatggcgttaaagttgtagacggatatcgcgagtttttcgtttatgatacaggccatgaaagttattgcgctgatggacgcatttattcagccgggactaaagttaaaattcctcgtgctgcagtggtttatgctcattctggattattagattgttgtggtaaaaacatcattggctatttgcaacgtgctattaagcctgcaaaccagcttaaattgatggaagacgcaatggtcatctaccgtattacacgtgctcctgaccgtcgtgtgttttatatcgatacaggtaatatgccttcacgtaaggctgcagcacaaatgcaacatatcatgaacacgatgaaaaaccgtgtggtgtatgatgcttcgacaggtaaaattaaaaaccaacaacacaatatgtccatgactgaagactattggttgcaacgtcgtgatggtaaagcggtaacagaagttgatacaatgccaggtgctactggtatgagtgatatggatgacgttctttatttccgcacagcactttatcgtgcgctgcgtgttcctgaatcgcgtatccctagcgagtctaattctggtgttatgtttgatgccggtacagcaatcactcgtgacgaattaaaattctctaaatggattcgtcaactacaaaacaaatttgaagaaattttcctagacccgttaaaaacaaacctcattcttaaaaagattattacagaagatgagtgggaaaaggaaataaataatattaaagttacgtttaaccgtgatagctatttcagtgaaatgaaagatgctgaaatcatggaacgcagaatcaatatgctaacgatggctgaaccatttattggtaagtatatttcacatcaaacggctatgaaagatttcctccaaatgaccgacgaagaaattaatcaagaagctaagcaaattgaagaagagtctaaagaggctcgtttccaaaacccagatgaagaagaagaggatttctaatggaagatttaatcgaagctattaaatcaaacgacctcgtagcagttcgtaaagcagcagccccgcttatcgaatctcgagtaaccgctttgattgaagcccgtaaagcagaaattgctcgctccgttatgattgaaggcgaagaagctgacgaagatgacgaagacgacgaaaaatccgataaagcagataagaaagacaaaaaagaatctgacgatgcggatgatgacgaggacgacgaataatgttccttatccctgatgattacgaattaactctagaaagcgtagaggccaaaattccagaagcacagggacgttttgctgctctttctgaagcgctcgagaaaagcgatataaataatcttgtagagaacatgattgctgaaggcgatatcgaatgtgctatcgctcttggttctttaaatgaatcaatggctcttaacgaatttatcgttaaacacgtttcctctaaaggtgagcttactcgtactaaagatattaaaacccgtcaacgtaatgcgttccaaacgacaggtttatctaaagcaaaacgccgtcagattgctcgtaaagcatctaaaaccaaacgtgctaatccgtctactcaagtacgtgccgaacgtaagcgtaagaaagcccgttctaaacgtaaagcttttggacttaactaatgaaacctgaattgctcatcgaacattggggacaaccaggtgaaattatcgatggggttcctatgttggaatctcatgatggaaaaaattctgggcttgctcccggcctttatatagaaggcattttcatgcaagcagaggtagttaaccgtaataaacgcctttacccaaaacctattttggaaaaagccgttgccgattatatggcagaacaggttgctactaaacaagctttaggagaattaaaccacccacctcgtgctaacgttgaccctatgcaagctgctatcattattgaagatatgtggtggaaaggtaatgatgtttatggacgtgcacgtatcatcgaaggtgaccatggccctggtgataaactagctgcaaatatccgagctggctgggttcctggtgttagttctcgcggtcttggttctttaactgaaaccaataaaggatataagcgtgtaaacgaaggttataaattaaccgtcggtgttgatgcagtatggggaccatctgctcctgatgcttatgtaactccgaagcaaattacagaatcacaaacggtagaaaccgataccagtgccgatgacgcctttatggctctcgcagaggccatgaaaaaagcgttataaatattattatctaaacaacaggactacaaaatgcttaaagaacaactgatcgccgaagcacagaatattgatgcttccgttgctcttgacagtattttcgaatcagttaatatttctccggaagcaaaagaaactttcggcactgtattcgaagctaccgtcaagcaacacgccgtgaaactggctgaatctcacatcgctaaaatcgctgaaaaagcggaagaagaagtcgagaaaaataaagaagaagctgaagaaaaagccgataagaaaatccaagaagctgcaggtcgtttccttgaccacgttgctaaagaatggatggctgaaaaccagctggctgttgataaaggtattaaagccgaactgttcgaatccatgttgatgggtatgaaagaactgtttgttgaacacaatgtggttgttccagaagaagcagtagatgttgttgctgaaatggaagaagaactccaagagcagaaagatgaaaccgctcgtctgttcgaagaagttggtaagcgcgacgcgtatattaattacgtacagcgtgaagttgctgttacggaagcaactaaagacctgactgaatcccaaaaagaaaaagttagttctctggtagaaggcatggattattccgatgcattcggtagaaaaattggcgctattgttgaaatggttaaaggtcagtctgacgttgaaaacccaatcaccgaagccgctataaataaaaatgtagacgatgctgcggcactgaattacatttcagaagcagttgaagaaaaaggcgctaagcctaccctgtccttcgcggacctgtctgcaatcgcagcatcacgaatttcttaatttaataaggttatacaacacatgaaaaagaatgcattagttcaaaaatggtccgctctgctggaaaacgaagcccttcctgaaatcgtgggtgcttctaaacaagctatcatcgctaaaattttcgaaaaccaggaacaagacatcctgactgccccggaataccgtgatgaaaaaatctctgaagcatttggttctttcctgaccgaagctgaaattggtggtgaccacggttatgatgctaccaatatcgcagctggccagacttctggtgctgtaactcagattgggccggcagtaatgggtatggttcgtcgtgctattcctcatctgattgcttttgatatttgtggtgttcagcctctgaataaccctaccggccaggtatttgccctgcgcgcagtttatggtaaagaccctgtcgctgctggcgctaaagaagctttccacccgatgtattctccggactctatgttctctggtcagggtgctgctgaatctttcgaagcactggctgcaagcaaagttctggaagttggtaaaatttattctcacttcttcgaagctaccggtgctgcacacttccaggctgttgaagccgtaaccgttgatgctgctgctactgatgccgctaaactggatgctgctgttaccgctttgattgaagcaggtaagttggctgaattggctgaaggtatggctacttctatcgctgaacttcaggaaggctttaacggttctaccgataacccgtggaacgaaatgggcttccgcatcgacaaacaagttatcgaagctaaatcccgtcagctgaaagcaagctactctatcgaactggcacaggaccttcgtgcagtacacggtatggatgcagatgctgaactgtccggtatccttgctaccgaaattatgctcgaaatcaaccgtgaagttatcgattggattaactactctgcacaggttggtaaatctggtatgaccaacaccgttggcgctaaagctggtgtgtttgacttccaggacccgattgatatccgtggtgctcgttgggccggtgagagctttaaagcccttctgttccagattgataaagaagcagccgaaatcgctcgtcagaccggtcgtggtgctggtaacttcatcatcgcttcccgtaacgtagttaacgtactggctgcagttgatacttctgtaagttatgcagctcaaggtctgggtcaaggtttcaacgttgacacaaccaaagcagtatttgccggtgttcttggtggtaaatatcgcgtttacatcgaccagtatgcacgttccgattacttcaccatcggttataaaggcgctaacgaaatggacgcaggtatctactatgctccgtacgttgcactgaccccgctgcgtggttccgatccgaagaacttccaaccggtaatgggcttcaaaactcgttacggtatcggtatcaacccgttcgctgaccctgctgctcaggctcctaccaaacgtatccagaatggtatgcctgacatcgttaacagccttggtctgaatggttacttccgtcgcgtatatgttaaaggtatctaagatataaccttattatgggagacttcggtctcccattcttgtttctgtattatgcaatcttaactcggcggttgatgatatcacggaagtcaatacgattttcttggattttcagccagttaccagatttgtctttggtatgggtagagtattcaccgttccaccagaagtcggtagcataagccatggcttcgtatttcttaactaaggcattcactgcattgccattaggattgttaccgaatttttctaccagagctttgatgtctttatcaagagcggaaagagtagtacgaataaagtttaacttgttcatttttaatctcctcatgttttgataggtctatagtaacatgtgagaatcttgctgtaaacaacttttataaataaacatataccctcaataaggaaagcgcaatggcaaagattaacgaattactgcgcgagtcaacaactacttccagcaactcattgggtcgccctaatcttgttgctttgacccgtgctacaaccaaattgatttaccgtgatattatcgccgaacaacgtactagccagcctattgctgcactgtatggtgtcaaatatcttacccctgataatgaatttagtttccagacaggtgcctcttatggtggtgaagttggttctaaagaccgtgaaactatcccagaactcacagataaggcccaggcgattgctcagggtgaatatttcaagtaccagaatgtggtttataaggctcttaaagcaagcccactcgcgtccactagcgccacagaattggctgatgctcttcaagaaggtttagtgtcattaacatgtcgtctggttcctgatgctgcccataccactaaatttgaagcgagtgatgtagaaatctctgatgctgtattccaggttaataaatggaatgctccggttaagacccgtaaattgaagacggctttgactgtagaattagcgcaggatatggaatcaaatggctttgacgcgccggcgttcttagaagacctcttggctacagtaatggcagatgaaattaataaagacgttctgcaatctctaataaccgtatccaaacgttataaagttactggtgtatctgataacggcatcatcgatttgtcttatgacagtgctcctgaatctgcacgtaaactttatgaactcgtttgtgagatgaattctgaaatccagaaaactacttcttattctggcacgtttgttgtggcttcaagtcgtgtggctgcaatgcttgcaggttctggctggttaaaacataaacccgaagataataattggcttccggaaactgcatacggatatttgttgaatggtctgcctctgttttgtgacgttaacagtccattagattatgttaccgttggtgttaaagagaattacggcggtaatgaagttgtcggttctattttctacgctccctataccgaaggcttagatttagatgaccaagaacacgtcggtgcttataaggttattgttgacccggattcattacaaccttctatttctctgatggttcgttatgcactatcagctaacccgtacaccgtggctaaagacgataaagaagctcgtgttatcgatgcaaccaatatggatttaatggctggacagagcaatatgtcttatctggttggcgttaaacttccggcaattatttacgaggctgattaatgtctaagattgtagacctaattaaagaatccacattgacggctgccagctcggttggccgtcctgctcttctttcatacacccaagcaactaataaacgaatctttaaagccctagttgctgaacaaaaaacaaatcaaccggttgctgctctgtatggggtacgtgtactgaatcctgacgacaaaatgacttatcttggtggagcaacatttgcgggccagattggtatgacggaacgtgaaaatattccagaatttactgattcatctacagcttatgcggtcggtgatatgttccagtttgaaagcgtagtgtttaaagttctagaagcatctcctttcgccggaaccacagaaaccaacctcagcgaagttatttctgaagcagtggcagccggccatatccgtatggtgtcggatgctgctattacttctaaatttgaacaaggccatcctgaaattgctgaaaccggattccgtatcgacaaatggcaatctgaagttaaatcacgtaaactgaaaacttcattgacagtcgaattagcccaagacctagaatctaacgggtttaatgctcctaatttcgttgaaaatctgctaggcattcaaatggcagaagaaattaataaggatgtattacagtcattaattaccgtgagctctcgttttaaagtccagggtgtttctgaaaagggtgtattagaccttaccaaccctcgctacgataatgcccaggaccgtgctcgcacattatattattatatgtgtgagatgaactctgccgtccaacgacagacttcttttgccgggacttatgcagtagctagttctcgttgtgctgctattctcgccgcctctggttgggttgagaaaaaggaagaccaggacgaattggcttatggtatattaaagaatggcctaccactttatgctgatatgaatagtccatgtgattatgttattgttggtgtaaatgcccagatgggtgaaggacagacggtcgcatctttatattatgcgccttatacggaaggtttgaatgtggttgacgaagaaggtgatacttcagttggtgaatttaaggttattgttgacccggaaagcttacaacctacagtagcattgcttgctcgttatgcattgactgcaaacccttataccgtcgctaaggacgataaagaagcccgcattattgatggttctgatatggacaaaatggctaatcaaagtcaattgagttcttatctcggcgtaaaattaccgcctttagaaaaataaaagggaccgtaaggtccctttatcgtttatttggatactagttcaatccatacatgtcttaatgtttcttttacgcactcaacgagctgctttttaacttcaacgggattttccgcatcagttaattccaattcttcacgggcggcttcttcaaggatatcctggactgtcaagcccatcacctttccgaaatccttcggcgatacttcgccaatcttactgatgacattgttaatgcggttaacagtcacataatcagtgaattgccacatcaaatccatatcatcttgggataaaaccactgcaactttaataggcttatcagactttttcttctcgctgaatttagagttcttacatttaatcgctacacgatttccattaggaagccaggtaggaacatcaggtttcagtacaaagccttcagccgtgaatactttaccttctaccttaggaataaagtctgtcgagtttgcaatagttaagccagcgttatccactgcaaaattataatcaggaacaactgaatcaaaatcattaggaagtttaataaggtcttcaaagctaccggtggccagacatggagctaccttaaacttatggataatacagaaggcttccatcaatgtatcggttagaacagattctgagccatcttctttagtaactcggatatcgaacacataaaagtctttatcaccatagtccacattcttctggatacctggcccagcgaattcgccgtaaatctgatatgactggtaattaatcgattcgattagatgttgaacagatttaatagaatcggcatagttcttaagtacaatttcataaccatagaaatcttcagcagggaggatagggccagtgcgcttggcgcatgtgactgcgtcacgttctatgattaaactaaagttggttccatgaatcttctcacgtgctacccattcaccaccagtcaaaccgttagtacggagtttttcgataaacttactgttgtagtggttttcgagactgctatatttcttgaacataaatcaccataataaatataattaaatagaagagctagtagtcttctgtcaccaagccaaatggtttaacggaaggacctagacccattatatcacacctaaatttaaagcatattactttgaactagaacgcgctttgcgccgaaccttgttgttcaatcttttacgataaacaaccttttctttcgctttaaatttggccttggcttgttctacatcaacccatgctttggccatgtccttagcggtcccgcccatttttttagcaatttctataaaattcaacccagattcgtgtaaaaaatgtactttaaccttatccataacaattctctcgttgagttggtaaacccatcttaacatagaatttttaacttgtaaacaggaattttgtactttaatgcaaaatgggccgcaaggcccattattaataaatgtaatcgtatataataccagcttctaaagcggtgcgatgaataattcgaccattacgagattcttgtacatcaacctctgaatagtcggtaatcattttttgaagtgtatatcggtgcaaataatacgggctatccgggtcatctgttttccagtctttgccttcaagagtcattttctggatttcatccataacccaccaaccaacccaaatatatgctgaattacgaacagggagtggatgaacgtaaggtaattcgccatccggaaccggtgcgactttagccgtgactgttacattaccggtttttgtgacagtcgccgggttataatcagtcgccgaaaccacaacagaaacttcaataacctgtgaaccttcagtgcttgtatcgattgctagagtatccgtggtgccaactacaggagaaccgtctttcttccaagaataggcaaaagtagcaccagcaggagcgccgaccacatccgctttaaaagaagctggagtgccttccggaacattaatcgaagctggggttaatgtcacagaaacaccggaaatggttttattctggatagttaaagttgtttcggcttcagctgtttctggttcgccgtccgccggtgtagttgttgcaacaactttaatagtcttgctgcctgccgggccaacagcaacataatccattgcagcagtcacagaagattgaggaacgccatcaacggtccagacaaatgattcggtaccttcagctgcagcaccggaaccggtcgcagtgaaattggttgttgctccaataacggccgtagccgccaaaggagcaatagttacggtataagccataataaacccttattttaaagtgacaaaagatgagttacgagtttcacgtactaatactgaaccattacgattaatgtaataaatcagactaaataatgtttggtgggcagaaggatgttggaaagcagttggacgttctttccaatccggagtctcagaaatccattggtaaatccaccaaggaacggtgcaataacctgggttcttaccgataagcaaaagattaggactgaagttttcaggtaaagagaatacaggtttttcagattcaacaaccttggctatagcccctttgaatttctcttcgtcaaatggaacatcctcttcgataatctctaccttaggaagttcggctacctcaacgacttctactgcagcctcaggggcatcgaacaacagggttgcttcttctttagctggttctacaccttcgataaaatctttatcacctgtaagttcgtcggcagcatcaatcaaatcagaaatggacaacccttcggtttccggaagtggttcgtcagccaaggctttaaggccttcagagatatcgataatcaaattatcaaacgaacgggttttcttaagttttaaaccgaactgttcgccgtattcgattaacttagctttagcttcttttttatcttcgagtgcacgaagctcttcaatatattgagtatccataattagtctcttgttggtgtataaatataactatatttataactgagaattacttatgcaaattcaagtacattttgataattttagtcatgtccgtattgaatgcgatgaatctacattctacgaactcagagactattttagctttgaagctgatgggtataaattcaaccctaaatttcgttatggccaatgggacggacgtattcgccttctggattacaaccgtaaacttccttatggattggtccctcaaattaaaaagttcgctgaacaatttgaatactctctgtggattgacccacgtattcttgaacaggaagatatttctcgtgaagattttgattcatgggtggcttctcaagaaatttattcagggtctaccaagattgagcctcattggtatcagaatgaagccgtatacaacggcctgacaaaacgtcgcgcaattctgaatttacctacatctgcaggtaaatcattaatccaggcactcctgagtcgatattacgttgagaactatgaaggtaaaatcctcatcttagttcctactactgcacttgtcgaccagatgattaacgacttcatcgattatcgtctgttccctaaagccgcaatgcttggtattcgttcaggtactgctcgtgattccgatgcaatgatttatgtttcaacttatcaaaccgctatcaagcaacctaaagaatggtttgctcagttcggtatgtttatgaacgacgaatgccatttggctacaggtaaatctatttctactatcatcgaaggcctaaccaactgtatgtttaaattcggtttgtctggttctttaaaagatggtaaagctaatttaatgcaatatatgggtttgtttggtgatgtgtttaagccagtatccacctcccagttaatggaagaaggacaggttactgaccttaaaatcaacagtattttccttcgatacccagacgaattcacggttaaaatgaaaggtaaagattaccaatcagaaatcaaggtcattactaaggctactcgtcgtaataaatgggttgctaatttagctgttaaactcgctaagaaagaagagaacgtattcctgatgtttaaaaacatcgaacacggtaaaactctttttgaaatggttaaagagcaacataaagaagtttattacgtatcaggtgaagttaataccgaaacgcgtaatgctctgaaagtaatggcggaaaatggtaagggtattattgttgtggcaagttatggtgtgttctctacaggtatttccgttaagaaccttcaccacgttgtatttgcccatccagtaaaatctaaaatcattgtactccagacaattggtcgtgtactccgtaaacatgcctctaaatcaacagcacaggtatgggatatcatcgacgacatgggtgttaagcctaaatcagctacggctaaaaagaaatatgttcatttgaactacgccctcaaacacgctttagaacgtattcaacgttatgctgatgagaaatttaattacgtaatgaaacaggtggatttatgaaaacctttaaagaagttattcaagaagcatctattgaaagcttcatggctaaaattggttcttgtcagactatggatggtctgaaggaattggaaaagtattacaaaactcgtagtaaggaagccgaacttcgtgattcggatgatattagcgtgcgtgatgcattggctggtaagagagctgaattggagtcgatggacgacgaggaagaggaagatttctaaacaaaaaaggcccaacctttcggaagggccaataaccataaatggctatacacactagactaaagtagtaattgggtttcgttcagctgttcttcagtgttttccgtaaccggcaagctttgaacgtaattatagcatgagcccggatgaaccggacctttttctgtttcaacaaccaatgcagcatcgattggagttttacagacaacgcaaatcttatctgacatgattgtctccttagtttaacttacatacctatttattacttgctaaagcagcattaatgaatttttggagttcgtccatccgctctttagatggtttagggcatttattgatgactggtttacgataactcatttgcccgcctcaaattg